European Patent Application EP 4 129 319 A1, published February 8, 2023. Title: Pore-forming antimicrobial peptides. Applicant: Masarykova univerzita. The sequence listing filed with the application follows.

SEQUENCE LISTING (290 sequences)

SEQ ID NO: 1 - protein, 22 aa, artificial
  antimicrobial peptide pattern
  variant (1)..(1): Ala or Met or Val or Leu or Ile
  variant (4)..(4): Ala or Met or Val or Leu or Ile
  variant (5)..(5): Ala or Met or Val or Leu or Ile
  variant (8)..(8): Ala or Met or Val or Leu or Ile
  variant (9)..(9): Trp or Phe
  variant (10)..(10): Thr or Gln or Ser or Asn
  variant (11)..(11): Trp or Phe
  variant (12)..(12): Ala or Met or Val or Leu or Ile
  variant (13)..(13): Thr or Gln or Ser or Asn
  variant (14)..(14): Thr or Gln or Ser or Asn
  variant (15)..(15): Ala or Met or Val or Leu or Ile
  variant (16)..(16): Asp or Glu
  variant (17)..(17): Thr or Gln or Ser or Asn
  variant (18)..(18): Thr or Gln or Ser or Asn
  variant (19)..(19): Ala or Met or Val or Leu or Ile
  variant (20)..(20): Thr or Gln or Ser or Asn
  variant (21)..(21): Asp or Glu
  variant (22)..(22): Ala or Met or Val or Leu or Ile
XKKXXKKXXXXXXXXXXXXXXX

SEQ ID NO: 2 - protein, 22 aa, artificial
  antimicrobial peptide pattern
  variant (1)..(1): Ala or Met or Val or Leu or Ile
  variant (2)..(2): Asp or Glu
  variant (3)..(3): Asp or Glu
  variant (4)..(4): Ala or Met or Val or Leu or Ile
  variant (5)..(5): Ala or Met or Val or Leu or Ile
  variant (6)..(6): Thr or Gln or Ser or Asn
  variant (7)..(7): Thr or Gln or Ser or Asn
  variant (8)..(8): Ala or Met or Val or Leu or Ile
  variant (9)..(9): Trp or Phe
  variant (10)..(10): Thr or Gln or Ser or Asn
  variant (11)..(11): Trp or Phe
  variant (12)..(12): Ala or Met or Val or Leu or Ile
  variant (14)..(14): Thr or Gln or Ser or Asn
  variant (15)..(15): Ala or Met or Val or Leu or Ile
  variant (17)..(17): Thr or Gln or Ser or Asn
  variant (19)..(19): Ala or Met or Val or Leu or Ile
  variant (20)..(20): Thr or Gln or Ser or Asn
  variant (22)..(22): Ala or Met or Val or Leu or Ile
XXXXXXXXXXXXKXXKXKXXKX

SEQ ID NO: 3 - protein, 22 aa, artificial
  antimicrobial peptide pattern
  variant (1)..(1): Ala or Met or Val or Leu or Ile
  variant (4)..(4): Ala or Met or Val or Leu or Ile
  variant (5)..(5): Ala or Met or Val or Leu or Ile
  variant (8)..(8): Ala or Met or Val or Leu or Ile
  variant (9)..(9): Trp or Phe
  variant (10)..(10): Thr or Gln or Ser or Asn
  variant (11)..(11): Trp or Phe
  variant (12)..(12): Ala or Met or Val or Leu or Ile
  variant (13)..(13): Thr or Gln or Ser or Asn
  variant (14)..(14): Thr or Gln or Ser or Asn
  variant (15)..(15): Ala or Met or Val or Leu or Ile
  variant (16)..(16): Asp or Glu
  variant (17)..(17): Thr or Gln or Ser or Asn
  variant (18)..(18): Asp or Glu
  variant (19)..(19): Ala or Met or Val or Leu or Ile
  variant (20)..(20): Thr or Gln or Ser or Asn
  variant (21)..(21): Thr or Gln or Ser or Asn
  variant (22)..(22): Ala or Met or Val or Leu or Ile
XKKXXKKXXXXXXXXXXXXXXX

SEQ ID NO: 4 - protein, 22 aa, artificial
  antimicrobial peptide pattern
  variant (1)..(1): Ala or Met or Val or Leu or Ile
  variant (2)..(2): Asp or Glu
  variant (3)..(3): Thr or Gln or Ser or Asn
  variant (4)..(4): Ala or Met or Val or Leu or Ile
  variant (5)..(5): Ala or Met or Val or Leu or Ile
  variant (6)..(6): Thr or Gln or Ser or Asn
  variant (7)..(7): Asp or Glu
  variant (8)..(8): Ala or Met or Val or Leu or Ile
  variant (9)..(9): Trp or Phe
  variant (10)..(10): Thr or Gln or Ser or Asn
  variant (11)..(11): Trp or Phe
  variant (12)..(12): Ala or Met or Val or Leu or Ile
  variant (14)..(14): Thr or Gln or Ser or Asn
  variant (15)..(15): Ala or Met or Val or Leu or Ile
  variant (17)..(17): Thr or Gln or Ser or Asn
  variant (19)..(19): Ala or Met or Val or Leu or Ile
  variant (20)..(20): Thr or Gln or Ser or Asn
  variant (22)..(22): Ala or Met or Val or Leu or Ile
XXXXXXXXXXXXKXXKXKXXKX

SEQ ID NO: 5 - protein, 22 aa, artificial
  antimicrobial peptide pattern
  variant (1)..(1): Ala or Met or Val or Leu or Ile
  variant (4)..(4): Ala or Met or Val or Leu or Ile
  variant (5)..(5): Ala or Met or Val or Leu or Ile
  variant (8)..(8): Ala or Met or Val or Leu or Ile
  variant (9)..(9): Trp or Phe
  variant (10)..(10): Thr or Gln or Ser or Asn
  variant (11)..(11): Trp or Phe
  variant (12)..(12): Ala or Met or Val or Leu or Ile
  variant (13)..(13): Asp or Glu
  variant (14)..(14): Thr or Gln or Ser or Asn
  variant (15)..(15): Ala or Met or Val or Leu or Ile
  variant (16)..(16): Ala or Met or Val or Leu or Ile
  variant (17)..(17): Thr or Gln or Ser or Asn
  variant (18)..(18): Thr or Gln or Ser or Asn
  variant (19)..(19): Ala or Met or Val or Leu or Ile
  variant (20)..(20): Thr or Gln or Ser or Asn
  variant (21)..(21): Asp or Glu
  variant (22)..(22): Ala or Met or Val or Leu or Ile
XKKXXKKXXXXXXXXXXXXXXX

SEQ ID NO: 6 - protein, 22 aa, artificial
  antimicrobial peptide pattern
  variant (1)..(1): Ala or Met or Val or Leu or Ile
  variant (2)..(2): Thr or Gln or Ser or Asn
  variant (3)..(3): Asp or Glu
  variant (4)..(4): Ala or Met or Val or Leu or Ile
  variant (5)..(5): Ala or Met or Val or Leu or Ile
  variant (6)..(6): Asp or Glu
  variant (7)..(7): Thr or Gln or Ser or Asn
  variant (8)..(8): Ala or Met or Val or Leu or Ile
  variant (9)..(9): Trp or Phe
  variant (10)..(10): Thr or Gln or Ser or Asn
  variant (11)..(11): Trp or Phe
  variant (12)..(12): Ala or Met or Val or Leu or Ile
  variant (14)..(14): Thr or Gln or Ser or Asn
  variant (15)..(15): Ala or Met or Val or Leu or Ile
  variant (17)..(17): Thr or Gln or Ser or Asn
  variant (19)..(19): Ala or Met or Val or Leu or Ile
  variant (20)..(20): Thr or Gln or Ser or Asn
  variant (22)..(22): Ala or Met or Val or Leu or Ile
XXXXXXXXXXXXKXXKXKXXKX

SEQ ID NO: 7 - protein, 22 aa, artificial
  antimicrobial peptide pattern
  variant (1)..(1): Ala or Met or Val or Leu or Ile
  variant (4)..(4): Ala or Met or Val or Leu or Ile
  variant (5)..(5): Ala or Met or Val or Leu or Ile
  variant (8)..(8): Ala or Met or Val or Leu or Ile
  variant (9)..(9): Trp or Phe
  variant (10)..(10): Thr or Gln or Ser or Asn
  variant (11)..(11): Trp or Phe
  variant (12)..(12): Ala or Met or Val or Leu or Ile
  variant (13)..(13): Asp or Glu
  variant (14)..(14): Thr or Gln or Ser or Asn
  variant (15)..(15): Ala or Met or Val or Leu or Ile
  variant (16)..(16): Ala or Met or Val or Leu or Ile
  variant (17)..(17): Thr or Gln or Ser or Asn
  variant (18)..(18): Asp or Glu
  variant (19)..(19): Ala or Met or Val or Leu or Ile
  variant (20)..(20): Thr or Gln or Ser or Asn
  variant (21)..(21): Thr or Gln or Ser or Asn
  variant (22)..(22): Ala or Met or Val or Leu or Ile
XKKXXKKXXXXXXXXXXXXXXX

SEQ ID NO: 8 - protein, 22 aa, artificial
  antimicrobial peptide pattern
  variant (1)..(1): Ala or Met or Val or Leu or Ile
  variant (2)..(2): Thr or Gln or Ser or Asn
  variant (3)..(3): Thr or Gln or Ser or Asn
  variant (4)..(4): Ala or Met or Val or Leu or Ile
  variant (5)..(5): Ala or Met or Val or Leu or Ile
  variant (6)..(6): Asp or Glu
  variant (7)..(7): Asp or Glu
  variant (8)..(8): Ala or Met or Val or Leu or Ile
  variant (9)..(9): Trp or Phe
  variant (10)..(10): Thr or Gln or Ser or Asn
  variant (11)..(11): Trp or Phe
  variant (12)..(12): Ala or Met or Val or Leu or Ile
  variant (14)..(14): Thr or Gln or Ser or Asn
  variant (15)..(15): Ala or Met or Val or Leu or Ile
  variant (17)..(17): Thr or Gln or Ser or Asn
  variant (19)..(19): Ala or Met or Val or Leu or Ile
  variant (20)..(20): Thr or Gln or Ser or Asn
  variant (22)..(22): Ala or Met or Val or Leu or Ile
XXXXXXXXXXXXKXXKXKXXKX

SEQ ID NO: 9 - protein, 22 aa, artificial
  antimicrobial peptide pattern
  variant (1)..(1): Ala or Met or Val or Leu or Ile
  variant (4)..(4): Trp or Phe
  variant (5)..(5): Trp or Phe
  variant (8)..(8): Ala or Met or Val or Leu or Ile
  variant (9)..(9): Ala or Met or Val or Leu or Ile
  variant (10)..(10): Thr or Gln or Ser or Asn
  variant (11)..(11): Ala or Met or Val or Leu or Ile
  variant (12)..(12): Ala or Met or Val or Leu or Ile
  variant (13)..(13): Thr or Gln or Ser or Asn
  variant (14)..(14): Thr or Gln or Ser or Asn
  variant (15)..(15): Ala or Met or Val or Leu or Ile
  variant (16)..(16): Trp or Phe
  variant (17)..(17): Thr or Gln or Ser or Asn
  variant (18)..(18): Thr or Gln or Ser or Asn
  variant (19)..(19): Ala or Met or Val or Leu or Ile
  variant (20)..(20): Asp or Glu
  variant (21)..(21): Asp or Glu
  variant (22)..(22): Trp or Phe
XKKXXKKXXXXXXXXXXXXXXX

SEQ ID NO: 10 - protein, 22 aa, artificial
  antimicrobial peptide pattern
  variant (1)..(1): Ala or Met or Val or Leu or Ile
  variant (2)..(2): Asp or Glu
  variant (3)..(3): Asp or Glu
  variant (4)..(4): Trp or Phe
  variant (5)..(5): Trp or Phe
  variant (6)..(6): Thr or Gln or Ser or Asn
  variant (7)..(7): Thr or Gln or Ser or Asn
  variant (8)..(8): Ala or Met or Val or Leu or Ile
  variant (9)..(9): Ala or Met or Val or Leu or Ile
  variant (10)..(10): Thr or Gln or Ser or Asn
  variant (11)..(11): Ala or Met or Val or Leu or Ile
  variant (12)..(12): Ala or Met or Val or Leu or Ile
  variant (14)..(14): Thr or Gln or Ser or Asn
  variant (15)..(15): Ala or Met or Val or Leu or Ile
  variant (16)..(16): Trp or Phe
  variant (17)..(17): Thr or Gln or Ser or Asn
  variant (19)..(19): Ala or Met or Val or Leu or Ile
  variant (22)..(22): Trp or Phe
XXXXXXXXXXXXKXXXXKXKKX

SEQ ID NO: 11 - protein, 22 aa, artificial
  antimicrobial peptide pattern
  variant (1)..(1): Ala or Met or Val or Leu or Ile
  variant (4)..(4): Trp or Phe
  variant (5)..(5): Trp or Phe
  variant (8)..(8): Ala or Met or Val or Leu or Ile
  variant (9)..(9): Ala or Met or Val or Leu or Ile
  variant (10)..(10): Thr or Gln or Ser or Asn
  variant (11)..(11): Ala or Met or Val or Leu or Ile
  variant (12)..(12): Ala or Met or Val or Leu or Ile
  variant (13)..(13): Thr or Gln or Ser or Asn
  variant (14)..(14): Thr or Gln or Ser or Asn
  variant (15)..(15): Ala or Met or Val or Leu or Ile
  variant (16)..(16): Trp or Phe
  variant (17)..(17): Thr or Gln or Ser or Asn
  variant (18)..(18): Asp or Glu
  variant (19)..(19): Ala or Met or Val or Leu or Ile
  variant (20)..(20): Asp or Glu
  variant (21)..(21): Thr or Gln or Ser or Asn
  variant (22)..(22): Trp or Phe
XKKXXKKXXXXXXXXXXXXXXX

SEQ ID NO: 12 - protein, 22 aa, artificial
  antimicrobial peptide pattern
  variant (1)..(1): Ala or Met or Val or Leu or Ile
  variant (2)..(2): Asp or Glu
  variant (3)..(3): Thr or Gln or Ser or Asn
  variant (4)..(4): Trp or Phe
  variant (5)..(5): Trp or Phe
  variant (6)..(6): Thr or Gln or Ser or Asn
  variant (7)..(7): Asp or Glu
  variant (8)..(8): Ala or Met or Val or Leu or Ile
  variant (9)..(9): Ala or Met or Val or Leu or Ile
  variant (10)..(10): Thr or Gln or Ser or Asn
  variant (11)..(11): Ala or Met or Val or Leu or Ile
  variant (12)..(12): Ala or Met or Val or Leu or Ile
  variant (14)..(14): Thr or Gln or Ser or Asn
  variant (15)..(15): Ala or Met or Val or Leu or Ile
  variant (16)..(16): Trp or Phe
  variant (17)..(17): Thr or Gln or Ser or Asn
  variant (19)..(19): Ala or Met or Val or Leu or Ile
  variant (22)..(22): Trp or Phe
XXXXXXXXXXXXKXXXXKXKKX

SEQ ID NO: 13 - protein, 22 aa, artificial
  antimicrobial peptide pattern
  variant (1)..(1): Ala or Met or Val or Leu or Ile
  variant (4)..(4): Trp or Phe
  variant (5)..(5): Trp or Phe
  variant (8)..(8): Ala or Met or Val or Leu or Ile
  variant (9)..(9): Ala or Met or Val or Leu or Ile
  variant (10)..(10): Thr or Gln or Ser or Asn
  variant (11)..(11): Ala or Met or Val or Leu or Ile
  variant (12)..(12): Ala or Met or Val or Leu or Ile
  variant (13)..(13): Asp or Glu
  variant (14)..(14): Thr or Gln or Ser or Asn
  variant (15)..(15): Ala or Met or Val or Leu or Ile
  variant (16)..(16): Trp or Phe
  variant (17)..(17): Thr or Gln or Ser or Asn
  variant (18)..(18): Thr or Gln or Ser or Asn
  variant (19)..(19): Ala or Met or Val or Leu or Ile
  variant (20)..(20): Thr or Gln or Ser or Asn
  variant (21)..(21): Asp or Glu
  variant (22)..(22): Trp or Phe
XKKXXKKXXXXXXXXXXXXXXX

SEQ ID NO: 14 - protein, 22 aa, artificial
  antimicrobial peptide pattern
  variant (1)..(1): Ala or Met or Val or Leu or Ile
  variant (2)..(2): Thr or Gln or Ser or Asn
  variant (3)..(3): Asp or Glu
  variant (4)..(4): Trp or Phe
  variant (5)..(5): Trp or Phe
  variant (6)..(6): Asp or Glu
  variant (7)..(7): Thr or Gln or Ser or Asn
  variant (8)..(8): Ala or Met or Val or Leu or Ile
  variant (9)..(9): Ala or Met or Val or Leu or Ile
  variant (10)..(10): Thr or Gln or Ser or Asn
  variant (11)..(11): Ala or Met or Val or Leu or Ile
  variant (12)..(12): Ala or Met or Val or Leu or Ile
  variant (14)..(14): Thr or Gln or Ser or Asn
  variant (15)..(15): Ala or Met or Val or Leu or Ile
  variant (16)..(16): Trp or Phe
  variant (17)..(17): Thr or Gln or Ser or Asn
  variant (19)..(19): Ala or Met or Val or Leu or Ile
  variant (22)..(22): Trp or Phe
XXXXXXXXXXXXKXXXXKXKKX

SEQ ID NO: 15 - protein, 22 aa, artificial
  antimicrobial peptide pattern
  variant (1)..(1): Ala or Met or Val or Leu or Ile
  variant (4)..(4): Trp or Phe
  variant (5)..(5): Trp or Phe
  variant (8)..(8): Ala or Met or Val or Leu or Ile
  variant (9)..(9): Ala or Met or Val or Leu or Ile
  variant (10)..(10): Thr or Gln or Ser or Asn
  variant (11)..(11): Ala or Met or Val or Leu or Ile
  variant (12)..(12): Ala or Met or Val or Leu or Ile
  variant (13)..(13): Asp or Glu
  variant (14)..(14): Thr or Gln or Ser or Asn
  variant (15)..(15): Ala or Met or Val or Leu or Ile
  variant (16)..(16): Trp or Phe
  variant (17)..(17): Thr or Gln or Ser or Asn
  variant (18)..(18): Asp or Glu
  variant (19)..(19): Ala or Met or Val or Leu or Ile
  variant (20)..(20): Thr or Gln or Ser or Asn
  variant (21)..(21): Thr or Gln or Ser or Asn
  variant (22)..(22): Trp or Phe
XKKXXKKXXXXXXXXXXXXXXX

SEQ ID NO: 16 - protein, 22 aa, artificial
  antimicrobial peptide pattern
  variant (1)..(1): Ala or Met or Val or Leu or Ile
  variant (2)..(2): Thr or Gln or Ser or Asn
  variant (3)..(3): Thr or Gln or Ser or Asn
  variant (4)..(4): Trp or Phe
  variant (5)..(5): Trp or Phe
  variant (6)..(6): Asp or Glu
  variant (7)..(7): Asp or Glu
  variant (8)..(8): Ala or Met or Val or Leu or Ile
  variant (9)..(9): Ala or Met or Val or Leu or Ile
  variant (10)..(10): Thr or Gln or Ser or Asn
  variant (11)..(11): Ala or Met or Val or Leu or Ile
  variant (12)..(12): Ala or Met or Val or Leu or Ile
  variant (14)..(14): Thr or Gln or Ser or Asn
  variant (15)..(15): Ala or Met or Val or Leu or Ile
  variant (16)..(16): Trp or Phe
  variant (17)..(17): Thr or Gln or Ser or Asn
  variant (19)..(19): Ala or Met or Val or Leu or Ile
  variant (22)..(22): Trp or Phe
XXXXXXXXXXXXKXXXXKXKKX

SEQ ID NO: 17 - protein, 22 aa, artificial
  antimicrobial peptide pattern
  variant (1)..(1): Ala or Met or Val or Leu or Ile
  variant (4)..(4): Ala or Met or Val or Leu or Ile
  variant (5)..(5): Ala or Met or Val or Leu or Ile
  variant (8)..(8): Ala or Met or Val or Leu or Ile
  variant (9)..(9): Trp or Phe
  variant (10)..(10): Thr or Gln or Ser or Asn
  variant (11)..(11): Trp or Phe
  variant (12)..(12): Ala or Met or Val or Leu or Ile
  variant (13)..(13): Asp or Glu
  variant (14)..(14): Thr or Gln or Ser or Asn
  variant (15)..(15): Ala or Met or Val or Leu or Ile
  variant (16)..(16): Asp or Glu
  variant (17)..(17): Thr or Gln or Ser or Asn
  variant (18)..(18): Asp or Glu
  variant (19)..(19): Ala or Met or Val or Leu or Ile
  variant (20)..(20): Thr or Gln or Ser or Asn
  variant (21)..(21): Asp or Glu
  variant (22)..(22): Ala or Met or Val or Leu or Ile
XKKXXKKXXXXXXXXXXXXXXX

SEQ ID NO: 18 - protein, 22 aa, artificial
  antimicrobial peptide pattern
  variant (1)..(1): Ala or Met or Val or Leu or Ile
  variant (2)..(2): Asp or Glu
  variant (3)..(3): Asp or Glu
  variant (4)..(4): Ala or Met or Val or Leu or Ile
  variant (5)..(5): Ala or Met or Val or Leu or Ile
  variant (6)..(6): Asp or Glu
  variant (7)..(7): Asp or Glu
  variant (8)..(8): Ala or Met or Val or Leu or Ile
  variant (9)..(9): Trp or Phe
  variant (10)..(10): Thr or Gln or Ser or Asn
  variant (11)..(11): Trp or Phe
  variant (12)..(12): Ala or Met or Val or Leu or Ile
  variant (14)..(14): Thr or Gln or Ser or Asn
  variant (15)..(15): Ala or Met or Val or Leu or Ile
  variant (17)..(17): Thr or Gln or Ser or Asn
  variant (19)..(19): Ala or Met or Val or Leu or Ile
  variant (20)..(20): Thr or Gln or Ser or Asn
  variant (22)..(22): Ala or Met or Val or Leu or Ile
XXXXXXXXXXXXKXXKXKXXKX

SEQ ID NO: 19 - protein, 22 aa, artificial
  antimicrobial peptide pattern
  variant (1)..(1): Ala or Met or Val or Leu or Ile
  variant (4)..(4): Ala or Met or Val or Leu or Ile
  variant (5)..(5): Ala or Met or Val or Leu or Ile
  variant (8)..(8): Ala or Met or Val or Leu or Ile
  variant (9)..(9): Trp or Phe
  variant (10)..(10): Thr or Gln or Ser or Asn
  variant (11)..(11): Trp or Phe
  variant (12)..(12): Ala or Met or Val or Leu or Ile
  variant (13)..(13): Asp or Glu
  variant (14)..(14): Thr or Gln or Ser or Asn
  variant (15)..(15): Ala or Met or Val or Leu or Ile
  variant (16)..(16): Ala or Met or Val or Leu or Ile
  variant (17)..(17): Asp or Glu
  variant (18)..(18): Asp or Glu
  variant (19)..(19): Ala or Met or Val or Leu or Ile
  variant (20)..(20): Thr or Gln or Ser or Asn
  variant (21)..(21): Asp or Glu
  variant (22)..(22): Ala or Met or Val or Leu or Ile
XKKXXKKXXXXXXXXXXXXXXX

SEQ ID NO: 20 - protein, 22 aa, artificial
  antimicrobial peptide pattern
  variant (1)..(1): Ala or Met or Val or Leu or Ile
  variant (2)..(2): Asp or Glu
  variant (3)..(3): Asp or Glu
  variant (4)..(4): Ala or Met or Val or Leu or Ile
  variant (5)..(5): Ala or Met or Val or Leu or Ile
  variant (6)..(6): Asp or Glu
  variant (7)..(7): Asp or Glu
  variant (8)..(8): Ala or Met or Val or Leu or Ile
  variant (9)..(9): Trp or Phe
  variant (10)..(10): Thr or Gln or Ser or Asn
  variant (11)..(11): Trp or Phe
  variant (12)..(12): Ala or Met or Val or Leu or Ile
  variant (14)..(14): Thr or Gln or Ser or Asn
  variant (15)..(15): Ala or Met or Val or Leu or Ile
  variant (16)..(16): Ala or Met or Val or Leu or Ile
  variant (19)..(19): Ala or Met or Val or Leu or Ile
  variant (20)..(20): Thr or Gln or Ser or Asn
  variant (22)..(22): Ala or Met or Val or Leu or Ile
XXXXXXXXXXXXKXXXKKXXKX

SEQ ID NO: 21 - protein, 22 aa, artificial
  antimicrobial peptide pattern
  variant (1)..(1): Ala or Met or Val or Leu or Ile
  variant (4)..(4): Ala or Met or Val or Leu or Ile
  variant (5)..(5): Ala or Met or Val or Leu or Ile
  variant (8)..(8): Ala or Met or Val or Leu or Ile
  variant (9)..(9): Trp or Phe
  variant (10)..(10): Thr or Gln or Ser or Asn
  variant (11)..(11): Trp or Phe
  variant (12)..(12): Ala or Met or Val or Leu or Ile
  variant (13)..(13): Asp or Glu
  variant (14)..(14): Thr or Gln or Ser or Asn
  variant (15)..(15): Ala or Met or Val or Leu or Ile
  variant (16)..(16): Ala or Met or Val or Leu or Ile
  variant (17)..(17): Thr or Gln or Ser or Asn
  variant (18)..(18): Asp or Glu
  variant (19)..(19): Ala or Met or Val or Leu or Ile
  variant (20)..(20): Asp or Glu
  variant (21)..(21): Asp or Glu
  variant (22)..(22): Ala or Met or Val or Leu or Ile
XKKXXKKXXXXXXXXXXXXXXX

SEQ ID NO: 22 - protein, 22 aa, artificial
  antimicrobial peptide pattern
  variant (1)..(1): Ala or Met or Val or Leu or Ile
  variant (2)..(2): Asp or Glu
  variant (3)..(3): Asp or Glu
  variant (4)..(4): Ala or Met or Val or Leu or Ile
  variant (5)..(5): Ala or Met or Val or Leu or Ile
  variant (6)..(6): Asp or Glu
  variant (7)..(7): Asp or Glu
  variant (8)..(8): Ala or Met or Val or Leu or Ile
  variant (9)..(9): Trp or Phe
  variant (10)..(10): Thr or Gln or Ser or Asn
  variant (11)..(11): Trp or Phe
  variant (12)..(12): Ala or Met or Val or Leu or Ile
  variant (14)..(14): Thr or Gln or Ser or Asn
  variant (15)..(15): Ala or Met or Val or Leu or Ile
  variant (16)..(16): Ala or Met or Val or Leu or Ile
  variant (17)..(17): Thr or Gln or Ser or Asn
  variant (19)..(19): Ala or Met or Val or Leu or Ile
  variant (22)..(22): Ala or Met or Val or Leu or Ile
XXXXXXXXXXXXKXXXXKXKKX

SEQ ID NO: 23 - protein, 22 aa, artificial
  antimicrobial peptide pattern
  variant (1)..(1): Ala or Met or Val or Leu or Ile
  variant (4)..(4): Ala or Met or Val or Leu or Ile
  variant (5)..(5): Ala or Met or Val or Leu or Ile
  variant (8)..(8): Ala or Met or Val or Leu or Ile
  variant (9)..(9): Trp or Phe
  variant (10)..(10): Thr or Gln or Ser or Asn
  variant (11)..(11): Trp or Phe
  variant (12)..(12): Ala or Met or Val or Leu or Ile
  variant (13)..(13): Thr or Gln or Ser or Asn
  variant (14)..(14): Thr or Gln or Ser or Asn
  variant (15)..(15): Ala or Met or Val or Leu or Ile
  variant (16)..(16): Asp or Glu
  variant (17)..(17): Asp or Glu
  variant (18)..(18): Asp or Glu
  variant (19)..(19): Ala or Met or Val or Leu or Ile
  variant (20)..(20): Thr or Gln or Ser or Asn
  variant (21)..(21): Asp or Glu
  variant (22)..(22): Ala or Met or Val or Leu or Ile
XKKXXKKXXXXXXXXXXXXXXX

SEQ ID NO: 24 - protein, 22 aa, artificial
  antimicrobial peptide pattern
  variant (1)..(1): Ala or Met or Val or Leu or Ile
  variant (2)..(2): Asp or Glu
  variant (3)..(3): Asp or Glu
  variant (4)..(4): Ala or Met or Val or Leu or Ile
  variant (5)..(5): Ala or Met or Val or Leu or Ile
  variant (6)..(6): Asp or Glu
  variant (7)..(7): Asp or Glu
  variant (8)..(8): Ala or Met or Val or Leu or Ile
  variant (9)..(9): Trp or Phe
  variant (10)..(10): Thr or Gln or Ser or Asn
  variant (11)..(11): Trp or Phe
  variant (12)..(12): Ala or Met or Val or Leu or Ile
  variant (13)..(13): Thr or Gln or Ser or Asn
  variant (14)..(14): Thr or Gln or Ser or Asn
  variant (15)..(15): Ala or Met or Val or Leu or Ile
  variant (19)..(19): Ala or Met or Val or Leu or Ile
  variant (20)..(20): Thr or Gln or Ser or Asn
  variant (22)..(22): Ala or Met or Val or Leu or Ile
XXXXXXXXXXXXXXXKKKXXKX

SEQ ID NO: 25 - protein, 22 aa, artificial
  antimicrobial peptide pattern
  variant (1)..(1): Ala or Met or Val or Leu or Ile
  variant (4)..(4): Ala or Met or Val or Leu or Ile
  variant (5)..(5): Ala or Met or Val or Leu or Ile
  variant (8)..(8): Ala or Met or Val or Leu or Ile
  variant (9)..(9): Trp or Phe
  variant (10)..(10): Thr or Gln or Ser or Asn
  variant (11)..(11): Trp or Phe
  variant (12)..(12): Ala or Met or Val or Leu or Ile
  variant (13)..(13): Thr or Gln or Ser or Asn
  variant (14)..(14): Thr or Gln or Ser or Asn
  variant (15)..(15): Ala or Met or Val or Leu or Ile
  variant (16)..(16): Asp or Glu
  variant (17)..(17): Thr or Gln or Ser or Asn
  variant (18)..(18): Asp or Glu
  variant (19)..(19): Ala or Met or Val or Leu or Ile
  variant (20)..(20): Asp or Glu
  variant (21)..(21): Asp or Glu
  variant (22)..(22): Ala or Met or Val or Leu or Ile
XKKXXKKXXXXXXXXXXXXXXX

SEQ ID NO: 26 - protein, 22 aa, artificial
  antimicrobial peptide pattern
  variant (1)..(1): Ala or Met or Val or Leu or Ile
  variant (2)..(2): Asp or Glu
  variant (3)..(3): Asp or Glu
  variant (4)..(4): Ala or Met or Val or Leu or Ile
  variant (5)..(5): Ala or Met or Val or Leu or Ile
  variant (6)..(6): Asp or Glu
  variant (7)..(7): Asp or Glu
  variant (8)..(8): Ala or Met or Val or Leu or Ile
  variant (9)..(9): Trp or Phe
  variant (10)..(10): Thr or Gln or Ser or Asn
  variant (11)..(11): Trp or Phe
  variant (12)..(12): Ala or Met or Val or Leu or Ile
  variant (13)..(13): Thr or Gln or Ser or Asn
  variant (14)..(14): Thr or Gln or Ser or Asn
  variant (15)..(15): Ala or Met or Val or Leu or Ile
  variant (17)..(17): Thr or Gln or Ser or Asn
  variant (19)..(19): Ala or Met or Val or Leu or Ile
  variant (22)..(22): Ala or Met or Val or Leu or Ile
XXXXXXXXXXXXXXXKXKXKKX

SEQ ID NO: 27 - protein, 22 aa, artificial
  antimicrobial peptide pattern
  variant (1)..(1): Ala or Met or Val or Leu or Ile
  variant (4)..(4): Ala or Met or Val or Leu or Ile
  variant (5)..(5): Ala or Met or Val or Leu or Ile
  variant (8)..(8): Ala or Met or Val or Leu or Ile
  variant (9)..(9): Trp or Phe
  variant (10)..(10): Thr or Gln or Ser or Asn
  variant (11)..(11): Trp or Phe
  variant (12)..(12): Ala or Met or Val or Leu or Ile
  variant (13)..(13): Thr or Gln or Ser or Asn
  variant (14)..(14): Thr or Gln or Ser or Asn
  variant (15)..(15): Ala or Met or Val or Leu or Ile
  variant (16)..(16): Ala or Met or Val or Leu or Ile
  variant (17)..(17): Asp or Glu
  variant (18)..(18): Asp or Glu
  variant (19)..(19): Ala or Met or Val or Leu or Ile
  variant (20)..(20): Asp or Glu
  variant (21)..(21): Asp or Glu
  variant (22)..(22): Ala or Met or Val or Leu or Ile
XKKXXKKXXXXXXXXXXXXXXX

SEQ ID NO: 28 - protein, 22 aa, artificial
  antimicrobial peptide pattern
  variant (1)..(1): Ala or Met or Val or Leu or Ile
  variant (2)..(2): Asp or Glu
  variant (3)..(3): Asp or Glu
  variant (4)..(4): Ala or Met or Val or Leu or Ile
  variant (5)..(5): Ala or Met or Val or Leu or Ile
  variant (6)..(6): Asp or Glu
  variant (7)..(7): Asp or Glu
  variant (8)..(8): Ala or Met or Val or Leu or Ile
  variant (9)..(9): Trp or Phe
  variant (10)..(10): Thr or Gln or Ser or Asn
  variant (11)..(11): Trp or Phe
  variant (12)..(12): Ala or Met or Val or Leu or Ile
  variant (13)..(13): Thr or Gln or Ser or Asn
  variant (14)..(14): Thr or Gln or Ser or Asn
  variant (15)..(15): Ala or Met or Val or Leu or Ile
  variant (16)..(16): Ala or Met or Val or Leu or Ile
  variant (19)..(19): Ala or Met or Val or Leu or Ile
  variant (22)..(22): Ala or Met or Val or Leu or Ile
XXXXXXXXXXXXXXXXKKXKKX

SEQ ID NO: 29 - protein, 22 aa, artificial
  antimicrobial peptide pattern
  variant (1)..(1): Ala or Met or Val or Leu or Ile
  variant (2)..(2): Asp or Glu
  variant (3)..(3): Asp or Glu
  variant (4)..(4): Ala or Met or Val or Leu or Ile
  variant (5)..(5): Ala or Met or Val or Leu or Ile
  variant (6)..(6): Asp or Glu
  variant (7)..(7): Asp or Glu
  variant (8)..(8): Ala or Met or Val or Leu or Ile
  variant (9)..(9): Trp or Phe
  variant (10)..(10): Thr or Gln or Ser or Asn
  variant (11)..(11): Trp or Phe
  variant (12)..(12): Ala or Met or Val or Leu or Ile
  variant (14)..(14): Thr or Gln or Ser or Asn
  variant (15)..(15): Ala or Met or Val or Leu or Ile
  variant (19)..(19): Ala or Met or Val or Leu or Ile
  variant (22)..(22): Ala or Met or Val or Leu or Ile
XXXXXXXXXXXXKXXKKKXKKX

SEQ ID NO: 30 - protein, 22 aa, artificial
  antimicrobial peptide pattern
  variant (1)..(1): Ala or Met or Val or Leu or Ile
  variant (4)..(4): Trp or Phe
  variant (5)..(5): Trp or Phe
  variant (8)..(8): Ala or Met or Val or Leu or Ile
  variant (9)..(9): Ala or Met or Val or Leu or Ile
  variant (10)..(10): Thr or Gln or Ser or Asn
  variant (11)..(11): Ala or Met or Val or Leu or Ile
  variant (12)..(12): Ala or Met or Val or Leu or Ile
  variant (13)..(13): Asp or Glu
  variant (14)..(14): Thr or Gln or Ser or Asn
  variant (15)..(15): Ala or Met or Val or Leu or Ile
  variant (16)..(16): Trp or Phe
  variant (17)..(17): Asp or Glu
  variant (18)..(18): Asp or Glu
  variant (19)..(19): Ala or Met or Val or Leu or Ile
  variant (20)..(20): Thr or Gln or Ser or Asn
  variant (21)..(21): Asp or Glu
  variant (22)..(22): Trp or Phe
XKKXXKKXXXXXXXXXXXXXXX

SEQ ID NO: 31 - protein, 22 aa, artificial
  antimicrobial peptide pattern
  variant (1)..(1): Ala or Met or Val or Leu or Ile
  variant (2)..(2): Asp or Glu
  variant (3)..(3): Asp or Glu
  variant (4)..(4): Trp or Phe
  variant (5)..(5): Trp or Phe
  variant (6)..(6): Asp or Glu
  variant (7)..(7): Asp or Glu
  variant (8)..(8): Ala or Met or Val or Leu or Ile
  variant (9)..(9): Ala or Met or Val or Leu or Ile
  variant (10)..(10): Thr or Gln or Ser or Asn
  variant (11)..(11): Ala or Met or Val or Leu or Ile
  variant (12)..(12): Ala or Met or Val or Leu or Ile
  variant (14)..(14): Thr or Gln or Ser or Asn
  variant (15)..(15): Ala or Met or Val or Leu or Ile
  variant (16)..(16): Trp or Phe
  variant (19)..(19): Ala or Met or Val or Leu or Ile
  variant (20)..(20): Thr or Gln or Ser or Asn
  variant (22)..(22): Trp or Phe
XXXXXXXXXXXXKXXXKKXXKX

SEQ ID NO: 32 - protein, 22 aa, artificial
  antimicrobial peptide pattern
  variant (1)..(1): Ala or Met or Val or Leu or Ile
  variant (4)..(4): Trp or Phe
  variant (5)..(5): Trp or Phe
  variant (8)..(8): Ala or Met or Val or Leu or Ile
  variant (9)..(9): Ala or Met or Val or Leu or Ile
  variant (10)..(10): Thr or Gln or Ser or Asn
  variant (11)..(11): Ala or Met or Val or Leu or Ile
  variant (12)..(12): Ala or Met or Val or Leu or Ile
  variant (13)..(13): Asp or Glu
  variant (14)..(14): Thr or Gln or Ser or Asn
  variant (15)..(15): Ala or Met or Val or Leu or Ile
  variant (16)..(16): Trp or Phe
  variant (17)..(17): Thr or Gln or Ser or Asn
  variant (18)..(18): Asp or Glu
  variant (19)..(19): Ala or Met or Val or Leu or Ile
  variant (20)..(20): Asp or Glu
  variant (21)..(21): Asp or Glu
  variant (22)..(22): Trp or Phe
XKKXXKKXXXXXXXXXXXXXXX

SEQ ID NO: 33 - protein, 22 aa, artificial
  antimicrobial peptide pattern
  variant (1)..(1): Ala or Met or Val or Leu or Ile
  variant (2)..(2): Asp or Glu
  variant (3)..(3): Asp or Glu
  variant (4)..(4): Trp or Phe
  variant (5)..(5): Trp or Phe
  variant (6)..(6): Asp or Glu
  variant (7)..(7): Asp or Glu
  variant (8)..(8): Ala or Met or Val or Leu or Ile
  variant (9)..(9): Ala or Met or Val or Leu or Ile
  variant (10)..(10): Thr or Gln or Ser or Asn
  variant (11)..(11): Ala or Met or Val or Leu or Ile
  variant (12)..(12): Ala or Met or Val or Leu or Ile
  variant (14)..(14): Thr or Gln or Ser or Asn
  variant (15)..(15): Ala or Met or Val or Leu or Ile
  variant (16)..(16): Trp or Phe
  variant (17)..(17): Thr or Gln or Ser or Asn
  variant (19)..(19): Ala or Met or Val or Leu or Ile
  variant (22)..(22): Trp or Phe
XXXXXXXXXXXXKXXXXKXKKX

SEQ ID NO: 34 - protein, 22 aa, artificial
  antimicrobial peptide pattern
  variant (1)..(1): Ala or Met or Val or Leu or Ile
  variant (4)..(4): Trp or Phe
  variant (5)..(5): Trp or Phe
  variant (8)..(8): Ala or Met or Val or Leu or Ile
  variant (9)..(9): Ala or Met or Val or Leu or Ile
  variant (10)..(10): Thr or Gln or Ser or Asn
  variant (11)..(11): Ala or Met or Val or Leu or Ile
  variant (12)..(12): Ala or Met or Val or Leu or Ile
  variant (13)..(13): Thr or Gln or Ser or Asn
  variant (14)..(14): Thr or Gln or Ser or Asn
  variant (15)..(15): Ala or Met or Val or Leu or Ile
  variant (16)..(16): Trp or Phe
  variant (17)..(17): Asp or Glu
  variant (18)..(18): Asp or Glu
  variant (19)..(19): Ala or Met or Val or Leu or Ile
  variant (20)..(20): Asp or Glu
  variant (21)..(21): Asp or Glu
  variant (22)..(22): Trp or Phe
XKKXXKKXXXXXXXXXXXXXXX

SEQ ID NO: 35 - protein, 22 aa, artificial
  antimicrobial peptide pattern
  variant (1)..(1): Ala or Met or Val or Leu or Ile
  variant (2)..(2): Asp or Glu
  variant (3)..(3): Asp or Glu
  variant (4)..(4): Trp or Phe
  variant (5)..(5): Trp or Phe
  variant (6)..(6): Asp or Glu
  variant (7)..(7): Asp or Glu
  variant (8)..(8): Ala or Met or Val or Leu or Ile
  variant (9)..(9): Ala or Met or Val or Leu or Ile
  variant (10)..(10): Thr or Gln or Ser or Asn
  variant (11)..(11): Ala or Met or Val or Leu or Ile
  variant (12)..(12): Ala or Met or Val or Leu or Ile
  variant (13)..(13): Thr or Gln or Ser or Asn
  variant (14)..(14): Thr or Gln or Ser or Asn
  variant (15)..(15): Ala or Met or Val or Leu or Ile
  variant (16)..(16): Trp or Phe
  variant (19)..(19): Ala or Met or Val or Leu or Ile
  variant (22)..(22): Trp or Phe
XXXXXXXXXXXXXXXXKKXKKX

SEQ ID NO: 36 - protein, 22 aa, artificial
  antimicrobial peptide pattern
  variant (1)..(1): Ala or Met or Val or Leu or Ile
  variant (2)..(2): Asp or Glu
  variant (3)..(3): Asp or Glu
  variant (4)..(4): Trp or Phe
  variant (5)..(5): Trp or Phe
  variant (6)..(6): Asp or Glu
  variant (7)..(7): Asp or Glu
  variant (8)..(8): Ala or Met or Val or Leu or Ile
  variant (9)..(9): Ala or Met or Val or Leu or Ile
  variant (10)..(10): Thr or Gln or Ser or Asn
  variant (11)..(11): Ala or Met or Val or Leu or Ile
  variant (12)..(12): Ala or Met or Val or Leu or Ile
  variant (14)..(14): Thr or Gln or Ser or Asn
  variant (15)..(15): Ala or Met or Val or Leu or Ile
  variant (16)..(16): Trp or Phe
  variant (19)..(19): Ala or Met or Val or Leu or Ile
  variant (22)..(22): Trp or Phe
XXXXXXXXXXXXKXXXKKXKKX

SEQ ID NO: 37 - protein, 30 aa, artificial
  antimicrobial peptide pattern
  variant (5)..(5): Ala or Met or Val or Leu or Ile
  variant (8)..(8): Ala or Met or Val or Leu or Ile
  variant (9)..(9): Ala or Met or Val or Leu or Ile
  variant (12)..(12): Ala or Met or Val or Leu or Ile
  variant (13)..(13): Trp or Phe
  variant (14)..(14): Thr or Gln or Ser or Asn
  variant (15)..(15): Trp or Phe
  variant (16)..(16): Ala or Met or Val or Leu or Ile
  variant (17)..(17): Thr or Gln or Ser or Asn
  variant (18)..(18): Thr or Gln or Ser or Asn
  variant (19)..(19): Ala or Met or Val or Leu or Ile
  variant (20)..(20): Asp or Glu
  variant (21)..(21): Thr or Gln or Ser or Asn
  variant (22)..(22): Thr or Gln or Ser or Asn
  variant (23)..(23): Ala or Met or Val or Leu or Ile
  variant (24)..(24): Thr or Gln or Ser or Asn
  variant (25)..(25): Asp or Glu
  variant (26)..(26): Ala or Met or Val or Leu or Ile
  variant (28)..(28): Thr or Gln or Ser or Asn
  variant (29)..(29): Thr or Gln or Ser or Asn
KKKKXKKXXKKXXXXXXXXXXXXXXXKXXK

SEQ ID NO: 38 - protein, 30 aa, artificial
  antimicrobial peptide pattern
  variant (2)..(2): Thr or Gln or Ser or Asn
  variant (3)..(3): Thr or Gln or Ser or Asn
  variant (4)..(4): Thr or Gln or Ser or Asn
  variant (5)..(5): Ala or Met or Val or Leu or Ile
  variant (6)..(6): Asp or Glu
  variant (7)..(7): Asp or Glu
  variant (8)..(8): Ala or Met or Val or Leu or Ile
  variant (9)..(9): Ala or Met or Val or Leu or Ile
  variant (10)..(10): Thr or Gln or Ser or Asn
  variant (11)..(11): Thr or Gln or Ser or Asn
  variant (12)..(12): Ala or Met or Val or Leu or Ile
  variant (13)..(13): Trp or Phe
  variant (14)..(14): Thr or Gln or Ser or Asn
  variant (15)..(15): Trp or Phe
  variant (16)..(16): Ala or Met or Val or Leu or Ile
  variant (18)..(18): Thr or Gln or Ser or Asn
  variant (19)..(19): Ala or Met or Val or Leu or Ile
  variant (21)..(21): Thr or Gln or Ser or Asn
  variant (23)..(23): Ala or Met or Val or Leu or Ile
  variant (24)..(24): Thr or Gln or Ser or Asn
  variant (26)..(26): Ala or Met or Val or Leu or Ile
KXXXXXXXXXXXXXXXKXXKXKXXKXKKKK

SEQ ID NO: 39 - protein, 30 aa, artificial
  antimicrobial peptide pattern
  variant (5)..(5): Ala or Met or Val or Leu or Ile
  variant (8)..(8): Ala or Met or Val or Leu or Ile
  variant (9)..(9): Ala or Met or Val or Leu or Ile
  variant (12)..(12): Ala or Met or Val or Leu or Ile
  variant (13)..(13): Trp or Phe
  variant (14)..(14): Thr or Gln or Ser or Asn
  variant (15)..(15): Trp or Phe
  variant (16)..(16): Ala or Met or Val or Leu or Ile
  variant (17)..(17): Thr or Gln or Ser or Asn
  variant (18)..(18): Thr or Gln or Ser or Asn
  variant (19)..(19): Ala or Met or Val or Leu or Ile
  variant (20)..(20): Asp or Glu
  variant (21)..(21): Thr or Gln or Ser or Asn
  variant (22)..(22): Asp or Glu
  variant (23)..(23): Ala or Met or Val or Leu or Ile
  variant (24)..(24): Thr or Gln or Ser or Asn
  variant (25)..(25): Thr or Gln or Ser or Asn
  variant (26)..(26): Ala or Met or Val or Leu or Ile
KKKKXKKXXKKXXXXXXXXXXXXXXXKKKK

SEQ ID NO: 40 - protein, 30 aa, artificial
  antimicrobial peptide pattern
  variant (2)..(2): Thr or Gln or Ser or Asn
  variant (3)..(3): Thr or Gln or Ser or Asn
  variant (5)..(5): Ala or Met or Val or Leu or Ile
  variant (6)..(6): Asp or Glu
  variant (7)..(7): Thr or Gln or Ser or Asn
  variant (8)..(8): Ala or Met or Val or Leu or Ile
  variant (9)..(9): Ala or Met or Val or Leu or Ile
  variant (10)..(10): Thr or Gln or Ser or Asn
  variant (11)..(11): Asp or Glu
  variant (12)..(12): Ala or Met or Val or Leu or Ile
  variant (13)..(13): Trp or Phe
  variant (14)..(14): Thr or Gln or Ser or Asn
  variant (15)..(15): Trp or Phe
  variant (16)..(16): Ala or Met or Val or Leu or Ile
  variant (18)..(18): Thr or Gln or Ser or Asn
  variant (19)..(19): Ala or Met or Val or Leu or Ile
  variant (21)..(21): Thr or Gln or Ser or Asn
  variant (23)..(23): Ala or Met or Val or Leu or Ile
  variant (24)..(24): Thr or Gln or Ser or Asn
  variant (26)..(26): Ala or Met or Val or Leu or Ile
KXXKXXXXXXXXXXXXKXXKXKXXKXKKKK

SEQ ID NO: 41 - protein, 30 aa, artificial; identical to SEQ ID NO: 37
  antimicrobial peptide pattern
  variant (5)..(5): Ala or Met or Val or Leu or Ile
  variant (8)..(8): Ala or Met or Val or Leu or Ile
  variant (9)..(9): Ala or Met or Val or Leu or Ile
  variant (12)..(12): Ala or Met or Val or Leu or Ile
  variant (13)..(13): Trp or Phe
  variant (14)..(14): Thr or Gln or Ser or Asn
  variant (15)..(15): Trp or Phe
  variant (16)..(16): Ala or Met or Val or Leu or Ile
  variant (17)..(17): Asp or Glu
  variant (18)..(18): Thr or Gln or Ser or Asn
  variant (19)..(19): Ala or Met or Val or Leu or Ile
  variant (20)..(20): Ala or Met or Val or Leu or Ile
  variant (21)..(21): Thr or Gln or Ser or Asn
  variant (22)..(22): Thr or Gln or Ser or Asn
  variant (23)..(23): Ala or Met or Val or Leu or Ile
  variant (24)..(24): Thr or Gln or Ser or Asn
  variant (25)..(25): Asp or Glu
  variant (26)..(26): Ala or Met or Val or Leu or Ile
  variant (28)..(28): Thr or Gln or Ser or Asn
  variant (29)..(29): Thr or Gln or Ser or Asn

SEQ ID NO: 42 - protein, 30 aa, artificial
  antimicrobial peptide pattern
  variant (3)..(3): Thr or Gln or Ser or Asn
  variant (4)..(4): Thr or Gln or Ser or Asn
  variant (5)..(5): Ala or Met or Val or Leu or Ile
  variant (6)..(6): Thr or Gln or Ser or Asn
  variant (7)..(7): Asp or Glu
  variant (8)..(8): Ala or Met or Val or Leu or Ile
  variant (9)..(9): Ala or Met or Val or Leu or Ile
  variant (10)..(10): Asp or Glu
  variant (11)..(11): Thr or Gln or Ser or Asn
  variant (12)..(12): Ala or Met or Val or Leu or Ile
  variant (13)..(13): Trp or Phe
  variant (14)..(14): Thr or Gln or Ser or Asn
  variant (15)..(15): Trp or Phe
  variant (16)..(16): Ala or Met or Val or Leu or Ile
  variant (18)..(18): Thr or Gln or Ser or Asn
  variant (19)..(19): Ala or Met or Val or Leu or Ile
  variant (21)..(21): Thr or Gln or Ser or Asn
  variant (23)..(23): Ala or Met or Val or Leu or Ile
  variant (24)..(24): Thr or Gln or Ser or Asn
  variant (26)..(26): Ala or Met or Val or Leu or Ile
KKXXXXXXXXXXXXXXKXXKXKXXKXKKKK

SEQ ID NO: 43 - protein, 30 aa, artificial; identical to SEQ ID NO: 39
  antimicrobial peptide pattern
  variant (5)..(5): Ala or Met or Val or Leu or Ile
  variant (8)..(8): Ala or Met or Val or Leu or Ile
  variant (9)..(9): Ala or Met or Val or Leu or Ile
  variant (12)..(12): Ala or Met or Val or Leu or Ile
  variant (13)..(13): Trp or Phe
  variant (14)..(14): Thr or Gln or Ser or Asn
  variant (15)..(15): Trp or Phe
  variant (16)..(16): Ala or Met or Val or Leu or Ile
  variant (17)..(17): Asp or Glu
  variant (18)..(18): Thr or Gln or Ser or Asn
  variant (19)..(19): Ala or Met or Val or Leu or Ile
  variant (20)..(20): Ala or Met or Val or Leu or Ile
  variant (21)..(21): Thr or Gln or Ser or Asn
  variant (22)..(22): Asp or Glu
  variant (23)..(23): Ala or Met or Val or Leu or Ile
  variant (24)..(24): Thr or Gln or Ser or Asn
  variant (25)..(25): Thr or Gln or Ser or Asn
  variant (26)..(26): Ala or Met or Val or Leu or Ile

SEQ ID NO: 44 - protein, 30 aa, artificial
  antimicrobial peptide pattern
  variant (5)..(5): Ala or Met or Val or Leu or Ile
  variant (6)..(6): Thr or Gln or Ser or Asn
  variant (7)..(7): Thr or Gln or Ser or Asn
  variant (8)..(8): Ala or Met or Val or Leu or Ile
  variant (9)..(9): Ala or Met or Val or Leu or Ile
  variant (10)..(10): Asp or Glu
  variant (11)..(11): Asp or Glu
  variant (12)..(12): Ala or Met or Val or Leu or Ile
  variant (13)..(13): Trp or Phe
  variant (14)..(14): Thr or Gln or Ser or Asn
  variant (15)..(15): Trp or Phe
  variant (16)..(16): Ala or Met or Val or Leu or Ile
  variant (18)..(18): Thr or Gln or Ser or Asn
  variant (19)..(19): Ala or Met or Val or Leu or Ile
  variant (21)..(21): Thr or Gln or Ser or Asn
  variant (23)..(23): Ala or Met or Val or Leu or Ile
  variant (24)..(24): Thr or Gln or Ser or Asn
  variant (26)..(26): Ala or Met or Val or Leu or Ile
KKKKXXXXXXXXXXXXKXXKXKXXKXKKKK

SEQ ID NO: 45 - protein, 30 aa, artificial
  antimicrobial peptide pattern
  variant (5)..(5): Ala or Met or Val or Leu or Ile
  variant (8)..(8): Trp or Phe
  variant (9)..(9): Trp or Phe
  variant (12)..(12): Ala or Met or Val or Leu or Ile
  variant (13)..(13): Ala or Met or Val or Leu or Ile
  variant (14)..(14): Thr or Gln or Ser or Asn
  variant (15)..(15): Ala or Met or Val or Leu or Ile
  variant (16)..(16): Ala or Met or Val or Leu or Ile
  variant (17)..(17): Thr or Gln or Ser or Asn
  variant (18)..(18): Thr or Gln or Ser or Asn
  variant (19)..(19): Ala or Met or Val or Leu or Ile
  variant (20)..(20): Trp or Phe
  variant (21)..(21): Thr or Gln or Ser or Asn
  variant (22)..(22): Thr or Gln or Ser or Asn
  variant (23)..(23): Ala or Met or Val or Leu or Ile
  variant (24)..(24): Asp or Glu
  variant (25)..(25): Asp or Glu
  variant (26)..(26): Trp or Phe
  variant (27)..(27): Thr or Gln or Ser or Asn
  variant (28)..(28): Thr or Gln or Ser or Asn
  variant (29)..(29): Thr or Gln or Ser or Asn
KKKKXKKXXKKXXXXXXXXXXXXXXXXXXK

SEQ ID NO: 46 - protein, 30 aa, artificial
  antimicrobial peptide pattern
  variant (2)..(2): Thr or Gln or Ser or Asn
  variant (3)..(3): Thr or Gln or Ser or Asn
  variant (4)..(4): Thr or Gln or Ser or Asn
  variant (5)..(5): Ala or Met or Val or Leu or Ile
  variant (6)..(6): Asp or Glu
  variant (7)..(7): Asp or Glu
  variant (8)..(8): Trp or Phe
  variant (9)..(9): Trp or Phe
  variant (10)..(10): Thr or Gln or Ser or Asn
  variant (11)..(11): Thr or Gln or Ser or Asn
  variant (12)..(12): Ala or Met or Val or Leu or Ile
  variant (13)..(13): Ala or Met or Val or Leu or Ile
  variant (14)..(14): Thr or Gln or Ser or Asn
  variant (15)..(15): Ala or Met or Val or Leu or Ile
  variant (16)..(16): Ala or Met or Val or Leu or Ile
  variant (18)..(18): Thr or Gln or Ser or Asn
  variant (19)..(19): Ala or Met or Val or Leu or Ile
  variant (20)..(20): Trp or Phe
  variant (21)..(21): Thr or Gln or Ser or Asn
  variant (23)..(23): Ala or Met or Val or Leu or Ile
  variant (26)..(26): Trp or Phe
KXXXXXXXXXXXXXXXKXXXXKXKKXKKKK

SEQ ID NO: 47 - protein, 30 aa, artificial
  antimicrobial peptide pattern
  variant (5)..(5): Ala or Met or Val or Leu or Ile
  variant (8)..(8): Trp or Phe
  variant (9)..(9): Trp or Phe
  variant (12)..(12): Ala or Met or Val or Leu or Ile
  variant (13)..(13): Ala or Met or Val or Leu or Ile
  variant (14)..(14): Thr or Gln or Ser or Asn
  variant (15)..(15): Ala or Met or Val or Leu or Ile
  variant (16)..(16): Ala or Met or Val or Leu or Ile
  variant (17)..(17): Thr or Gln or Ser or Asn
  variant (18)..(18): Thr or Gln or Ser or Asn
  variant (19)..(19): Ala or Met or Val or Leu or Ile
  variant (20)..(20): Trp or Phe
  variant (21)..(21): Thr or Gln or Ser or Asn
  variant (22)..(22): Asp or Glu
  variant (23)..(23): Ala or Met or Val or Leu or Ile
  variant (24)..(24): Asp or Glu
  variant (25)..(25): Thr or Gln or Ser or Asn
  variant (26)..(26): Trp or Phe
  variant (27)..(27): Thr or Gln or Ser or Asn
KKKKXKKXXKKXXXXXXXXXXXXXXXXKKK

SEQ ID NO: 48 - protein, 30 aa, artificial
  antimicrobial peptide pattern
  variant (2)..(2): Thr or Gln or Ser or Asn
  variant (3)..(3): Thr or Gln or Ser or Asn
  variant (5)..(5): Ala or Met or Val or Leu or Ile
  variant (6)..(6): Asp or Glu
  variant (7)..(7): Thr or Gln or Ser or Asn
  variant (8)..(8): Trp or Phe
  variant (9)..(9): Trp or Phe
  variant (10)..(10): Thr or Gln or Ser or Asn
  variant (11)..(11): Asp or Glu
  variant (12)..(12): Ala or Met or Val or Leu or Ile
  variant (13)..(13): Ala or Met or Val or Leu or Ile
  variant (14)..(14): Thr or Gln or Ser or Asn
  variant (15)..(15): Ala or Met or Val or Leu or Ile
  variant (16)..(16): Ala or Met or Val or Leu or Ile
  variant (18)..(18): Thr or Gln or Ser or Asn
  variant (19)..(19): Ala or Met or Val or Leu or Ile
  variant (20)..(20): Trp or Phe
  variant (21)..(21): Thr or Gln or Ser or Asn
  variant (23)..(23): Ala or Met or Val or Leu or Ile
  variant (26)..(26): Trp or Phe
KXXKXXXXXXXXXXXXKXXXXKXKKXKKKK

SEQ ID NO: 49 - protein, 30 aa, artificial; identical to SEQ ID NO: 37
  antimicrobial peptide pattern
  variant (5)..(5): Ala or Met or Val or Leu or Ile
  variant (8)..(8): Trp or Phe
  variant (9)..(9): Trp or Phe
  variant (12)..(12): Ala or Met or Val or Leu or Ile
  variant (13)..(13): Ala or Met or Val or Leu or Ile
  variant (14)..(14): Thr or Gln or Ser or Asn
  variant (15)..(15): Ala or Met or Val or Leu or Ile
  variant (16)..(16): Ala or Met or Val or Leu or Ile
  variant (17)..(17): Asp or Glu
  variant (18)..(18): Thr or Gln or Ser or Asn
  variant (19)..(19): Ala or Met or Val or Leu or Ile
  variant (20)..(20): Trp or Phe
  variant (21)..(21): Thr or Gln or Ser or Asn
  variant (22)..(22): Thr or Gln or Ser or Asn
  variant (23)..(23): Ala or Met or Val or Leu or Ile
  variant (24)..(24): Thr or Gln or Ser or Asn
  variant (25)..(25): Asp or Glu
  variant (26)..(26): Trp or Phe
  variant (28)..(28): Thr or Gln or Ser or Asn
  variant (29)..(29): Thr or Gln or Ser or Asn

SEQ ID NO: 50 - protein, 30 aa, artificial
  antimicrobial peptide pattern
  variant (3)..(3): Thr or Gln or Ser or Asn
  variant (4)..(4): Thr or Gln or Ser or Asn
  variant (5)..(5): Ala or Met or Val or Leu or Ile
  variant (6)..(6): Thr or Gln or Ser or Asn
  variant (7)..(7): Asp or Glu
  variant (8)..(8): Trp or Phe
  variant (9)..(9): Trp or Phe
  variant (10)..(10): Asp or Glu
  variant (11)..(11): Thr or Gln or Ser or Asn
  variant (12)..(12): Ala or Met or Val or Leu or Ile
  variant (13)..(13): Ala or Met or Val or Leu or Ile
  variant (14)..(14): Thr or Gln or Ser or Asn
  variant (15)..(15): Ala or Met or Val or Leu or Ile
  variant (16)..(16): Ala or Met or Val or Leu or Ile
  variant (18)..(18): Thr or Gln or Ser or Asn
  variant (19)..(19): Ala or Met or Val or Leu or Ile
  variant (20)..(20): Trp or Phe
  variant (21)..(21): Thr or Gln or Ser or Asn
  variant (23)..(23): Ala or Met or Val or Leu or Ile
  variant (26)..(26): Trp or Phe
KKXXXXXXXXXXXXXXKXXXXKXKKXKKKK

SEQ ID NO: 51 - protein, 30 aa, artificial; identical to SEQ ID NO: 39
  antimicrobial peptide pattern
  variant (5)..(5): Ala or Met or Val or Leu or Ile
  variant (8)..(8): Trp or Phe
  variant (9)..(9): Trp or Phe
  variant (12)..(12): Ala or Met or Val or Leu or Ile
  variant (13)..(13): Ala or Met or Val or Leu or Ile
  variant (14)..(14): Thr or Gln or Ser or Asn
  variant (15)..(15): Ala or Met or Val or Leu or Ile
  variant (16)..(16): Ala or Met or Val or Leu or Ile
  variant (17)..(17): Asp or Glu
  variant (18)..(18): Thr or Gln or Ser or Asn
  variant (19)..(19): Ala or Met or Val or Leu or Ile
  variant (20)..(20): Trp or Phe
  variant (21)..(21): Thr or Gln or Ser or Asn
  variant (22)..(22): Asp or Glu
  variant (23)..(23): Ala or Met or Val or Leu or Ile
  variant (24)..(24): Thr or Gln or Ser or Asn
  variant (25)..(25): Thr or Gln or Ser or Asn
  variant (26)..(26): Trp or Phe

SEQ ID NO: 52 - protein, 30 aa, artificial
  antimicrobial peptide pattern
  variant (5)..(5): Ala or Met or Val or Leu or Ile
  variant (6)..(6): Thr or Gln or Ser or Asn
  variant (7)..(7): Thr or Gln or Ser or Asn
  variant (8)..(8): Trp or Phe
  variant (9)..(9): Trp or Phe
  variant (10)..(10): Asp or Glu
  variant (11)..(11): Asp or Glu
  variant (12)..(12): Ala or Met or Val or Leu or Ile
  variant (13)..(13): Ala or Met or Val or Leu or Ile
  variant (14)..(14): Thr or Gln or Ser or Asn
  variant (15)..(15): Ala or Met or Val or Leu or Ile
  variant (16)..(16): Ala or Met or Val or Leu or Ile
  variant (18)..(18): Thr or Gln or Ser or Asn
  variant (19)..(19): Ala or Met or Val or Leu or Ile
  variant (20)..(20): Trp or Phe
  variant (21)..(21): Thr or Gln or Ser or Asn
  variant (23)..(23): Ala or Met or Val or Leu or Ile
  variant (26)..(26): Trp or Phe
KKKKXXXXXXXXXXXXKXXXXKXKKXKKKK

SEQ ID NO: 53 - protein, 30 aa, artificial; identical to SEQ ID NO: 39
  antimicrobial peptide pattern
  variant (5)..(5): Ala or Met or Val or Leu or Ile
  variant (8)..(8): Ala or Met or Val or Leu or Ile
  variant (9)..(9): Ala or Met or Val or Leu or Ile
  variant (12)..(12): Ala or Met or Val or Leu or Ile
  variant (13)..(13): Trp or Phe
  variant (14)..(14): Thr or Gln or Ser or Asn
  variant (15)..(15): Trp or Phe
  variant (16)..(16): Ala or Met or Val or Leu or Ile
  variant (17)..(17): Asp or Glu
  variant (18)..(18): Thr or Gln or Ser or Asn
  variant (19)..(19): Ala or Met or Val or Leu or Ile
  variant (20)..(20): Asp or Glu
  variant (21)..(21): Thr or Gln or Ser or Asn
  variant (22)..(22): Asp or Glu
  variant (23)..(23): Ala or Met or Val or Leu or Ile
  variant (24)..(24): Thr or Gln or Ser or Asn
  variant (25)..(25): Asp or Glu
  variant (26)..(26): Ala or Met or Val or Leu or Ile

SEQ ID NO: 54 - protein, 30 aa, artificial; identical to SEQ ID NO: 44
  antimicrobial peptide pattern
  variant (5)..(5): Ala or Met or Val or Leu or Ile
  variant (6)..(6): Asp or Glu
  variant (7)..(7): Asp or Glu
  variant (8)..(8): Ala or Met or Val or Leu or Ile
  variant (9)..(9): Ala or Met or Val or Leu or Ile
  variant (10)..(10): Asp or Glu
  variant (11)..(11): Asp or Glu
  variant (12)..(12): Ala or Met or Val or Leu or Ile
  variant (13)..(13): Trp or Phe
  variant (14)..(14): Thr or Gln or Ser or Asn
  variant (15)..(15): Trp or Phe
  variant (16)..(16): Ala or Met or Val or Leu or Ile
  variant (18)..(18): Thr or Gln or Ser or Asn
  variant (19)..(19): Ala or Met or Val or Leu or Ile
  variant (21)..(21): Thr or Gln or Ser or Asn
  variant (23)..(23): Ala or Met or Val or Leu or Ile
  variant (24)..(24): Thr or Gln or Ser or Asn
  variant (26)..(26): Ala or Met or Val or Leu or Ile

SEQ ID NO: 55 - protein, 30 aa, artificial; identical to SEQ ID NO: 39
  antimicrobial peptide pattern
  variant (5)..(5): Ala or Met or Val or Leu or Ile
  variant (8)..(8): Ala or Met or Val or Leu or Ile
  variant (9)..(9): Ala or Met or Val or Leu or Ile
  variant (12)..(12): Ala or Met or Val or Leu or Ile
  variant (13)..(13): Trp or Phe
  variant (14)..(14): Thr or Gln or Ser or Asn
  variant (15)..(15): Trp or Phe
  variant (16)..(16): Ala or Met or Val or Leu or Ile
  variant (17)..(17): Asp or Glu
  variant (18)..(18): Thr or Gln or Ser or Asn
  variant (19)..(19): Ala or Met or Val or Leu or Ile
  variant (20)..(20): Ala or Met or Val or Leu or Ile
  variant (21)..(21): Asp or Glu
  variant (22)..(22): Asp or Glu
  variant (23)..(23): Ala or Met or Val or Leu or Ile
  variant (24)..(24): Thr or Gln or Ser or Asn
  variant (25)..(25): Asp or Glu
  variant (26)..(26): Ala or Met or Val or Leu or Ile

SEQ ID NO: 56 - protein, 30 aa, artificial
  antimicrobial peptide pattern
  variant (5)..(5): Ala or Met or Val or Leu or Ile
  variant (6)..(6): Asp or Glu
  variant (7)..(7): Asp or Glu
  variant (8)..(8): Ala or Met or Val or Leu or Ile
  variant (9)..(9): Ala or Met or Val or Leu or Ile
  variant (10)..(10): Asp or Glu
  variant (11)..(11): Asp or Glu
  variant (12)..(12): Ala or Met or Val or Leu or Ile
  variant (13)..(13): Trp or Phe
  variant (14)..(14): Thr or Gln or Ser or Asn
  variant (15)..(15): Trp or Phe
  variant (16)..(16): Ala or Met or Val or Leu or Ile
  variant (18)..(18): Thr or Gln or Ser or Asn
  variant (19)..(19): Ala or Met or Val or Leu or Ile
  variant (20)..(20): Ala or Met or Val or Leu or Ile
  variant (23)..(23): Ala or Met or Val or Leu or Ile
  variant (24)..(24): Thr or Gln or Ser or Asn
  variant (26)..(26): Ala or Met or Val or Leu or Ile
KKKKXXXXXXXXXXXXKXXXKKXXKXKKKK

SEQ ID NO: 57 - protein, 30 aa, artificial; identical to SEQ ID NO: 39
  antimicrobial peptide pattern
  variant (5)..(5): Ala or Met or Val or Leu or Ile
  variant (8)..(8): Ala or Met or Val or Leu or Ile
  variant (9)..(9): Ala or Met or Val or Leu or Ile
  variant (12)..(12): Ala or Met or Val or Leu or Ile
  variant (13)..(13): Trp or Phe
  variant (14)..(14): Thr or Gln or Ser or Asn
  variant (15)..(15): Trp or Phe
  variant (16)..(16): Ala or Met or Val or Leu or Ile
  variant (17)..(17): Asp or Glu
  variant (18)..(18): Thr or Gln or Ser or Asn
  variant (19)..(19): Ala or Met or Val or Leu or Ile
  variant (20)..(20): Ala or Met or Val or Leu or Ile
  variant (21)..(21): Thr or Gln or Ser or Asn
  variant (22)..(22): Asp or Glu
  variant (23)..(23): Ala or Met or Val or Leu or Ile
  variant (24)..(24): Asp or Glu
  variant (25)..(25): Asp or Glu
  variant (26)..(26): Ala or Met or Val or Leu or Ile

SEQ ID NO: 58 - protein, 30 aa, artificial; identical to SEQ ID NO: 52
  antimicrobial peptide pattern
  variant (5)..(5): Ala or Met or Val or Leu or Ile
  variant (6)..(6): Asp or Glu
  variant (7)..(7): Asp or Glu
  variant (8)..(8): Ala or Met or Val or Leu or Ile
  variant (9)..(9): Ala or Met or Val or Leu or Ile
  variant (10)..(10): Asp or Glu
  variant (11)..(11): Asp or Glu
  variant (12)..(12): Ala or Met or Val or Leu or Ile
  variant (13)..(13): Trp or Phe
  variant (14)..(14): Thr or Gln or Ser or Asn
  variant (15)..(15): Trp or Phe
  variant (16)..(16): Ala or Met or Val or Leu or Ile
  variant (18)..(18): Thr or Gln or Ser or Asn
  variant (19)..(19): Ala or Met or Val or Leu or Ile
  variant (20)..(20): Ala or Met or Val or Leu or Ile
  variant (21)..(21): Thr or Gln or Ser or Asn
  variant (23)..(23): Ala or Met or Val or Leu or Ile
  variant (26)..(26): Ala or Met or Val or Leu or Ile

SEQ ID NO: 59 - protein, 30 aa, artificial; identical to SEQ ID NO: 39
  antimicrobial peptide pattern
  variant (5)..(5): Ala or Met or Val or Leu or Ile
  variant (8)..(8): Ala or Met or Val or Leu or Ile
  variant (9)..(9): Ala or Met or Val or Leu or Ile
  variant (12)..(12): Ala or Met or Val or Leu or Ile
  variant (13)..(13): Trp or Phe
  variant (14)..(14): Thr or Gln or Ser or Asn
  variant (15)..(15): Trp or Phe
  variant (16)..(16): Ala or Met or Val or Leu or Ile
  variant (17)..(17): Thr or Gln or Ser or Asn
  variant (18)..(18): Thr or Gln or Ser or Asn
  variant (19)..(19): Ala or Met or Val or Leu or Ile
  variant (20)..(20): Asp or Glu
  variant (21)..(21): Asp or Glu
  variant (22)..(22): Asp or Glu
  variant (23)..(23): Ala or Met or Val or Leu or Ile
  variant (24)..(24): Thr or Gln or Ser or Asn
  variant (25)..(25): Asp or Glu
  variant (26)..(26): Ala or Met or Val or Leu or Ile

SEQ ID NO: 60 - protein, 30 aa, artificial
  antimicrobial peptide pattern
  variant (5)..(5): Ala or Met or Val or Leu or Ile
  variant (6)..(6): Asp or Glu
  variant (7)..(7): Asp or Glu
  variant (8)..(8): Ala or Met or Val or Leu or Ile
  variant (9)..(9): Ala or Met or Val or Leu or Ile
  variant (10)..(10): Asp or Glu
  variant (11)..(11): Asp or Glu
  variant (12)..(12): Ala or Met or Val or Leu or Ile
  variant (13)..(13): Trp or Phe
  variant (14)..(14): Thr or Gln or Ser or Asn
  variant (15)..(15): Trp or Phe
  variant (16)..(16): Ala or Met or Val or Leu or Ile
  variant (17)..(17): Thr or Gln or Ser or Asn
  variant (18)..(18): Thr or Gln or Ser or Asn
  variant (19)..(19): Ala or Met or Val or Leu or Ile
  variant (23)..(23): Ala or Met or Val or Leu or Ile
  variant (24)..(24): Thr or Gln or Ser or Asn
  variant (26)..(26): Ala or Met or Val or Leu or Ile
KKKKXXXXXXXXXXXXXXXKKKXXKXKKKK

SEQ ID NO: 61 - protein, 30 aa, artificial; identical to SEQ ID NO: 39
  antimicrobial peptide pattern
  variant (5)..(5): Ala or Met or Val or Leu or Ile
  variant (8)..(8): Ala or Met or Val or Leu or Ile
  variant (9)..(9): Ala or Met or Val or Leu or Ile
  variant (12)..(12): Ala or Met or Val or Leu or Ile
  variant (13)..(13): Trp or Phe
  variant (14)..(14): Thr or Gln or Ser or Asn
  variant (15)..(15): Trp or Phe
  variant (16)..(16): Ala or Met or Val or Leu or Ile
  variant (17)..(17): Thr or Gln or Ser or Asn
  variant (18)..(18): Thr or Gln or Ser or Asn
  variant (19)..(19): Ala or Met or Val or Leu or Ile
  variant (20)..(20): Asp or Glu
  variant (21)..(21): Thr or Gln or Ser or Asn
  variant (22)..(22): Asp or Glu
  variant (23)..(23): Ala or Met or Val or Leu or Ile
  variant (24)..(24): Asp or Glu
  variant (25)..(25): Asp or Glu
  variant (26)..(26): Ala or Met or Val or Leu or Ile

SEQ ID NO: 62 - protein, 30 aa, artificial
  antimicrobial peptide pattern
  variant (5)..(5): Ala or Met or Val or Leu or Ile
  variant (6)..(6): Asp or Glu
  variant (7)..(7): Asp or Glu
  variant (8)..(8): Ala or Met or Val or Leu or Ile
  variant (9)..(9): Ala or Met or Val or Leu or Ile
  variant (10)..(10): Asp or Glu
  variant (11)..(11): Asp or Glu
  variant (12)..(12): Ala or Met or Val or Leu or Ile
  variant (13)..(13): Trp or Phe
  variant (14)..(14): Thr or Gln or Ser or Asn
  variant (15)..(15): Trp or Phe
  variant (16)..(16): Ala or Met or Val or Leu or Ile
  variant (17)..(17): Thr or Gln or Ser or Asn
  variant (18)..(18): Thr or Gln or Ser or Asn
  variant (19)..(19): Ala or Met or Val or Leu or Ile
  variant (21)..(21): Thr or Gln or Ser or Asn
  variant (23)..(23): Ala or Met or Val or Leu or Ile
  variant (26)..(26): Ala or Met or Val or Leu or Ile
KKKKXXXXXXXXXXXXXXXKXKXKKXKKKK

SEQ ID NO: 63 - protein, 30 aa, artificial; identical to SEQ ID NO: 39
  antimicrobial peptide pattern
  variant (5)..(5): Ala or Met or Val or Leu or Ile
  variant (8)..(8): Ala or Met or Val or Leu or Ile
  variant (9)..(9): Ala or Met or Val or Leu or Ile
  variant (12)..(12): Ala or Met or Val or Leu or Ile
  variant (13)..(13): Trp or Phe
  variant (14)..(14): Thr or Gln or Ser or Asn
  variant (15)..(15): Trp or Phe
  variant (16)..(16): Ala or Met or Val or Leu or Ile
  variant (17)..(17): Thr or Gln or Ser or Asn
  variant (18)..(18): Thr or Gln or Ser or Asn
  variant (19)..(19): Ala or Met or Val or Leu or Ile
  variant (20)..(20): Ala or Met or Val or Leu or Ile
  variant (21)..(21): Asp or Glu
  variant (22)..(22): Asp or Glu
  variant (23)..(23): Ala or Met or Val or Leu or Ile
  variant (24)..(24): Asp or Glu
  variant (25)..(25): Asp or Glu
  variant (26)..(26): Ala or Met or Val or Leu or Ile

SEQ ID NO: 64 - protein, 30 aa, artificial
  antimicrobial peptide pattern
  variant (5)..(5): Ala or Met or Val or Leu or Ile
  variant (6)..(6): Asp or Glu
  variant (7)..(7): Asp or Glu
  variant (8)..(8): Ala or Met or Val or Leu or Ile
  variant (9)..(9): Ala or Met or Val or Leu or Ile
  variant (10)..(10): Asp or Glu
  variant (11)..(11): Asp or Glu
  variant (12)..(12): Ala or Met or Val or Leu or Ile
  variant (13)..(13): Trp or Phe
  variant (14)..(14): Thr or Gln or Ser or Asn
  variant (15)..(15): Trp or Phe
  variant (16)..(16): Ala or Met or Val or Leu or Ile
  variant (17)..(17): Thr or Gln or Ser or Asn
  variant (18)..(18): Thr or Gln or Ser or Asn
  variant (19)..(19): Ala or Met or Val or Leu or Ile
  variant (20)..(20): Ala or Met or Val or Leu or Ile
  variant (23)..(23): Ala or Met or Val or Leu or Ile
  variant (26)..(26): Ala or Met or Val or Leu or Ile
KKKKXXXXXXXXXXXXXXXXKKXKKXKKKK

SEQ ID NO: 65 - protein, 30 aa, artificial
  antimicrobial peptide pattern
  variant (5)..(5): Ala or Met or Val or Leu or Ile
  variant (6)..(6): Asp or Glu
  variant (7)..(7): Asp or Glu
  variant (8)..(8): Ala or Met or Val or Leu or Ile
  variant (9)..(9): Ala or Met or Val or Leu or Ile
  variant (10)..(10): Asp or Glu
  variant (11)..(11): Asp or Glu
  variant (12)..(12): Ala or Met or Val or Leu or Ile
  variant (13)..(13): Trp or Phe
  variant (14)..(14): Thr or Gln or Ser or Asn
  variant (15)..(15): Trp or Phe
  variant (16)..(16): Ala or Met or Val or Leu or Ile
  variant (18)..(18): Thr or Gln or Ser or Asn
  variant (19)..(19): Ala or Met or Val or Leu or Ile
  variant (23)..(23): Ala or Met or Val or Leu or Ile
  variant (26)..(26): Ala or Met or Val or Leu or Ile
KKKKXXXXXXXXXXXXKXXKKKXKKXKKKK

SEQ ID NO: 66 - protein, 30 aa, artificial; identical to SEQ ID NO: 39
  antimicrobial peptide pattern
  variant (5)..(5): Ala or Met or Val or Leu or Ile
  variant (8)..(8): Trp or Phe
  variant (9)..(9): Trp or Phe
  variant (12)..(12): Ala or Met or Val or Leu or Ile
  variant (13)..(13): Ala or Met or Val or Leu or Ile
  variant (14)..(14): Thr or Gln or Ser or Asn
  variant (15)..(15): Ala or Met or Val or Leu or Ile
  variant (16)..(16): Ala or Met or Val or Leu or Ile
  variant (17)..(17): Asp or Glu
  variant (18)..(18): Thr or Gln or Ser or Asn
  variant (19)..(19): Ala or Met or Val or Leu or Ile
  variant (20)..(20): Trp or Phe
  variant (21)..(21): Asp or Glu
  variant (22)..(22): Asp or Glu
  variant (23)..(23): Ala or Met or Val or Leu or Ile
  variant (24)..(24): Thr or Gln or Ser or Asn
  variant (25)..(25): Asp or Glu
  variant (26)..(26): Trp or Phe

SEQ ID NO: 67 - protein, 30 aa, artificial; identical to SEQ ID NO: 56
  antimicrobial peptide pattern
  variant (5)..(5): Ala or Met or Val or Leu or Ile
  variant (6)..(6): Asp or Glu
  variant (7)..(7): Asp or Glu
  variant (8)..(8): Trp or Phe
  variant (9)..(9): Trp or Phe
  variant (10)..(10): Asp or Glu
  variant (11)..(11): Asp or Glu
  variant (12)..(12): Ala or Met or Val or Leu or Ile
  variant (13)..(13): Ala or Met or Val or Leu or Ile
  variant (14)..(14): Thr or Gln or Ser or Asn
  variant (15)..(15): Ala or Met or Val or Leu or Ile
  variant (16)..(16): Ala or Met or Val or Leu or Ile
  variant (18)..(18): Thr or Gln or Ser or Asn
  variant (19)..(19): Ala or Met or Val or Leu or Ile
  variant (20)..(20): Trp or Phe
  variant (23)..(23): Ala or Met or Val or Leu or Ile
  variant (24)..(24): Thr or Gln or Ser or Asn
  variant (26)..(26): Trp or Phe

SEQ ID NO: 68 - protein, 30 aa, artificial; identical to SEQ ID NO: 39
  antimicrobial peptide pattern
  variant (5)..(5): Ala or Met or Val or Leu or Ile
  variant (8)..(8): Trp or Phe
  variant (9)..(9): Trp or Phe
  variant (12)..(12): Ala or Met or Val or Leu or Ile
  variant (13)..(13): Ala or Met or Val or Leu or Ile
  variant (14)..(14): Thr or Gln or Ser or Asn
  variant (15)..(15): Ala or Met or Val or Leu or Ile
  variant (16)..(16): Ala or Met or Val or Leu or Ile
  variant (17)..(17): Asp or Glu
  variant (18)..(18): Thr or Gln or Ser or Asn
  variant (19)..(19): Ala or Met or Val or Leu or Ile
  variant (20)..(20): Trp or Phe
  variant (21)..(21): Thr or Gln or Ser or Asn
  variant (22)..(22): Asp or Glu
  variant (23)..(23): Ala or Met or Val or Leu or Ile
  variant (24)..(24): Asp or Glu
  variant (25)..(25): Asp or Glu
  variant (26)..(26): Trp or Phe

SEQ ID NO: 69 - protein, 30 aa, artificial; identical to SEQ ID NO: 52
  antimicrobial peptide pattern
  variant (5)..(5): Ala or Met or Val or Leu or Ile
  variant (6)..(6): Asp or Glu
  variant (7)..(7): Asp or Glu
  variant (8)..(8): Trp or Phe
  variant (9)..(9): Trp or Phe
  variant (10)..(10): Asp or Glu
  variant (11)..(11): Asp or Glu
  variant (12)..(12): Ala or Met or Val or Leu or Ile
  variant (13)..(13): Ala or Met or Val or Leu or Ile
  variant (14)..(14): Thr or Gln or Ser or Asn
  variant (15)..(15): Ala or Met or Val or Leu or Ile
  variant (16)..(16): Ala or Met or Val or Leu or Ile
  variant (18)..(18): Thr or Gln or Ser or Asn
  variant (19)..(19): Ala or Met or Val or Leu or Ile
  variant (20)..(20): Trp or Phe
  variant (21)..(21): Thr or Gln or Ser or Asn
  variant (23)..(23): Ala or Met or Val or Leu or Ile
  variant (26)..(26): Trp or Phe

SEQ ID NO: 70 - protein, 30 aa, artificial; identical to SEQ ID NO: 39
  antimicrobial peptide pattern
  variant (5)..(5): Ala or Met or Val or Leu or Ile
  variant (8)..(8): Trp or Phe
  variant (9)..(9): Trp or Phe
  variant (12)..(12): Ala or Met or Val or Leu or Ile
  variant (13)..(13): Ala or Met or Val or Leu or Ile
  variant (14)..(14): Thr or Gln or Ser or Asn
  variant (15)..(15): Ala or Met or Val or Leu or Ile
  variant (16)..(16): Ala or Met or Val or Leu or Ile
  variant (17)..(17): Thr or Gln or Ser or Asn
  variant (18)..(18): Thr or Gln or Ser or Asn
  variant (19)..(19): Ala or Met or Val or Leu or Ile
  variant (20)..(20): Trp or Phe
  variant (21)..(21): Asp or Glu
  variant (22)..(22): Asp or Glu
  variant (23)..(23): Ala or Met or Val or Leu or Ile
  variant (24)..(24): Asp or Glu
  variant (25)..(25): Asp or Glu
  variant (26)..(26): Trp or Phe

SEQ ID NO: 71 - protein, 30 aa, artificial; identical to SEQ ID NO: 64
  antimicrobial peptide pattern
  variant (5)..(5): Ala or Met or Val or Leu or Ile
  variant (6)..(6): Asp or Glu
  variant (7)..(7): Asp or Glu
  variant (8)..(8): Trp or Phe
  variant (9)..(9): Trp or Phe
  variant (10)..(10): Asp or Glu
  variant (11)..(11): Asp or Glu
  variant (12)..(12): Ala or Met or Val or Leu or Ile
  variant (13)..(13): Ala or Met or Val or Leu or Ile
  variant (14)..(14): Thr or Gln or Ser or Asn
  variant (15)..(15): Ala or Met or Val or Leu or Ile
  variant (16)..(16): Ala or Met or Val or Leu or Ile
  variant (17)..(17): Thr or Gln or Ser or Asn
  variant (18)..(18): Thr or Gln or Ser or Asn
  variant (19)..(19): Ala or Met or Val or Leu or Ile
  variant (20)..(20): Trp or Phe
  variant (23)..(23): Ala or Met or Val or Leu or Ile
  variant (26)..(26): Trp or Phe

SEQ ID NO: 72 - protein, 30 aa, artificial
  antimicrobial peptide pattern
  variant (5)..(5): Ala or Met or Val or Leu or Ile
  variant (6)..(6): Asp or Glu
  variant (7)..(7): Asp or Glu
  variant (8)..(8): Trp or Phe
  variant (9)..(9): Trp or Phe
  variant (10)..(10): Asp or Glu
  variant (11)..(11): Asp or Glu
  variant (12)..(12): Ala or Met or Val or Leu or Ile
  variant (13)..(13): Ala or Met or Val or Leu or Ile
  variant (14)..(14): Thr or Gln or Ser or Asn
  variant (15)..(15): Ala or Met or Val or Leu or Ile
  variant (16)..(16): Ala or Met or Val or Leu or Ile
  variant (18)..(18): Thr or Gln or Ser or Asn
  variant (19)..(19): Ala or Met or Val or Leu or Ile
  variant (20)..(20): Trp or Phe
  variant (23)..(23): Ala or Met or Val or Leu or Ile
  variant (26)..(26): Trp or Phe
KKKKXXXXXXXXXXXXKXXXKKXKKXKKKK

SEQ ID NO: 73 - protein, 5 aa, artificial
  fragment pattern
  variant (1)..(1): Ala or Met or Val or Leu or Ile
  variant (2)..(2): Ala or Met or Val or Leu or Ile
  variant (3)..(3): Thr or Gln or Ser or Asn
  variant (4)..(4): Ala or Met or Val or Leu or Ile
  variant (5)..(5): Ala or Met or Val or Leu or Ile
XXXXX

SEQ ID NO: 74 - protein, 5 aa, artificial
  fragment pattern
  variant (1)..(1): Ala or Met or Val or Leu or Ile
  variant (2)..(2): Trp or Phe
  variant (3)..(3): Thr or Gln or Ser or Asn
  variant (4)..(4): Trp or Phe
  variant (5)..(5): Ala or Met or Val or Leu or Ile
XXXXX

SEQ ID NO: 75 - protein, 5 aa, artificial
  fragment pattern
  variant (5)..(5): Ala or Met or Val or Leu or Ile
KKKKX

SEQ ID NO: 76 - protein, 5 aa, artificial
  fragment pattern
  variant (2)..(2): Thr or Gln or Ser or Asn
  variant (3)..(3): Thr or Gln or Ser or Asn
  variant (4)..(4): Thr or Gln or Ser or Asn
  variant (5)..(5): Ala or Met or Val or Leu or Ile
KXXXX

SEQ ID NO: 77 - protein, 5 aa, artificial
  fragment pattern
  variant (2)..(2): Thr or Gln or Ser or Asn
  variant (3)..(3): Thr or Gln or Ser or Asn
  variant (5)..(5): Ala or Met or Val or Leu or Ile
KXXKX

SEQ ID NO: 78 - protein, 5 aa, artificial
  fragment pattern
  variant (3)..(3): Thr or Gln or Ser or Asn
  variant (4)..(4): Thr or Gln or Ser or Asn
  variant (5)..(5): Ala or Met or Val or Leu or Ile
KKXXX

SEQ ID NO: 79 - protein, 4 aa, artificial
  fragment pattern
  variant (1)..(1): Thr or Gln or Ser or Asn
  variant (2)..(2): Thr or Gln or Ser or Asn
  variant (3)..(3): Thr or Gln or Ser or Asn
XXXK

SEQ ID NO: 80 - protein, 4 aa, artificial
  fragment pattern
  variant (2)..(2): Thr or Gln or Ser or Asn
  variant (3)..(3): Thr or Gln or Ser or Asn
KXXK

SEQ ID NO: 81 - protein, 4 aa, artificial
  fragment pattern
  variant (1)..(1): Thr or Gln or Ser or Asn
XKKK

SEQ ID NO: 82 - protein, 4 aa, artificial
  fragment pattern
KKKK

SEQ ID NO: 83 - protein, 30 aa, artificial
  antimicrobial peptide
KKKKLKKILKKLFQFINQLDNQLQDIKQNK

SEQ ID NO: 84 - protein, 30 aa, artificial
  antimicrobial peptide
KKKKLKKILKKLWQWINQLDNQLQDIKQNK

SEQ ID NO: 85 - protein, 30 aa, artificial
  antimicrobial peptide
KKKKLKKILKKLFQFINQLENQLQEIKQNK

SEQ ID NO: 86 - protein, 30 aa, artificial
  antimicrobial peptide
KKKKLKKILKKLFQFINQLDNQLQDFKQNK

SEQ ID NO: 87 - protein, 30 aa, artificial
  antimicrobial peptide
KKKKLKKILKKLFQFINQLDNQLQDIKKKK

SEQ ID NO: 88 - protein, 32 aa, artificial
  antimicrobial peptide
KKKKKLKKILKKLFQFINQLDNQLQDIKKKKK

SEQ ID NO: 89 - protein, 30 aa, artificial
  antimicrobial peptide
KKKKLKKILKKLFQFIDQLDNDLQDIKKKK

SEQ ID NO: 90 - protein, 4 aa, artificial
  artificial
LLQQ

SEQ ID NO: 91 - protein, 4 aa, artificial
  artificial
LIQN

SEQ ID NO: 92 - protein, 30 aa, artificial
  P1
LLQQLQQLLQQLLQLLQQLLQQLQQLLQQL

SEQ ID NO: 93 - protein, 30 aa, artificial
  P2
LIQNLQNILNQLIQLINQLINQLQNILQNL

SEQ ID NO: 94 - protein, 30 aa, artificial
  P3
QNQNLQNQLNQLNQNINQNQNQLQNQLQNL

SEQ ID NO: 95 - protein, 30 aa, artificial
  P4
LIQILLNILNILIQLILILINILLNILQIL

SEQ ID NO: 96 - protein, 30 aa, artificial
  P5
WWQNWQNWWNQWWQWWNQWWNQWQNWWQNW

SEQ ID NO: 97 - protein, 30 aa, artificial
  P6
FFQNFQNFFNQFFQFFNQFFNQFQNFFQNF

SEQ ID NO: 98 - protein, 30 aa, artificial
  P7
WWQWWWNWWNWWWQWWWWWWNWWWNWWQWW

SEQ ID NO: 99 - protein, 30 aa, artificial
  P8
WWQNLQNILNQLIQLINQLINQLQNILQWW

SEQ ID NO: 100 - protein, 30 aa, artificial
  P9
LIQNLQNILNQLIQWWNQLINQLQNILQNL

SEQ ID NO: 101 - protein, 30 aa, artificial
  P10
LIQNLQNILNQWWQWWNQWWNQLQNILQNL

SEQ ID NO: 102 - protein, 30 aa, artificial
  P11
LIQNLQNILNQWIQLWNQLWNQLQNILQNL

SEQ ID NO: 103 - protein, 30 aa, artificial
  P12
LIQNLQNILNQLWQLWNQWINQLQNILQNL

SEQ ID NO: 104 - protein, 30 aa, artificial
  P13
LIQNLQNILNQFFQFFNQFFNQLQNILQNL

SEQ ID NO: 105 - protein, 30 aa, artificial
  P14
LIQNLQNILNQFIQLFNQLFNQLQNILQNL

SEQ ID NO: 106 - protein, 30 aa, artificial
  P15
LIQNLQNILNQLFQLFNQFINQLQNILQNL

SEQ ID NO: 107 - protein, 30 aa, artificial
  P16
LIQNLQNILNQLWQLINQWINQLQNILQNL

SEQ ID NO: 108 - protein, 30 aa, artificial
  P17
LIQNLQNILNQLFQLINQFINQLQNILQNL

SEQ ID NO: 109 - protein, 30 aa, artificial
  P18
LIQNLQNILNQLWQWINQLINQLQNILQNL

SEQ ID NO: 110 - protein, 30 aa, artificial
  P19
LIQNLQNILNQLFQFINQLINQLQNILQNL

SEQ ID NO: 111 - protein, 30 aa, artificial
  P20
NQRRLQNILNQLWQWINQLINQLQNIRRQN

SEQ ID NO: 112 - protein, 30 aa, artificial
  P21
NQRRLQNILNQLFQFINQLINQLQNIRRQN

SEQ ID NO: 113 - protein, 30 aa, artificial
  P22
LIQNLQNWWNQLIQLINQLWNQLQNWLQNL

SEQ ID NO: 114 - protein, 30 aa, artificial
  P23
LIQNLQNFFNQLIQLINQLFNQLQNFLQNL

SEQ ID NO: 115 - protein, 30 aa, artificial
  P24
NQRRLQNWWNQLIQLINQLWNQLQNWRRQN

SEQ ID NO: 116 - protein, 30 aa, artificial
  P25
NQRRLQNFFNQLIQLINQLFNQLQNFRRQN

SEQ ID NO: 117 - protein, 30 aa, artificial
  P26
RRQNLQNWWNQLIQLINQLWNQLQNWNQRR

SEQ ID NO: 118 - protein, 30 aa, artificial
  P27
RRQNLQNFFNQLIQLINQLFNQLQNFNQRR

SEQ ID NO: 119 - protein, 4 aa, artificial
  artificial
NQRR

SEQ ID NO: 120 - protein, 4 aa, artificial
  artificial
RRQN

SEQ ID NO: 121 - protein, 30 aa, artificial
  pattern
  variant (1)..(1): Thr or Gln or Ser or Asn or Arg or Lys
  variant (2)..(2): Thr or Gln or Ser or Asn or Arg or Lys
  variant (3)..(3): Thr or Gln or Ser or Asn or Arg or Lys
  variant (4)..(4): Thr or Gln or Ser or Asn or Arg or Lys
  variant (5)..(5): Ala or Met or Val or Leu or Ile
  variant (6)..(6): Arg or Lys
  variant (7)..(7): Arg or Lys
  variant (8)..(8): Ala or Met or Val or Leu or Ile
  variant (9)..(9): Ala or Met or Val or Leu or Ile
  variant (10)..(10): Thr or Gln or Ser or Asn
  variant (11)..(11): Thr or Gln or Ser or Asn
  variant (12)..(12): Ala or Met or Val or Leu or Ile
  variant (13)..(13): Trp or Phe
  variant (14)..(14): Thr or Gln or Ser or Asn
  variant (15)..(15): Trp or Phe
  variant (16)..(16): Ala or Met or Val or Leu or Ile
  variant (17)..(17): Thr or Gln or Ser or Asn
  variant (18)..(18): Thr or Gln or Ser or Asn
  variant (19)..(19): Ala or Met or Val or Leu or Ile
  variant (20)..(20): Asp or Glu
  variant (21)..(21): Thr or Gln or Ser or Asn
  variant (22)..(22): Thr or Gln or Ser or Asn
  variant (23)..(23): Ala or Met or Val or Leu or Ile
  variant (24)..(24): Thr or Gln or Ser or Asn
  variant (25)..(25): Asp or Glu
  variant (26)..(26): Ala or Met or Val or Leu or Ile
  variant (27)..(27): Thr or Gln or Ser or Asn or Arg or Lys
  variant (28)..(28): Thr or Gln or Ser or Asn
  variant (29)..(29): Thr or Gln or Ser or Asn
  variant (30)..(30): Thr or Gln or Ser or Asn or Arg or Lys
XXXXXXXXXXXXXXXXXXXXXXXXXXXXXX

SEQ ID NO: 122 - protein, 30 aa, artificial; identical to SEQ ID NO: 121
  pattern
  variant (1)..(1): Thr or Gln or Ser or Asn or Arg or Lys
  variant (2)..(2): Thr or Gln or Ser or Asn or Arg or Lys
  variant (3)..(3): Thr or Gln or Ser or Asn or Arg or Lys
  variant (4)..(4): Thr or Gln or Ser or Asn or Arg or Lys
  variant (5)..(5): Ala or Met or Val or Leu or Ile
  variant (6)..(6): Arg or Lys
  variant (7)..(7): Arg or Lys
  variant (8)..(8): Ala or Met or Val or Leu or Ile
  variant (9)..(9): Ala or Met or Val or Leu or Ile
  variant (10)..(10): Arg or Lys
  variant (11)..(11): Arg or Lys
  variant (12)..(12): Ala or Met or Val or Leu or Ile
  variant (13)..(13): Trp or Phe
  variant (14)..(14): Thr or Gln or Ser or Asn
  variant (15)..(15): Trp or Phe
  variant (16)..(16): Ala or Met or Val or Leu or Ile
  variant (17)..(17): Thr or Gln or Ser or Asn
  variant (18)..(18): Thr or Gln or Ser or Asn
  variant (19)..(19): Ala or Met or Val or Leu or Ile
  variant (20)..(20): Asp or Glu
  variant (21)..(21): Thr or Gln or Ser or Asn
  variant (22)..(22): Thr or Gln or Ser or Asn
  variant (23)..(23): Ala or Met or Val or Leu or Ile
  variant (24)..(24): Thr or Gln or Ser or Asn
  variant (25)..(25): Asp or Glu
  variant (26)..(26): Ala or Met or Val or Leu or Ile
  variant (27)..(27): Thr or Gln or Ser or Asn or Arg or Lys
  variant (28)..(28): Thr or Gln or Ser or Asn
  variant (29)..(29): Thr or Gln or Ser or Asn
  variant (30)..(30): Thr or Gln or Ser or Asn or Arg or Lys

SEQ ID NO: 123 - protein, 30 aa, artificial; identical to SEQ ID NO: 121
  pattern
  variant (1)..(1): Thr or Gln or Ser or Asn or Arg or Lys
  variant (2)..(2): Thr or Gln or Ser or Asn
  variant (3)..(3): Thr or Gln or Ser or Asn
  variant (4)..(4): Thr or Gln or Ser or Asn
  variant (5)..(5): Ala or Met or Val or Leu or Ile
  variant (6)..(6): Asp or Glu
  variant (7)..(7): Asp or Glu
  variant (8)..(8): Ala or Met or Val or Leu or Ile
  variant (9)..(9): Ala or Met or Val or Leu or Ile
  variant (10)..(10): Thr or Gln or Ser or Asn
  variant (11)..(11): Thr or Gln or Ser or Asn
  variant (12)..(12): Ala or Met or Val or Leu or Ile
  variant (13)..(13): Trp or Phe
  variant (14)..(14): Thr or Gln or Ser or Asn
  variant (15)..(15): Trp or Phe
  variant (16)..(16): Ala or Met or Val or Leu or Ile
  variant (17)..(17): Thr or Gln or Ser or Asn
  variant (18)..(18): Thr or Gln or Ser or Asn
  variant (19)..(19): Ala or Met or Val or Leu or Ile
  variant (20)..(20): Arg or Lys
  variant (21)..(21): Thr or Gln or Ser or Asn
  variant (22)..(22): Thr or Gln or Ser or Asn
  variant (23)..(23): Ala or Met or Val or Leu or Ile
  variant (24)..(24): Thr or Gln or Ser or Asn
  variant (25)..(25): Arg or Lys
  variant (26)..(26): Ala or Met or Val or Leu or Ile
  variant (27)..(27): Thr or Gln or Ser or Asn or Arg or Lys
  variant (28)..(28): Thr or Gln or Ser or Asn or Arg or Lys
  variant (29)..(29): Thr or Gln or Ser or Asn or Arg or Lys
  variant (30)..(30): Thr or Gln or Ser or Asn or Arg or Lys

SEQ ID NO: 124 - protein, 30 aa, artificial; identical to SEQ ID NO: 121
  pattern
  variant (1)..(1): Thr or Gln or Ser or Asn or Arg or Lys
  variant (2)..(2): Thr or Gln or Ser or Asn
  variant (3)..(3): Thr or Gln or Ser or Asn
  variant (4)..(4): Thr or Gln or Ser or Asn
  variant (5)..(5): Ala or Met or Val or Leu or Ile
  variant (6)..(6): Asp or Glu
  variant (7)..(7): Asp or Glu
  variant (8)..(8): Ala or Met or Val or Leu or Ile
  variant (9)..(9): Ala or Met or Val or Leu or Ile
  variant (10)..(10): Thr or Gln or Ser or Asn
  variant (11)..(11): Thr or Gln or Ser or Asn
  variant (12)..(12): Ala or Met or Val or Leu or Ile
  variant (13)..(13): Trp or Phe
  variant (14)..(14): Thr or Gln or Ser or Asn
  variant (15)..(15): Trp or Phe
  variant (16)..(16): Ala or Met or Val or Leu or Ile
  variant (17)..(17): Arg or Lys
  variant (18)..(18): Thr or Gln or Ser or Asn
  variant (19)..(19): Ala or Met or Val or Leu or Ile
  variant (20)..(20): Arg or Lys
  variant (21)..(21): Thr or Gln or Ser or Asn
  variant (22)..(22): Arg or Lys
  variant (23)..(23): Ala or Met or Val or Leu or Ile
  variant (24)..(24): Thr or Gln or Ser or Asn
  variant (25)..(25): Arg or Lys
  variant (26)..(26): Ala or Met or Val or Leu or Ile
  variant (27)..(27): Thr or Gln or Ser or Asn or Arg or Lys
  variant (28)..(28): Thr or Gln or Ser or Asn or Arg or Lys
  variant (29)..(29): Thr or Gln or Ser or Asn or Arg or Lys
  variant (30)..(30): Thr or Gln or Ser or Asn or Arg or Lys

SEQ ID NO: 125 - protein, 30 aa, artificial; identical to SEQ ID NO: 121
  pattern
  variant (1)..(1): Thr or Gln or Ser or Asn or Arg or Lys
  variant (2)..(2): Thr or Gln or Ser or Asn or Arg or Lys
  variant (3)..(3): Thr or Gln or Ser or Asn or Arg or Lys
  variant (4)..(4): Thr or Gln or Ser or Asn or Arg or Lys
  variant (5)..(5): Ala or Met or Val or Leu or Ile
  variant (6)..(6): Arg or Lys
  variant (7)..(7): Thr or Gln or Ser or Asn
  variant (8)..(8): Ala or Met or Val or Leu or Ile
  variant (9)..(9): Ala or Met or Val or Leu or Ile
  variant (10)..(10): Thr or Gln or Ser or Asn
  variant (11)..(11): Arg or Lys
  variant (12)..(12): Ala or Met or Val or Leu or Ile
  variant (13)..(13): Trp or Phe
  variant (14)..(14): Thr or Gln or Ser or Asn
  variant (15)..(15): Trp or Phe
  variant (16)..(16): Ala or Met or Val or Leu or Ile
  variant (17)..(17): Thr or Gln or Ser or Asn
  variant (18)..(18): Thr or Gln or Ser or Asn
  variant (19)..(19): Ala or Met or Val or Leu or Ile
  variant (20)..(20): Asp or Glu
  variant (21)..(21): Thr or Gln or Ser or Asn
  variant (22)..(22): Asp or Glu
  variant (23)..(23): Ala or Met or Val or Leu or Ile
  variant (24)..(24): Thr or Gln or Ser or Asn
  variant (25)..(25): Thr or Gln or Ser or Asn
  variant (26)..(26): Ala or Met or Val or Leu or Ile
  variant (27)..(27): Thr or Gln or Ser or Asn or Arg or Lys
  variant (28)..(28): Thr or Gln or Ser or Asn or Arg or Lys
  variant (29)..(29): Thr or Gln or Ser or Asn or Arg or Lys
  variant (30)..(30): Thr or Gln or Ser or Asn or Arg or Lys

SEQ ID NO: 126 - protein, 30 aa, artificial; identical to SEQ ID NO: 121
  pattern
  variant (1)..(1): Thr or Gln or Ser or Asn or Arg or Lys
  variant (2)..(2): Thr or Gln or Ser or Asn or Arg or Lys
  variant (3)..(3): Thr or Gln or Ser or Asn or Arg or Lys
  variant (4)..(4): Thr or Gln or Ser or Asn or Arg or Lys
  variant (5)..(5): Ala or Met or Val or Leu or Ile
  variant (6)..(6): Arg or Lys
  variant (7)..(7): Arg or Lys
  variant (8)..(8): Ala or Met or Val or Leu or Ile
  variant (9)..(9): Ala or Met or Val or Leu or Ile
  variant (10)..(10): Arg or Lys
  variant (11)..(11): Arg or Lys
  variant (12)..(12): Ala or Met or Val or Leu or Ile
  variant (13)..(13): Trp or Phe
  variant (14)..(14): Thr or Gln or Ser or Asn
  variant (15)..(15): Trp or Phe
  variant (16)..(16): Ala or Met or Val or Leu or Ile
  variant (17)..(17): Thr or Gln or Ser or Asn
  variant (18)..(18): Thr or Gln or Ser or Asn
  variant (19)..(19): Ala or Met or Val or Leu or Ile
  variant (20)..(20): Asp or Glu
  variant (21)..(21): Thr or Gln or Ser or Asn
  variant (22)..(22): Asp or Glu
  variant (23)..(23): Ala or Met or Val or Leu or Ile
  variant (24)..(24): Thr or Gln or Ser or Asn
  variant (25)..(25): Thr or Gln or Ser or Asn
  variant (26)..(26): Ala or Met or Val or Leu or Ile
  variant (27)..(27): Thr or Gln or Ser or Asn or Arg or Lys
  variant (28)..(28): Thr or Gln or Ser or Asn or Arg or Lys
  variant (29)..(29): Thr or Gln or Ser or Asn or Arg or Lys
  variant (30)..(30): Thr or Gln or Ser or Asn or Arg or Lys

SEQ ID NO: 127 - protein, 30 aa, artificial; identical to SEQ ID NO: 121
  pattern
  variant (1)..(1): Thr or Gln or Ser or Asn or Arg or Lys
  variant (2)..(2): Thr or Gln or Ser or Asn
  variant (3)..(3): Thr or Gln or Ser or Asn
  variant (4)..(4): Thr or Gln or Ser or Asn or Arg or Lys
  variant (5)..(5): Ala or Met or Val or Leu or Ile
  variant (6)..(6): Asp or Glu
  variant (7)..(7): Thr or Gln or Ser or Asn
  variant (8)..(8): Ala or Met or Val or Leu or Ile
  variant (9)..(9): Ala or Met or Val or Leu or Ile
  variant (10)..(10): Thr or Gln or Ser or Asn
  variant (11)..(11): Asp or Glu
  variant (12)..(12): Ala or Met or Val or Leu or Ile
  variant (13)..(13): Trp or Phe
  variant (14)..(14): Thr or Gln or Ser or Asn
  variant (15)..(15): Trp or Phe
  variant (16)..(16): Ala or Met or Val or Leu or Ile
  variant (17)..(17): Thr or Gln or Ser or Asn
  variant (18)..(18): Thr or Gln or Ser or Asn
  variant (19)..(19): Ala or Met or Val or Leu or Ile
  variant (20)..(20): Arg or Lys
  variant (21)..(21): Thr or Gln or Ser or Asn
  variant (22)..(22): Arg or Lys
  variant (23)..(23): Ala or Met or Val or Leu or Ile
  variant (24)..(24): Thr or Gln or Ser or Asn
  variant (25)..(25): Thr or Gln or Ser or Asn
  variant (26)..(26): Ala or Met or Val or Leu or Ile
  variant (27)..(27): Thr or Gln or Ser or Asn or Arg or Lys
  variant (28)..(28): Thr or Gln or Ser or Asn or Arg or Lys
  variant (29)..(29): Thr or Gln or Ser or Asn or Arg or Lys
  variant (30)..(30): Thr or Gln or Ser or Asn or Arg or Lys

SEQ ID NO: 128 - protein, 30 aa, artificial; identical to SEQ ID NO: 121
  pattern
  variant (1)..(1): Thr or Gln or Ser or Asn or Arg or Lys
  variant (2)..(2): Thr or Gln or Ser or Asn
  variant (3)..(3): Thr or Gln or Ser or Asn
  variant (4)..(4): Thr or Gln or Ser or Asn or Arg or Lys
  variant (5)..(5): Ala or Met or Val or Leu or Ile
  variant (6)..(6): Asp or Glu
  variant (7)..(7): Thr or Gln or Ser or Asn
  variant (8)..(8): Ala or Met or Val or Leu or Ile
  variant (9)..(9): Ala or Met or Val or Leu or Ile
  variant (10)..(10): Thr or Gln or Ser or Asn
  variant (11)..(11): Asp or Glu
  variant (12)..(12): Ala or Met or Val or Leu or Ile
  variant (13)..(13): Trp or Phe
  variant (14)..(14): Thr or Gln or Ser or Asn
  variant (15)..(15): Trp or Phe
  variant (16)..(16): Ala or Met or Val or Leu or Ile
  variant (17)..(17): Arg or Lys
  variant (18)..(18): Thr or Gln or Ser or Asn
  variant (19)..(19): Ala or Met or Val or Leu or Ile
  variant (20)..(20): Arg or Lys
  variant (21)..(21): Thr or Gln or Ser or Asn
  variant (22)..(22): Arg or Lys
  variant (23)..(23): Ala or Met or Val or Leu or Ile
  variant (24)..(24): Thr or Gln or Ser or Asn
  variant (25)..(25): Arg or Lys
  variant (26)..(26): Ala or Met or Val or Leu or Ile
  variant (27)..(27): Thr or Gln or Ser or Asn or Arg or Lys
  variant (28)..(28): Thr or Gln or Ser or Asn or Arg or Lys
  variant (29)..(29): Thr or Gln or Ser or Asn or Arg or Lys
  variant (30)..(30): Thr or Gln or Ser or Asn or Arg or Lys

SEQ ID NO: 129 - protein, 30 aa, artificial; identical to SEQ ID NO: 121
  pattern
  variant (1)..(1): Thr or Gln or Ser or Asn or Arg or Lys
  variant (2)..(2): Thr or Gln or Ser or Asn or Arg or Lys
  variant (3)..(3): Thr or Gln or Ser or Asn or Arg or Lys
  variant (4)..(4): Thr or Gln or Ser or Asn or Arg or Lys
  variant (5)..(5): Ala or Met or Val or Leu or Ile
  variant (6)..(6): Thr or Gln or Ser or Asn
  variant (7)..(7): Arg or Lys
  variant (8)..(8): Ala or Met or Val or Leu or Ile
  variant (9)..(9): Ala or Met or Val or Leu or Ile
  variant (10)..(10): Arg or Lys
  variant (11)..(11): Thr or Gln or Ser or Asn
  variant (12)..(12): Ala or Met or Val or Leu or Ile
  variant (13)..(13): Trp or Phe
  variant (14)..(14): Thr or Gln or Ser or Asn
  variant (15)..(15): Trp or Phe
  variant (16)..(16): Ala or Met or Val or Leu or Ile
  variant (17)..(17): Asp or Glu
  variant (18)..(18): Thr or Gln or Ser or Asn
  variant (19)..(19): Ala or Met or Val or Leu or Ile
  variant (20)..(20): Ala or Met or Val or Leu or Ile
  variant (21)..(21): Thr or Gln or Ser or Asn
  variant (22)..(22): Thr or Gln or Ser or Asn
  variant (23)..(23): Ala or Met or Val or Leu or Ile
  variant (24)..(24): Thr or Gln or Ser or Asn
  variant (25)..(25): Asp or Glu
  variant (26)..(26): Ala or Met or Val or Leu or Ile
  variant (27)..(27): Thr or Gln or Ser or Asn or Arg or Lys
  variant (28)..(28): Thr or Gln or Ser or Asn
  variant (29)..(29): Thr or Gln or Ser or Asn
  variant (30)..(30): Thr or Gln or Ser or Asn or Arg or Lys

SEQ ID NO: 130 - protein, 30 aa, artificial; identical to SEQ ID NO: 121
  pattern
  variant (1)..(1): Thr or Gln or Ser or Asn or Arg or Lys
  variant (2)..(2): Thr or Gln or Ser or Asn or Arg or Lys
  variant (3)..(3): Thr or Gln or Ser or Asn or Arg or Lys
  variant (4)..(4): Thr or Gln or Ser or Asn or Arg or Lys
  variant (5)..(5): Ala or Met or Val or Leu or Ile
  variant (6)..(6): Arg or Lys
  variant (7)..(7): Arg or Lys
  variant (8)..(8): Ala or Met or Val or Leu or Ile
  variant (9)..(9): Ala or Met or Val or Leu or Ile
  variant (10)..(10): Arg or Lys
  variant (11)..(11): Arg or Lys
  variant (12)..(12): Ala or Met or Val or Leu or Ile
  variant (13)..(13): Trp or Phe
  variant (14)..(14): Thr or Gln or Ser or Asn
  variant (15)..(15): Trp or Phe
  variant (16)..(16): Ala or Met or Val or Leu or Ile
  variant (17)..(17): Asp or Glu
  variant (18)..(18): Thr or Gln or Ser or Asn
  variant (19)..(19): Ala or Met or Val or Leu or Ile
  variant (20)..(20): Ala or Met or Val or Leu or Ile
  variant (21)..(21): Thr or Gln or Ser or Asn
  variant (22)..(22): Thr or Gln or Ser or Asn
  variant (23)..(23): Ala or Met or Val or Leu or Ile
  variant (24)..(24): Thr or Gln or Ser or Asn
  variant (25)..(25): Asp or Glu
  variant (26)..(26): Ala or Met or Val or Leu or Ile
  variant (27)..(27): Thr or Gln or Ser or Asn or Arg or Lys
  variant (28)..(28): Thr or Gln or Ser or Asn
  variant (29)..(29): Thr or Gln or Ser or Asn
  variant (30)..(30): Thr or Gln or Ser or Asn or Arg or Lys

SEQ ID NO: 131 - protein, 30 aa, artificial; identical to SEQ ID NO: 121
  pattern
  variant (1)..(1): Thr or Gln or Ser or Asn or Arg or Lys
  variant (2)..(2): Thr or Gln or Ser or Asn or Arg or Lys
  variant (3)..(3): Thr or Gln or Ser or Asn
  variant (4)..(4): Thr or Gln or Ser or Asn
  variant (5)..(5): Ala or Met or Val or Leu or Ile
  variant (6)..(6): Thr or Gln or Ser or Asn
  variant (7)..(7): Asp or Glu
  variant (8)..(8): Ala or Met or Val or Leu or Ile
  variant (9)..(9): Ala or Met or Val or Leu or Ile
  variant (10)..(10): Asp or Glu
  variant (11)..(11): Thr or Gln or Ser or Asn
  variant (12)..(12): Ala or Met or Val or Leu or Ile
  variant (13)..(13): Trp or Phe
  variant (14)..(14): Thr or Gln or Ser or Asn
  variant (15)..(15): Trp or Phe
  variant (16)..(16): Ala or Met or Val or Leu or Ile
  variant (17)..(17): Arg or Lys
  variant (18)..(18): Thr or Gln or Ser or Asn
  variant (19)..(19): Ala or Met or Val or Leu or Ile
  variant (20)..(20): Ala or Met or Val or Leu or Ile
  variant (21)..(21): Thr or Gln or Ser or Asn
  variant (22)..(22): Thr or Gln or Ser or Asn
  variant (23)..(23): Ala or Met or Val or Leu or Ile
  variant (24)..(24): Thr or Gln or Ser or Asn
  variant (25)..(25): Arg or Lys
  variant (26)..(26): Ala or Met or Val or Leu or Ile
  variant (27)..(27): Thr or Gln or Ser or Asn or Arg or Lys
  variant (28)..(28): Thr or Gln or Ser or Asn or Arg or Lys
  variant (29)..(29): Thr or Gln or Ser or Asn or Arg or Lys
  variant (30)..(30): Thr or Gln or Ser or Asn or Arg or Lys

SEQ ID NO: 132 - protein, 30 aa, artificial; identical to SEQ ID NO: 121
  pattern
  variant (1)..(1): Thr or Gln or Ser or Asn or Arg or Lys
  variant (2)..(2): Thr or Gln or Ser or Asn or Arg or Lys
  variant (3)..(3): Thr or Gln or Ser or Asn
  variant (4)..(4): Thr or Gln or Ser or Asn
  variant (5)..(5): Ala or Met or Val or Leu or Ile
  variant (6)..(6): Thr or Gln or Ser or Asn
  variant (7)..(7): Asp or Glu
  variant (8)..(8): Ala or Met or Val or Leu or Ile
  variant (9)..(9): Ala or Met or Val or Leu or Ile
  variant (10)..(10): Asp or Glu
  variant (11)..(11): Thr or Gln or Ser or Asn
  variant (12)..(12): Ala or Met or Val or Leu or Ile
  variant (13)..(13): Trp or Phe
  variant (14)..(14): Thr or Gln or Ser or Asn
  variant (15)..(15): Trp or Phe
  variant (16)..(16): Ala or Met or Val or Leu or Ile
  variant (17)..(17): Arg or Lys
  variant (18)..(18): Thr or Gln or Ser or Asn
  variant (19)..(19): Ala or Met or Val or Leu or Ile
  variant (20)..(20): Arg or Lys
  variant (21)..(21): Thr or Gln or Ser or Asn
  variant (22)..(22): Arg or Lys
  variant (23)..(23): Ala or Met or Val or Leu or Ile
  variant (24)..(24): Thr or Gln or Ser or Asn
  variant (25)..(25): Arg or Lys
  variant (26)..(26): Ala or Met or Val or Leu or Ile
  variant (27)..(27): Thr or Gln or Ser or Asn or Arg or Lys
  variant (28)..(28): Thr or Gln or Ser or Asn or Arg or Lys
  variant (29)..(29): Thr or Gln or Ser or Asn or Arg or Lys
  variant (30)..(30): Thr or Gln or Ser or Asn or Arg or Lys

SEQ ID NO: 133 - protein, 30 aa, artificial; identical to SEQ ID NO: 121
  pattern
  variant (1)..(1): Thr or Gln or Ser or Asn or Arg or Lys
  variant (2)..(2): Thr or Gln or Ser or Asn or Arg or Lys
  variant (3)..(3): Thr or Gln or Ser or Asn or Arg or Lys
  variant (4)..(4): Thr or Gln or Ser or Asn or Arg or Lys
  variant (5)..(5): Ala or Met or Val or Leu or Ile
  variant (6)..(6): Thr or Gln or Ser or Asn
  variant (7)..(7): Thr or Gln or Ser or Asn
  variant (8)..(8): Ala or Met or Val or Leu or Ile
  variant (9)..(9): Ala or Met or Val or Leu or Ile
  variant (10)..(10): Arg or Lys
  variant (11)..(11): Arg or Lys
  variant (12)..(12): Ala or Met or Val or Leu or Ile
  variant (13)..(13): Trp or Phe
  variant (14)..(14): Thr or Gln or Ser or Asn
  variant (15)..(15): Trp or Phe
  variant (16)..(16): Ala or Met or Val or Leu or Ile
  variant (17)..(17): Asp or Glu
  variant (18)..(18): Thr or Gln or Ser or Asn
  variant (19)..(19): Ala or Met or Val or Leu or Ile
  variant (20)..(20): Ala or Met or Val or Leu or Ile
  variant (21)..(21): Thr or Gln or Ser or Asn
  variant (22)..(22): Asp or Glu
  variant (23)..(23): Ala or Met or Val or Leu or Ile
  variant (24)..(24): Thr or Gln or Ser or Asn
  variant (25)..(25): Thr or Gln or Ser or Asn
  variant (26)..(26): Ala or Met or Val or Leu or Ile
  variant (27)..(27): Thr or Gln or Ser or Asn or Arg or Lys
  variant (28)..(28): Thr or Gln or Ser or Asn or Arg or Lys
  variant (29)..(29): Thr or Gln or Ser or Asn or Arg or Lys
  variant (30)..(30): Thr or Gln or Ser or Asn or Arg or Lys

SEQ ID NO: 134 - protein, 30 aa, artificial; identical to SEQ ID NO: 121
  pattern
  variant (1)..(1): Thr or Gln or Ser or Asn or Arg or Lys
  variant (2)..(2): Thr or Gln or Ser or Asn or Arg or Lys
  variant (3)..(3): Thr or Gln or Ser or Asn or Arg or Lys
  variant (4)..(4): Thr or Gln or Ser or Asn or Arg or Lys
  variant (5)..(5): Ala or Met or Val or Leu or Ile
  variant (6)..(6): Arg or Lys
  variant (7)..(7): Arg or Lys
  variant (8)..(8): Ala or Met or Val or Leu or Ile
  variant (9)..(9): Ala or Met or Val or Leu or Ile
  variant (10)..(10): Arg or Lys
  variant (11)..(11): Arg or Lys
  variant (12)..(12): Ala or Met or Val or Leu or Ile
  variant (13)..(13): Trp or Phe
  variant (14)..(14): Thr or Gln or Ser or Asn
  variant (15)..(15): Trp or Phe
  variant (16)..(16): Ala or Met or Val or Leu or Ile
  variant (17)..(17): Asp or Glu
  variant (18)..(18): Thr or Gln or Ser or Asn
  variant (19)..(19): Ala or Met or Val or Leu or Ile
  variant (20)..(20): Ala or Met or Val or Leu or Ile
  variant (21)..(21): Thr or Gln or Ser or Asn
  variant (22)..(22): Asp or Glu
  variant (23)..(23): Ala or Met or Val or Leu or Ile
  variant (24)..(24): Thr or Gln or Ser or Asn
  variant (25)..(25): Thr or Gln or Ser or Asn
  variant (26)..(26): Ala or Met or Val or Leu or Ile
  variant (27)..(27): Thr or Gln or Ser or Asn or Arg or Lys
  variant (28)..(28): Thr or Gln or Ser or Asn or Arg or Lys
  variant (29)..(29): Thr or Gln or Ser or Asn or Arg or Lys
  variant (30)..(30): Thr or Gln or Ser or Asn or Arg or Lys

SEQ ID NO: 135 - protein, 30 aa, artificial; identical to SEQ ID NO: 121
  pattern
  variant (1)..(1): Thr or Gln or Ser or Asn or Arg or Lys
  variant (2)..(2): Thr or Gln or Ser or Asn or Arg or Lys
  variant (3)..(3): Thr or Gln or Ser or Asn or Arg or Lys
  variant (4)..(4): Thr or Gln or Ser or Asn or Arg or Lys
  variant (5)..(5): Ala or Met or Val or Leu or Ile
  variant (6)..(6): Thr or Gln or Ser or Asn
  variant (7)..(7): Thr or Gln or Ser or Asn
  variant (8)..(8): Ala or Met or Val or Leu or Ile
  variant (9)..(9): Ala or Met or Val or Leu or Ile
  variant (10)..(10): Asp or Glu
  variant (11)..(11): Asp or Glu
  variant (12)..(12): Ala or Met or Val or Leu or Ile
  variant (13)..(13): Trp or Phe
  variant (14)..(14): Thr or Gln or Ser or Asn
  variant (15)..(15): Trp or Phe
  variant (16)..(16): Ala or Met or Val or Leu or Ile
  variant (17)..(17): Arg or Lys
  variant (18)..(18): Thr or Gln or Ser or Asn
  variant (19)..(19): Ala or Met or Val or Leu or Ile
  variant (20)..(20): Ala or Met or Val or Leu or Ile
  variant (21)..(21): Thr or Gln or Ser or Asn
  variant (22)..(22): Arg or Lys
  variant (23)..(23): Ala or Met or Val or Leu or Ile
  variant (24)..(24): Thr or Gln or Ser or Asn
  variant (25)..(25): Thr or Gln or Ser or Asn
  variant (26)..(26): Ala or Met or Val or Leu or Ile
  variant (27)..(27): Thr or Gln or Ser or Asn or Arg or Lys
  variant (28)..(28): Thr or Gln or Ser or Asn or Arg or Lys
  variant (29)..(29): Thr or Gln or Ser or Asn or Arg or Lys
  variant (30)..(30): Thr or Gln or Ser or Asn or Arg or Lys

SEQ ID NO: 136 - protein, 30 aa, artificial; identical to SEQ ID NO: 121
  pattern
  variant (1)..(1): Thr or Gln or Ser or Asn or Arg or Lys
  variant (2)..(2): Thr or Gln or Ser or Asn or Arg or Lys
  variant (3)..(3): Thr or Gln or Ser or Asn or Arg or Lys
  variant (4)..(4): Thr or Gln or Ser or Asn or Arg or Lys
  variant (5)..(5): Ala or Met or Val or Leu or Ile
  variant (6)..(6): Thr or Gln or Ser or Asn
  variant (7)..(7): Thr or Gln or Ser or Asn
  variant (8)..(8): Ala or Met or Val or Leu or Ile
  variant (9)..(9): Ala or Met or Val or Leu or Ile
  variant (10)..(10): Asp or Glu
  variant (11)..(11): Asp or Glu
  variant (12)..(12): Ala or Met or Val or Leu or Ile
  variant (13)..(13): Trp or Phe
  variant (14)..(14): Thr or Gln or Ser or Asn
  variant (15)..(15): Trp or Phe
  variant (16)..(16): Ala or Met or Val or Leu or Ile
  variant (17)..(17): Arg or Lys
  variant (18)..(18): Thr or Gln or Ser or Asn
  variant (19)..(19): Ala or Met or Val or Leu or Ile
  variant (20)..(20): Arg or Lys
  variant (21)..(21): Thr or Gln or Ser or Asn
  variant (22)..(22): Arg or Lys
  variant (23)..(23): Ala or Met or Val or Leu or Ile
  variant (24)..(24): Thr or Gln or Ser or Asn
  variant (25)..(25): Arg or Lys
  variant (26)..(26): Ala or Met or Val or Leu or Ile
  variant (27)..(27): Thr or Gln or Ser or Asn or Arg or Lys
  variant (28)..(28): Thr or Gln or Ser or Asn or Arg or Lys
  variant (29)..(29): Thr or Gln or Ser or Asn or Arg or Lys
  variant (30)..(30): Thr or Gln or Ser or Asn or Arg or Lys

SEQ ID NO: 137 - protein, 30 aa, artificial; identical to SEQ ID NO: 121
  pattern
  variant (1)..(1): Thr or Gln or Ser or Asn or Arg or Lys
  variant (2)..(2): Thr or Gln or Ser or Asn or Arg or Lys
  variant (3)..(3): Thr or Gln or Ser or Asn or Arg or Lys
  variant (4)..(4): Thr or Gln or Ser or Asn or Arg or Lys
  variant (5)..(5): Ala or Met or Val or Leu or Ile
  variant (6)..(6): Arg or Lys
  variant (7)..(7): Arg or Lys
  variant (8)..(8): Trp or Phe
  variant (9)..(9): Trp or Phe
  variant (10)..(10): Thr or Gln or Ser or Asn
  variant (11)..(11): Thr or Gln or Ser or Asn
  variant (12)..(12): Ala or Met or Val or Leu or Ile
  variant (13)..(13): Ala or Met or Val or Leu or Ile
  variant (14)..(14): Thr or Gln or Ser or Asn
  variant (15)..(15): Ala or Met or Val or Leu or Ile
  variant (16)..(16): Ala or Met or Val or Leu or Ile
  variant (17)..(17): Thr or Gln or Ser or Asn
  variant (18)..(18): Thr or Gln or Ser or Asn
  variant (19)..(19): Ala or Met or Val or Leu or Ile
  variant (20)..(20): Trp or Phe
  variant (21)..(21): Thr or Gln or Ser or Asn
  variant (22)..(22): Thr or Gln or Ser or Asn
  variant (23)..(23): Ala or Met or Val or Leu or Ile
  variant (24)..(24): Asp or Glu
  variant (25)..(25): Asp or Glu
  variant (26)..(26): Trp or Phe
  variant (27)..(27): Thr or Gln or Ser or Asn
  variant (28)..(28): Thr or Gln or Ser or Asn
  variant (29)..(29): Thr or Gln or Ser or Asn
  variant (30)..(30): Thr or Gln or Ser or Asn or Arg or Lys

SEQ ID NO: 138 - protein, 30 aa, artificial; identical to SEQ ID NO: 121
  pattern
  variant (1)..(1): Thr or Gln or Ser or Asn or Arg or Lys
  variant (2)..(2): Thr or Gln or Ser or Asn or Arg or Lys
  variant (3)..(3): Thr or Gln or Ser or Asn or Arg or Lys
  variant (4)..(4): Thr or Gln or Ser or Asn or Arg or Lys
  variant (5)..(5): Ala or Met or Val or Leu or Ile
  variant (6)..(6): Arg or Lys
  variant (7)..(7): Arg or Lys
  variant (8)..(8): Trp or Phe
  variant (9)..(9): Trp or Phe
  variant (10)..(10): Arg or Lys
  variant (11)..(11): Arg or Lys
  variant (12)..(12): Ala or Met or Val or Leu or Ile
  variant (13)..(13): Ala or Met or Val or Leu or Ile
  variant (14)..(14): Thr or Gln or Ser or Asn
  variant (15)..(15): Ala or Met or Val or Leu or Ile
  variant (16)..(16): Ala or Met or Val or Leu or Ile
  variant (17)..(17): Thr or Gln or Ser or Asn
  variant (18)..(18): Thr or Gln or Ser or Asn
  variant (19)..(19): Ala or Met or Val or Leu or Ile
  variant (20)..(20): Trp or Phe
  variant (21)..(21): Thr or Gln or Ser or Asn
  variant (22)..(22): Thr or Gln or Ser or Asn
  variant (23)..(23): Ala or Met or Val or Leu or Ile
  variant (24)..(24): Asp or Glu
  variant (25)..(25): Asp or Glu
  variant (26)..(26): Trp or Phe
  variant (27)..(27): Thr or Gln or Ser or Asn
  variant (28)..(28): Thr or Gln or Ser or Asn
  variant (29)..(29): Thr or Gln or Ser or Asn
  variant (30)..(30): Thr or Gln or Ser or Asn or Arg or Lys

SEQ ID NO: 139 - protein, 30 aa, artificial; identical to SEQ ID NO: 121
  pattern
  variant (1)..(1): Thr or Gln or Ser or Asn or Arg or Lys
  variant (2)..(2): Thr or Gln or Ser or Asn
  variant (3)..(3): Thr or Gln or Ser or Asn
  variant (4)..(4): Thr or Gln or Ser or Asn
  variant (5)..(5): Ala or Met or Val or Leu or Ile
  variant (6)..(6): Asp or Glu
  variant (7)..(7): Asp or Glu
  variant (8)..(8): Trp or Phe
  variant (9)..(9): Trp or Phe
  variant (10)..(10): Thr or Gln or Ser or Asn
  variant (11)..(11): Thr or Gln or Ser or Asn
  variant (12)..(12): Ala or Met or Val or Leu or Ile
  variant (13)..(13): Ala or Met or Val or Leu or Ile
  variant (14)..(14): Thr or Gln or Ser or Asn
  variant (15)..(15): Ala or Met or Val or Leu or Ile
  variant (16)..(16): Ala or Met or Val or Leu or Ile
  variant (17)..(17): Thr or Gln or Ser or Asn
  variant (18)..(18): Thr or Gln or Ser or Asn
  variant (19)..(19): Ala or Met or Val or Leu or Ile
  variant (20)..(20): Trp or Phe
  variant (21)..(21): Thr or Gln or Ser or Asn
  variant (22)..(22): Thr or Gln or Ser or Asn
  variant (23)..(23): Ala or Met or Val or Leu or Ile
  variant (24)..(24): Arg or Lys
  variant (25)..(25): Arg or Lys
  variant (26)..(26): Trp or Phe
  variant (27)..(27): Thr or Gln or Ser or Asn or Arg or Lys
  variant (28)..(28): Thr or Gln or Ser or Asn or Arg or Lys
  variant (29)..(29): Thr or Gln or Ser or Asn or Arg or Lys
  variant (30)..(30): Thr or Gln or Ser or Asn or Arg or Lys

SEQ ID NO: 140 - protein, 30 aa, artificial; identical to SEQ ID NO: 121
  pattern
  variant (1)..(1): Thr or Gln or Ser or Asn or Arg or Lys
  variant (2)..(2): Thr or Gln or Ser or Asn
  variant (3)..(3): Thr or Gln or Ser or Asn
  variant (4)..(4): Thr or Gln or Ser or Asn
  variant (5)..(5): Ala or Met or Val or Leu or Ile
  variant (6)..(6): Asp or Glu
  variant (7)..(7): Asp or Glu
  variant (8)..(8): Trp or Phe
  variant (9)..(9): Trp or Phe
  variant (10)..(10): Thr or Gln or Ser or Asn
  variant (11)..(11): Thr or Gln or Ser or Asn
  variant (12)..(12): Ala or Met or Val or Leu or Ile
  variant (13)..(13): Ala or Met or Val or Leu or Ile
  variant (14)..(14): Thr or Gln or Ser or Asn
  variant (15)..(15): Ala or Met or Val or Leu or Ile
  variant (16)..(16): Ala or Met or Val or Leu or Ile
  variant (17)..(17): Arg or Lys
  variant (18)..(18): Thr or Gln or Ser or Asn
  variant (19)..(19): Ala or Met or Val or Leu or Ile
  variant (20)..(20): Trp or Phe
  variant (21)..(21): Thr or Gln or Ser or Asn
  variant (22)..(22): Arg or Lys
  variant (23)..(23): Ala or Met or Val or Leu or Ile
  variant (24)..(24): Arg or Lys
  variant (25)..(25): Arg or Lys
  variant (26)..(26): Trp or Phe
  variant (27)..(27): Thr or Gln or Ser or Asn or Arg or Lys
  variant (28)..(28): Thr or Gln or Ser or Asn or Arg or Lys
  variant (29)..(29): Thr or Gln or Ser or Asn or Arg or Lys
  variant (30)..(30): Thr or Gln or Ser or Asn or Arg or Lys

SEQ ID NO: 141 - protein, 30 aa, artificial; identical to SEQ ID NO: 121
  pattern
  variant (1)..(1): Thr or Gln or Ser or Asn or Arg or Lys
  variant (2)..(2): Thr or Gln or Ser or Asn or Arg or Lys
  variant (3)..(3): Thr or Gln or Ser or Asn or Arg or Lys
  variant (4)..(4): Thr or Gln or Ser or Asn or Arg or Lys
  variant (5)..(5): Ala or Met or Val or Leu or Ile
  variant (6)..(6): Arg or Lys
  variant (7)..(7): Thr or Gln or Ser or Asn
  variant (8)..(8): Trp or Phe
  variant (9)..(9): Trp or Phe
  variant (10)..(10): Thr or Gln or Ser or Asn
  variant (11)..(11): Arg or Lys
  variant (12)..(12): Ala or Met or Val or Leu or Ile
  variant (13)..(13): Ala or Met or Val or Leu or Ile
  variant (14)..(14): Thr or Gln or Ser or Asn
  variant (15)..(15): Ala or Met or Val or Leu or Ile
  variant (16)..(16): Ala or Met or Val or Leu or Ile
  variant (17)..(17): Thr or Gln or Ser or Asn
  variant (18)..(18): Thr or Gln or Ser or Asn
  variant (19)..(19): Ala or Met or Val or Leu or Ile
  variant (20)..(20): Trp or Phe
  variant (21)..(21): Thr or Gln or Ser or Asn
  variant (22)..(22): Asp or Glu
  variant (23)..(23): Ala or Met or Val or Leu or Ile
  variant (24)..(24): Asp or Glu
  variant (25)..(25): Thr or Gln or Ser or Asn
  variant (26)..(26): Trp or Phe
  variant (27)..(27): Thr or Gln or Ser or Asn
  variant (28)..(28): Thr or Gln or Ser or Asn or Arg or Lys
  variant (29)..(29): Thr or Gln or Ser or Asn or Arg or Lys
  variant (30)..(30): Thr or Gln or Ser or Asn or Arg or Lys

SEQ ID NO: 142 - protein, 30 aa, artificial; identical to SEQ ID NO: 121
  pattern
  variant (1)..(1): Thr or Gln or Ser or Asn or Arg or Lys
  variant (2)..(2): Thr or Gln or Ser or Asn or Arg or Lys
  variant (3)..(3): Thr or Gln or Ser or Asn or Arg or Lys
  variant (4)..(4): Thr or Gln or Ser or Asn or Arg or Lys
  variant (5)..(5): Ala or Met or Val or Leu or Ile
  variant (6)..(6): Arg or Lys
  variant (7)..(7): Arg or Lys
  variant (8)..(8): Trp or Phe
  variant (9)..(9): Trp or Phe
  variant (10)..(10): Arg or Lys
  variant (11)..(11): Arg or Lys
  variant (12)..(12): Ala or Met or Val or Leu or Ile
  variant (13)..(13): Ala or Met or Val or Leu or Ile
  variant (14)..(14): Thr or Gln or Ser or Asn
  variant (15)..(15): Ala or Met or Val or Leu or Ile
  variant (16)..(16): Ala or Met or Val or Leu or Ile
  variant (17)..(17): Thr or Gln or Ser or Asn
  variant (18)..(18): Thr or Gln or Ser or Asn
  variant (19)..(19): Ala or Met or Val or Leu or Ile
  variant (20)..(20): Trp or Phe
  variant (21)..(21): Thr or Gln or Ser or Asn
  variant (22)..(22): Asp or Glu
  variant (23)..(23): Ala or Met or Val or Leu or Ile
  variant (24)..(24): Asp or Glu
  variant (25)..(25): Thr or Gln or Ser or Asn
  variant (26)..(26): Trp or Phe
  variant (27)..(27): Thr or Gln or Ser or Asn
  variant (28)..(28): Thr or Gln or Ser or Asn or Arg or Lys
  variant (29)..(29): Thr or Gln or Ser or Asn or Arg or Lys
  variant (30)..(30): Thr or Gln or Ser or Asn or Arg or Lys

SEQ ID NO: 143 - protein, 30 aa, artificial; identical to SEQ ID NO: 121
  pattern
  variant (1)..(1): Thr or Gln or Ser or Asn or Arg or Lys
  variant (2)..(2): Thr or Gln or Ser or Asn
  variant (3)..(3): Thr or Gln or Ser or Asn
  variant (4)..(4): Thr or Gln or Ser or Asn or Arg or Lys
  variant (5)..(5): Ala or Met or Val or Leu or Ile
  variant (6)..(6): Asp or Glu
  variant (7)..(7): Thr or Gln or Ser or Asn
  variant (8)..(8): Trp or Phe
  variant (9)..(9): Trp or Phe
  variant (10)..(10): Thr or Gln or Ser or Asn
  variant (11)..(11): Asp or Glu
  variant (12)..(12): Ala or Met or Val or Leu or Ile
  variant (13)..(13): Ala or Met or Val or Leu or Ile
  variant (14)..(14): Thr or Gln or Ser or Asn
  variant (15)..(15): Ala or Met or Val or Leu or Ile
  variant (16)..(16): Ala or Met or Val or Leu or Ile
  variant (17)..(17): Thr or Gln or Ser or Asn
  variant (18)..(18): Thr or Gln or Ser or Asn
  variant (19)..(19): Ala or Met or Val or Leu or Ile
  variant (20)..(20): Trp or Phe
  variant (21)..(21): Thr or Gln or Ser or Asn
  variant (22)..(22): Arg or Lys
  variant (23)..(23): Ala or Met or Val or Leu or Ile
  variant (24)..(24): Arg or Lys
  variant (25)..(25): Thr or Gln or Ser or Asn
  variant (26)..(26): Trp or Phe
  variant (27)..(27): Thr or Gln or Ser or Asn or Arg or Lys
  variant (28)..(28): Thr or Gln or Ser or Asn or Arg or Lys
  variant (29)..(29): Thr or Gln or Ser or Asn or Arg or Lys
  variant (30)..(30): Thr or Gln or Ser or Asn or Arg or Lys

SEQ ID NO: 144 - protein, 30 aa, artificial; identical to SEQ ID NO: 121
  pattern
  variant (1)..(1): Thr or Gln or Ser or Asn or Arg or Lys
  variant (2)..(2): Thr or Gln or Ser or Asn
  variant (3)..(3): Thr or Gln or Ser or Asn
  variant (4)..(4): Thr or Gln or Ser or Asn or Arg or Lys
  variant (5)..(5): Ala or Met or Val or Leu or Ile
  variant (6)..(6): Asp or Glu
  variant (7)..(7): Thr or Gln or Ser or Asn
  variant (8)..(8): Trp or Phe
  variant (9)..(9): Trp or Phe
  variant (10)..(10): Thr or Gln or Ser or Asn
  variant (11)..(11): Asp or Glu
  variant (12)..(12): Ala or Met or Val or Leu or Ile
  variant (13)..(13): Ala or Met or Val or Leu or Ile
  variant (14)..(14): Thr or Gln or Ser or Asn
  variant (15)..(15): Ala or Met or Val or Leu or Ile
  variant (16)..(16): Ala or Met or Val or Leu or Ile
  variant (17)..(17): Arg or Lys
  variant (18)..(18): Thr or Gln or Ser or Asn
  variant (19)..(19): Ala or Met or Val or Leu or Ile
  variant (20)..(20): Trp or Phe
  variant (21)..(21): Thr or Gln or Ser or Asn
  variant (22)..(22): Arg or Lys
  variant (23)..(23): Ala or Met or Val or Leu or Ile
  variant (24)..(24): Arg or Lys
  variant (25)..(25): Arg or Lys
  variant (26)..(26): Trp or Phe
  variant (27)..(27): Thr or Gln or Ser or Asn or Arg or Lys
  variant (28)..(28): Thr or Gln or Ser or Asn or Arg or Lys
  variant (29)..(29): Thr or Gln or Ser or Asn or Arg or Lys
  variant (30)..(30): Thr or Gln or Ser or Asn or Arg or Lys

SEQ ID NO: 145 - protein, 30 aa, artificial; identical to SEQ ID NO: 121
  pattern
  variant (1)..(1): Thr or Gln or Ser or Asn or Arg or Lys
  variant (2)..(2): Thr or Gln or Ser or Asn or Arg or Lys
  variant (3)..(3): Thr or Gln or Ser or Asn or Arg or Lys
  variant (4)..(4): Thr or Gln or Ser or Asn or Arg or Lys
  variant (5)..(5): Ala or Met or Val or Leu or Ile
  variant (6)..(6): Thr or Gln or Ser or Asn
  variant (7)..(7): Arg or Lys
  variant (8)..(8): Trp or Phe
  variant (9)..(9): Trp or Phe
  variant (10)..(10): Arg or Lys
  variant (11)..(11): Thr or Gln or Ser or Asn
  variant (12)..(12): Ala or Met or Val or Leu or Ile
  variant (13)..(13): Ala or Met or Val or Leu or Ile
  variant (14)..(14): Thr or Gln or Ser or Asn
  variant (15)..(15): Ala or Met or Val or Leu or Ile
  variant (16)..(16): Ala or Met or Val or Leu or Ile
  variant (17)..(17): Asp or Glu
  variant (18)..(18): Thr or Gln or Ser or Asn
  variant (19)..(19): Ala or Met or Val or Leu or Ile
  variant (20)..(20): Trp or Phe
  variant (21)..(21): Thr or Gln or Ser or Asn
  variant (22)..(22): Thr or Gln or Ser or Asn
  variant (23)..(23): Ala or Met or Val or Leu or Ile
  variant (24)..(24): Thr or Gln or Ser or Asn
  variant (25)..(25): Asp or Glu
  variant (26)..(26): Trp or Phe
  variant (27)..(27): Thr or Gln or Ser or Asn or Arg or Lys
  variant (28)..(28): Thr or Gln or Ser or Asn
  variant (29)..(29): Thr or Gln or Ser or Asn
  variant (30)..(30): Thr or Gln or Ser or Asn or Arg or Lys

SEQ ID NO: 146 - protein, 30 aa, artificial; identical to SEQ ID NO: 121
  pattern
  variant (1)..(1): Thr or Gln or Ser or Asn or Arg or Lys
  variant (2)..(2): Thr or Gln or Ser or Asn or Arg or Lys
  variant (3)..(3): Thr or Gln or Ser or Asn or Arg or Lys
  variant (4)..(4): Thr or Gln or Ser or Asn or Arg or Lys
  variant (5)..(5): Ala or Met or Val or Leu or Ile
  variant (6)..(6): Arg or Lys
  variant (7)..(7): Arg or Lys
  variant (8)..(8): Trp or Phe
  variant (9)..(9): Trp or Phe
  variant (10)..(10): Arg or Lys
  variant (11)..(11): Arg or Lys
  variant (12)..(12): Ala or Met or Val or Leu or Ile
  variant (13)..(13): Ala or Met or Val or Leu or Ile
  variant (14)..(14): Thr or Gln or Ser or Asn
  variant (15)..(15): Ala or Met or Val or Leu or Ile
  variant (16)..(16): Ala or Met or Val or Leu or Ile
  variant (17)..(17): Asp or Glu
  variant (18)..(18): Thr or Gln or Ser or Asn
  variant (19)..(19): Ala or Met or Val or Leu or Ile
  variant (20)..(20): Trp or Phe
  variant (21)..(21): Thr or Gln or Ser or Asn
  variant (22)..(22): Thr or Gln or Ser or Asn
  variant (23)..(23): Ala or Met or Val or Leu or Ile
  variant (24)..(24): Thr or Gln or Ser or Asn
  variant (25)..(25): Asp or Glu
  variant (26)..(26): Trp or Phe
  variant (27)..(27): Thr or Gln or Ser or Asn or Arg or Lys
  variant (28)..(28): Thr or Gln or Ser or Asn
  variant (29)..(29): Thr or Gln or Ser or Asn
  variant (30)..(30): Thr or Gln or Ser or Asn or Arg or Lys

SEQ ID NO: 147 - protein, 30 aa, artificial; identical to SEQ ID NO: 121
  pattern
  variant (1)..(1): Thr or Gln or Ser or Asn or Arg or Lys
  variant (2)..(2): Thr or Gln or Ser or Asn or Arg or Lys
  variant (3)..(3): Thr or Gln or Ser or Asn
  variant (4)..(4): Thr or Gln or Ser or Asn
  variant (5)..(5): Ala or Met or Val or Leu or Ile
  variant (6)..(6): Thr or Gln or Ser or Asn
  variant (7)..(7): Asp or Glu
  variant (8)..(8): Trp or Phe
  variant (9)..(9): Trp or Phe
  variant (10)..(10): Asp or Glu
  variant (11)..(11): Thr or Gln or Ser or Asn
  variant (12)..(12): Ala or Met or Val or Leu or Ile
  variant (13)..(13): Ala or Met or Val or Leu or Ile
  variant (14)..(14): Thr or Gln or Ser or Asn
  variant (15)..(15): Ala or Met or Val or Leu or Ile
  variant (16)..(16): Ala or Met or Val or Leu or Ile
  variant (17)..(17): Arg or Lys
  variant (18)..(18): Thr or Gln or Ser or Asn
  variant (19)..(19): Ala or Met or Val or Leu or Ile
  variant (20)..(20): Trp or Phe
  variant (21)..(21): Thr or Gln or Ser or Asn
  variant (22)..(22): Thr or Gln or Ser or Asn
  variant (23)..(23): Ala or Met or Val or Leu or Ile
  variant (24)..(24): Thr or Gln or Ser or Asn
  variant (25)..(25): Arg or Lys
  variant (26)..(26): Trp or Phe
  variant (27)..(27): Thr or Gln or Ser or Asn or Arg or Lys
  variant (28)..(28): Thr or Gln or Ser or Asn or Arg or Lys
  variant (29)..(29): Thr or Gln or Ser or Asn or Arg or Lys
  variant (30)..(30): Thr or Gln or Ser or Asn or Arg or Lys

SEQ ID NO: 148 - protein, 30 aa, artificial; identical to SEQ ID NO: 121
  pattern
  variant (1)..(1): Thr or Gln or Ser or Asn or Arg or Lys
  variant (2)..(2): Thr or Gln or Ser or Asn or Arg or Lys
  variant (3)..(3): Thr or Gln or Ser or Asn
  variant (4)..(4): Thr or Gln or Ser or Asn
  variant (5)..(5): Ala or Met or Val or Leu or Ile
  variant (6)..(6): Thr or Gln or Ser or Asn
  variant (7)..(7): Asp or Glu
  variant (8)..(8): Trp or Phe
  variant (9)..(9): Trp or Phe
  variant (10)..(10): Asp or Glu
  variant (11)..(11): Thr or Gln or Ser or Asn
  variant (12)..(12): Ala or Met or Val or Leu or Ile
  variant (13)..(13): Ala or Met or Val or Leu or Ile
  variant (14)..(14): Thr or Gln or Ser or Asn
  variant (15)..(15): Ala or Met or Val or Leu or Ile
  variant (16)..(16): Ala or Met or Val or Leu or Ile
  variant (17)..(17): Arg or Lys
  variant (18)..(18): Thr or Gln or Ser or Asn
  variant (19)..(19): Ala or Met or Val or Leu or Ile
  variant (20)..(20): Trp or Phe
  variant (21)..(21): Thr or Gln or Ser or Asn
  variant (22)..(22): Arg or Lys
  variant (23)..(23): Ala or Met or Val or Leu or Ile
  variant (24)..(24): Arg or Lys
  variant (25)..(25): Arg or Lys
  variant (26)..(26): Trp or Phe
  variant (27)..(27): Thr or Gln or Ser or Asn or Arg or Lys
  variant (28)..(28): Thr or Gln or Ser or Asn or Arg or Lys
  variant (29)..(29): Thr or Gln or Ser or Asn or Arg or Lys
  variant (30)..(30): Thr or Gln or Ser or Asn or Arg or Lys

SEQ ID NO: 149 - protein, 30 aa, artificial; identical to SEQ ID NO: 121
  pattern
  variant (1)..(1): Thr or Gln or Ser or Asn or Arg or Lys
  variant (2)..(2): Thr or Gln or Ser or Asn or Arg or Lys
  variant (3)..(3): Thr or Gln or Ser or Asn or Arg or Lys
  variant (4)..(4): Thr or Gln or Ser or Asn or Arg or Lys
  variant (5)..(5): Ala or Met or Val or Leu or Ile
  variant (6)..(6): Thr or Gln or Ser or Asn
  variant (7)..(7): Thr or Gln or Ser or Asn
  variant (8)..(8): Trp or Phe
  variant (9)..(9): Trp or Phe
  variant (10)..(10): Arg or Lys
  variant (11)..(11): Arg or Lys
  variant (12)..(12): Ala or Met or Val or Leu or Ile
  variant (13)..(13): Ala or Met or Val or Leu or Ile
  variant (14)..(14): Thr or Gln or Ser or Asn
  variant (15)..(15): Ala or Met or Val or Leu or Ile
  variant (16)..(16): Ala or Met or Val or Leu or Ile
  variant (17)..(17): Asp or Glu
  variant (18)..(18): Thr or Gln or Ser or Asn
  variant (19)..(19): Ala or Met or Val or Leu or Ile
  variant (20)..(20): Trp or Phe
  variant (21)..(21): Thr or Gln or Ser or Asn
  variant (22)..(22): Asp or Glu
  variant (23)..(23): Ala or Met or Val or Leu or Ile
  variant (24)..(24): Thr or Gln or Ser or Asn
  variant (25)..(25): Thr or Gln or Ser or Asn
  variant (26)..(26): Trp or Phe
  variant (27)..(27): Thr or Gln or Ser or Asn or Arg or Lys
  variant (28)..(28): Thr or Gln or Ser or Asn or Arg or Lys
  variant (29)..(29): Thr or Gln or Ser or Asn or Arg or Lys
  variant (30)..(30): Thr or Gln or Ser or Asn or Arg or Lys

SEQ ID NO: 150 - protein, 30 aa, artificial; identical to SEQ ID NO: 121
  pattern
  variant (1)..(1): Thr or Gln or Ser or Asn or Arg or Lys
  variant (2)..(2): Thr or Gln or Ser or Asn or Arg or Lys
  variant (3)..(3): Thr or Gln or Ser or Asn or Arg or Lys
  variant (4)..(4): Thr or Gln or Ser or Asn or Arg or Lys
  variant (5)..(5): Ala or Met or Val or Leu or Ile
  variant (6)..(6): Arg or Lys
  variant (7)..(7): Arg or Lys
  variant (8)..(8): Trp or Phe
  variant (9)..(9): Trp or Phe
  variant (10)..(10): Arg or Lys
  variant (11)..(11): Arg or Lys
  variant (12)..(12): Ala or Met or Val or Leu or Ile
  variant (13)..(13): Ala or Met or Val or Leu or Ile
  variant (14)..(14): Thr or Gln or Ser or Asn
  variant (15)..(15): Ala or Met or Val or Leu or Ile
  variant (16)..(16): Ala or Met or Val or Leu or Ile
  variant (17)..(17): Asp or Glu
  variant (18)..(18): Thr or Gln or Ser or Asn
  variant (19)..(19): Ala or Met or Val or Leu or Ile
  variant (20)..(20): Trp or Phe
  variant (21)..(21): Thr or Gln or Ser or Asn
  variant (22)..(22): Asp or Glu
  variant (23)..(23): Ala or Met or Val or Leu or Ile
  variant (24)..(24): Thr or Gln or Ser or Asn
  variant (25)..(25): Thr or Gln or Ser or Asn
  variant (26)..(26): Trp or Phe
  variant (27)..(27): Thr or Gln or Ser or Asn or Arg or Lys
  variant (28)..(28): Thr or Gln or Ser or Asn or Arg or Lys
  variant (29)..(29): Thr or Gln or Ser or Asn or Arg or Lys
  variant (30)..(30): Thr or Gln or Ser or Asn or Arg or Lys

SEQ ID NO: 151 - protein, 30 aa, artificial; identical to SEQ ID NO: 121
  pattern
  variant (1)..(1): Thr or Gln or Ser or Asn or Arg or Lys
  variant (2)..(2): Thr or Gln or Ser or Asn or Arg or Lys
  variant (3)..(3): Thr or Gln or Ser or Asn or Arg or Lys
  variant (4)..(4): Thr or Gln or Ser or Asn or Arg or Lys
  variant (5)..(5): Ala or Met or Val or Leu or Ile
  variant (6)..(6): Thr or Gln or Ser or Asn
  variant (7)..(7): Thr or Gln or Ser or Asn
  variant (8)..(8): Trp or Phe
  variant (9)..(9): Trp or Phe
  variant (10)..(10): Asp or Glu
  variant (11)..(11): Asp or Glu
  variant (12)..(12): Ala or Met or Val or Leu or Ile
  variant (13)..(13): Ala or Met or Val or Leu or Ile
  variant (14)..(14): Thr or Gln or Ser or Asn
  variant (15)..(15): Ala or Met or Val or Leu or Ile
  variant (16)..(16): Ala or Met or Val or Leu or Ile
  variant (17)..(17): Arg or Lys
  variant (18)..(18): Thr or Gln or Ser or Asn
  variant (19)..(19): Ala or Met or Val or Leu or Ile
  variant (20)..(20): Trp or Phe
  variant (21)..(21): Thr or Gln or Ser or Asn
  variant (22)..(22): Arg or Lys
  variant (23)..(23): Ala or Met or Val or Leu or Ile
  variant (24)..(24): Thr or Gln or Ser or Asn
  variant (25)..(25): Thr or Gln or Ser or Asn
  variant (26)..(26): Trp or Phe
  variant (27)..(27): Thr or Gln or Ser or Asn or Arg or Lys
  variant (28)..(28): Thr or Gln or Ser or Asn or Arg or Lys
  variant (29)..(29): Thr or Gln or Ser or Asn or Arg or Lys
  variant (30)..(30): Thr or Gln or Ser or Asn or Arg or Lys

SEQ ID NO: 152 - protein, 30 aa, artificial; identical to SEQ ID NO: 121
  pattern
  variant (1)..(1): Thr or Gln or Ser or Asn or Arg or Lys
  variant (2)..(2): Thr or Gln or Ser or Asn or Arg or Lys
  variant (3)..(3): Thr or Gln or Ser or Asn or Arg or Lys
  variant (4)..(4): Thr or Gln or Ser or Asn or Arg or Lys
  variant (5)..(5): Ala or Met or Val or Leu or Ile
  variant (6)..(6): Thr or Gln or Ser or Asn
  variant (7)..(7): Thr or Gln or Ser or Asn
  variant (8)..(8): Trp or Phe
  variant (9)..(9): Trp or Phe
  variant (10)..(10): Asp or Glu
  variant (11)..(11): Asp or Glu
  variant (12)..(12): Ala or Met or Val or Leu or Ile
  variant (13)..(13): Ala or Met or Val or Leu or Ile
  variant (14)..(14): Thr or Gln or Ser or Asn
  variant (15)..(15): Ala or Met or Val or Leu or Ile
  variant (16)..(16): Ala or Met or Val or Leu or Ile
  variant (17)..(17): Arg or Lys
  variant (18)..(18): Thr or Gln or Ser or Asn
  variant (19)..(19): Ala or Met or Val or Leu or Ile
  variant (20)..(20): Trp or Phe
  variant (21)..(21): Thr or Gln or Ser or Asn
  variant (22)..(22): Arg or Lys
  variant (23)..(23): Ala or Met or Val or Leu or Ile
  variant (24)..(24): Arg or Lys
  variant (25)..(25): Arg or Lys
  variant (26)..(26): Trp or Phe
  variant (27)..(27): Thr or Gln or Ser or Asn or Arg or Lys
  variant (28)..(28): Thr or Gln or Ser or Asn or Arg or Lys
  variant (29)..(29): Thr or Gln or Ser or Asn or Arg or Lys
  variant (30)..(30): Thr or Gln or Ser or Asn or Arg or Lys

SEQ ID NO: 153 - protein, 30 aa, artificial; identical to SEQ ID NO: 121
  pattern
  variant (1)..(1): Thr or Gln or Ser or Asn or Arg or Lys
  variant (2)..(2): Thr or Gln or Ser or Asn or Arg or Lys
  variant (3)..(3): Thr or Gln or Ser or Asn or Arg or Lys
  variant (4)..(4): Thr or Gln or Ser or Asn or Arg or Lys
  variant (5)..(5): Ala or Met or Val or Leu or Ile
  variant (6)..(6): Arg or Lys
  variant (7)..(7): Arg or Lys
  variant (8)..(8): Ala or Met or Val or Leu or Ile
  variant (9)..(9): Ala or Met or Val or Leu or Ile
  variant (10)..(10): Arg or Lys
  variant (11)..(11): Arg or Lys
  variant (12)..(12): Ala or Met or Val or Leu or Ile
  variant (13)..(13): Trp or Phe
  variant (14)..(14): Thr or Gln or Ser or Asn
  variant (15)..(15): Trp or Phe
  variant (16)..(16): Ala or Met or Val or Leu or Ile
  variant (17)..(17): Asp or Glu
  variant (18)..(18): Thr or Gln or Ser or Asn
  variant (19)..(19): Ala or Met or Val or Leu or Ile
  variant (20)..(20): Asp or Glu
  variant (21)..(21): Thr or Gln or Ser or Asn
  variant (22)..(22): Asp or Glu
  variant (23)..(23): Ala or Met or Val or Leu or Ile
  variant (24)..(24): Thr or Gln or Ser or Asn
  variant (25)..(25): Asp or Glu
  variant (26)..(26): Ala or Met or Val or Leu or Ile
  variant (27)..(27): Thr or Gln or Ser or Asn or Arg or Lys
  variant (28)..(28): Thr or Gln or Ser or Asn or Arg or Lys
  variant (29)..(29): Thr or Gln or Ser or Asn or Arg or Lys
  variant (30)..(30): Thr or Gln or Ser or Asn or Arg or Lys

SEQ ID NO: 154 - protein, 30 aa, artificial; identical to SEQ ID NO: 121
  pattern
  variant (1)..(1): Thr or Gln or Ser or Asn or Arg or Lys
  variant (2)..(2): Thr or Gln or Ser or Asn or Arg or Lys
  variant (3)..(3): Thr or Gln or Ser or Asn or Arg or Lys
  variant (4)..(4): Thr or Gln or Ser or Asn or Arg or Lys
  variant (5)..(5): Ala or Met or Val or Leu or Ile
  variant (6)..(6): Asp or Glu
  variant (7)..(7): Asp or Glu
  variant (8)..(8): Ala or Met or Val or Leu or Ile
  variant (9)..(9): Ala or Met or Val or Leu or Ile
  variant (10)..(10): Asp or Glu
  variant (11)..(11): Asp or Glu
  variant (12)..(12): Ala or Met or Val or Leu or Ile
  variant (13)..(13): Trp or Phe
  variant (14)..(14): Thr or Gln or Ser or Asn
  variant (15)..(15): Trp or Phe
  variant (16)..(16): Ala or Met or Val or Leu or Ile
  variant (17)..(17): Arg or Lys
  variant (18)..(18): Thr or Gln or Ser or Asn
  variant (19)..(19): Ala or Met or Val or Leu or Ile
  variant (20)..(20): Arg or Lys
  variant (21)..(21): Thr or Gln or Ser or Asn
  variant (22)..(22): Arg or Lys
  variant (23)..(23): Ala or Met or Val or Leu or Ile
  variant (24)..(24): Thr or Gln or Ser or Asn
  variant (25)..(25): Arg or Lys
  variant (26)..(26): Ala or Met or Val or Leu or Ile
  variant (27)..(27): Thr or Gln or Ser or Asn or Arg or Lys
  variant (28)..(28): Thr or Gln or Ser or Asn or Arg or Lys
  variant (29)..(29): Thr or Gln or Ser or Asn or Arg or Lys
  variant (30)..(30): Thr or Gln or Ser or Asn or Arg or Lys

SEQ ID NO: 155 - protein, 30 aa, artificial; identical to SEQ ID NO: 121
  pattern
  variant (1)..(1): Thr or Gln or Ser or Asn or Arg or Lys
  variant (2)..(2): Thr or Gln or Ser or Asn or Arg or Lys
  variant (3)..(3): Thr or Gln or Ser or Asn or Arg or Lys
  variant (4)..(4): Thr or Gln or Ser or Asn or Arg or Lys
  variant (5)..(5): Ala or Met or Val or Leu or Ile
  variant (6)..(6): Arg or Lys
  variant (7)..(7): Arg or Lys
  variant (8)..(8): Ala or Met or Val or Leu or Ile
  variant (9)..(9): Ala or Met or Val or Leu or Ile
  variant (10)..(10): Arg or Lys
  variant (11)..(11): Arg or Lys
  variant (12)..(12): Ala or Met or Val or Leu or Ile
  variant (13)..(13): Trp or Phe
  variant (14)..(14): Thr or Gln or Ser or Asn
  variant (15)..(15): Trp or Phe
  variant (16)..(16): Ala or Met or Val or Leu or Ile
  variant (17)..(17): Asp or Glu
  variant (18)..(18): Thr or Gln or Ser or Asn
  variant (19)..(19): Ala or Met or Val or Leu or Ile
  variant (20)..(20): Ala or Met or Val or Leu or Ile
  variant (21)..(21): Asp or Glu
  variant (22)..(22): Asp or Glu
  variant (23)..(23): Ala or Met or Val or Leu or Ile
  variant (24)..(24): Thr or Gln or Ser or Asn
  variant (25)..(25): Asp or Glu
  variant (26)..(26): Ala or Met or Val or Leu or Ile
  variant (27)..(27): Thr or Gln or Ser or Asn or Arg or Lys
  variant (28)..(28): Thr or Gln or Ser or Asn or Arg or Lys
  variant (29)..(29): Thr or Gln or Ser or Asn or Arg or Lys
  variant (30)..(30): Thr or Gln or Ser or Asn or Arg or Lys

SEQ ID NO: 156 - protein, 30 aa, artificial; identical to SEQ ID NO: 121
  pattern
  variant (1)..(1): Thr or Gln or Ser or Asn or Arg or Lys
  variant (2)..(2): Thr or Gln or Ser or Asn or Arg or Lys
  variant (3)..(3): Thr or Gln or Ser or Asn or Arg or Lys
  variant (4)..(4): Thr or Gln or Ser or Asn or Arg or Lys
  variant (5)..(5): Ala or Met or Val or Leu or Ile
  variant (6)..(6): Asp or Glu
  variant (7)..(7): Asp or Glu
  variant (8)..(8): Ala or Met or Val or Leu or Ile
  variant (9)..(9): Ala or Met or Val or Leu or Ile
  variant (10)..(10): Asp or Glu
  variant (11)..(11): Asp or Glu
  variant (12)..(12): Ala or Met or Val or Leu or Ile
  variant (13)..(13): Trp or Phe
  variant (14)..(14): Thr or Gln or Ser or Asn
  variant (15)..(15): Trp or Phe
  variant (16)..(16): Ala or Met or Val or Leu or Ile
  variant (17)..(17): Arg or Lys
  variant (18)..(18): Thr or Gln or Ser or Asn
  variant (19)..(19): Ala or Met or Val or Leu or Ile
  variant (20)..(20): Ala or Met or Val or Leu or Ile
  variant (21)..(21): Arg or Lys
  variant (22)..(22): Arg or Lys
  variant (23)..(23): Ala or Met or Val or Leu or Ile
  variant (24)..(24): Thr or Gln or Ser or Asn
  variant (25)..(25): Arg or Lys
  variant (26)..(26): Ala or Met or Val or Leu or Ile
  variant (27)..(27): Thr or Gln or Ser or Asn or Arg or Lys
  variant (28)..(28): Thr or Gln or Ser or Asn or Arg or Lys
  variant (29)..(29): Thr or Gln or Ser or Asn or Arg or Lys
  variant (30)..(30): Thr or Gln or Ser or Asn or Arg or Lys

SEQ ID NO: 157 - protein, 30 aa, artificial; identical to SEQ ID NO: 121
  pattern
  variant (1)..(1): Thr or Gln or Ser or Asn or Arg or Lys
  variant (2)..(2): Thr or Gln or Ser or Asn or Arg or Lys
  variant (3)..(3): Thr or Gln or Ser or Asn or Arg or Lys
  variant (4)..(4): Thr or Gln or Ser or Asn or Arg or Lys
  variant (5)..(5): Ala or Met or Val or Leu or Ile
  variant (6)..(6): Arg or Lys
  variant (7)..(7): Arg or Lys
  variant (8)..(8): Ala or Met or Val or Leu or Ile
  variant (9)..(9): Ala or Met or Val or Leu or Ile
  variant (10)..(10): Arg or Lys
  variant (11)..(11): Arg or Lys
  variant (12)..(12): Ala or Met or Val or Leu or Ile
  variant (13)..(13): Trp or Phe
  variant (14)..(14): Thr or Gln or Ser or Asn
  variant (15)..(15): Trp or Phe
  variant (16)..(16): Ala or Met or Val or Leu or Ile
  variant (17)..(17): Asp or Glu
  variant (18)..(18): Thr or Gln or Ser or Asn
  variant (19)..(19): Ala or Met or Val or Leu or Ile
  variant (20)..(20): Ala or Met or Val or Leu or Ile
  variant (21)..(21): Thr or Gln or Ser or Asn
  variant (22)..(22): Asp or Glu
  variant (23)..(23): Ala or Met or Val or Leu or Ile
  variant (24)..(24): Asp or Glu
  variant (25)..(25): Asp or Glu
  variant (26)..(26): Ala or Met or Val or Leu or Ile
  variant (27)..(27): Thr or Gln or Ser or Asn or Arg or Lys
  variant (28)..(28): Thr or Gln or Ser or Asn or Arg or Lys
  variant (29)..(29): Thr or Gln or Ser or Asn or Arg or Lys
  variant (30)..(30): Thr or Gln or Ser or Asn or Arg or Lys

SEQ ID NO: 158 - protein, 30 aa, artificial; identical to SEQ ID NO: 121
  pattern
  variant (1)..(1): Thr or Gln or Ser or Asn or Arg or Lys
  variant (2)..(2): Thr or Gln or Ser or Asn or Arg or Lys
  variant (3)..(3): Thr or Gln or Ser or Asn or Arg or Lys
  variant (4)..(4): Thr or Gln or Ser or Asn or Arg or Lys
  variant (5)..(5): Ala or Met or Val or Leu or Ile
  variant (6)..(6): Asp or Glu
  variant (7)..(7): Asp or Glu
  variant (8)..(8): Ala or Met or Val or Leu or Ile
  variant (9)..(9): Ala or Met or Val or Leu or Ile
  variant (10)..(10): Asp or Glu
  variant (11)..(11): Asp or Glu
  variant (12)..(12): Ala or Met or Val or Leu or Ile
  variant (13)..(13): Trp or Phe
  variant (14)..(14): Thr or Gln or Ser or Asn
  variant (15)..(15): Trp or Phe
  variant (16)..(16): Ala or Met or Val or Leu or Ile
  variant (17)..(17): Arg or Lys
  variant (18)..(18): Thr or Gln or Ser or Asn
  variant (19)..(19): Ala or Met or Val or Leu or Ile
  variant (20)..(20): Ala or Met or Val or Leu or Ile
  variant (21)..(21): Thr or Gln or Ser or Asn
  variant (22)..(22): Arg or Lys
  variant (23)..(23): Ala or Met or Val or Leu or Ile
  variant (24)..(24): Arg or Lys
  variant (25)..(25): Arg or Lys
  variant (26)..(26): Ala or Met or Val or Leu or Ile
  variant (27)..(27): Thr or Gln or Ser or Asn or Arg or Lys
  variant (28)..(28): Thr or Gln or Ser or Asn or Arg or Lys
  variant (29)..(29): Thr or Gln or Ser or Asn or Arg or Lys
  variant (30)..(30): Thr or Gln or Ser or Asn or Arg or Lys

SEQ ID NO: 159 - protein, 30 aa, artificial; identical to SEQ ID NO: 121
  pattern
  variant (1)..(1): Thr or Gln or Ser or Asn or Arg or Lys
  variant (2)..(2): Thr or Gln or Ser or Asn or Arg or Lys
  variant (3)..(3): Thr or Gln or Ser or Asn or Arg or Lys
  variant (4)..(4): Thr or Gln or Ser or Asn or Arg or Lys
  variant (5)..(5): Ala or Met or Val or Leu or Ile
  variant (6)..(6): Arg or Lys
  variant (7)..(7): Arg or Lys
  variant (8)..(8): Ala or Met or Val or Leu or Ile
  variant (9)..(9): Ala or Met or Val or Leu or Ile
  variant (10)..(10): Arg or Lys
  variant (11)..(11): Arg or Lys
  variant (12)..(12): Ala or Met or Val or Leu or Ile
  variant (13)..(13): Trp or Phe
  variant (14)..(14): Thr or Gln or Ser or Asn
  variant (15)..(15): Trp or Phe
  variant (16)..(16): Ala or Met or Val or Leu or Ile
  variant (17)..(17): Thr or Gln or Ser or Asn
  variant (18)..(18): Thr or Gln or Ser or Asn
  variant (19)..(19): Ala or Met or Val or Leu or Ile
  variant (20)..(20): Asp or Glu
  variant (21)..(21): Asp or Glu
  variant (22)..(22): Asp or Glu
  variant (23)..(23): Ala or Met or Val or Leu or Ile
  variant (24)..(24): Thr or Gln or Ser or Asn
  variant (25)..(25): Asp or Glu
  variant (26)..(26): Ala or Met or Val or Leu or Ile
  variant (27)..(27): Thr or Gln or Ser or Asn or Arg or Lys
  variant (28)..(28): Thr or Gln or Ser or Asn or Arg or Lys
  variant (29)..(29): Thr or Gln or Ser or Asn or Arg or Lys
  variant (30)..(30): Thr or Gln or Ser or Asn or Arg or Lys

SEQ ID NO: 160 - protein, 30 aa, artificial; identical to SEQ ID NO: 121
  pattern
  variant (1)..(1): Thr or Gln or Ser or Asn or Arg or Lys
  variant (2)..(2): Thr or Gln or Ser or Asn or Arg or Lys
  variant (3)..(3): Thr or Gln or Ser or Asn or Arg or Lys
  variant (4)..(4): Thr or Gln or Ser or Asn or Arg or Lys
  variant (5)..(5): Ala or Met or Val or Leu or Ile
  variant (6)..(6): Asp or Glu
  variant (7)..(7): Asp or Glu
  variant (8)..(8): Ala or Met or Val or Leu or Ile
  variant (9)..(9): Ala or Met or Val or Leu or Ile
  variant (10)..(10): Asp or Glu
  variant (11)..(11): Asp or Glu
  variant (12)..(12): Ala or Met or Val or Leu or Ile
  variant (13)..(13): Trp or Phe
  variant (14)..(14): Thr or Gln or Ser or Asn
  variant (15)..(15): Trp or Phe
  variant (16)..(16): Ala or Met or Val or Leu or Ile
  variant (17)..(17): Thr or Gln or Ser or Asn
  variant (18)..(18): Thr or Gln or Ser or Asn
  variant (19)..(19): Ala or Met or Val or Leu or Ile
  variant (20)..(20): Arg or Lys
  variant (21)..(21): Arg or Lys
  variant (22)..(22): Arg or Lys
  variant (23)..(23): Ala or Met or Val or Leu or Ile
  variant (24)..(24): Thr or Gln or Ser or Asn
  variant (25)..(25): Arg or Lys
  variant (26)..(26): Ala or Met or Val or Leu or Ile
  variant (27)..(27): Thr or Gln or Ser or Asn or Arg or Lys
  variant (28)..(28): Thr or Gln or Ser or Asn or Arg or Lys
  variant (29)..(29): Thr or Gln or Ser or Asn or Arg or Lys
  variant (30)..(30): Thr or Gln or Ser or Asn or Arg or Lys

SEQ ID NO: 161 - protein, 30 aa, artificial; identical to SEQ ID NO: 121
  pattern
  variant (1)..(1): Thr or Gln or Ser or Asn or Arg or Lys
  variant (2)..(2): Thr or Gln or Ser or Asn or Arg or Lys
  variant (3)..(3): Thr or Gln or Ser or Asn or Arg or Lys
  variant (4)..(4): Thr or Gln or Ser or Asn or Arg or Lys
  variant (5)..(5): Ala or Met or Val or Leu or Ile
  variant (6)..(6): Arg or Lys
  variant (7)..(7): Arg or Lys
  variant (8)..(8): Ala or Met or Val or Leu or Ile
  variant (9)..(9): Ala or Met or Val or Leu or Ile
  variant (10)..(10): Arg or Lys
  variant (11)..(11): Arg or Lys
  variant (12)..(12): Ala or Met or Val or Leu or Ile
  variant (13)..(13): Trp or Phe
  variant (14)..(14): Thr or Gln or Ser or Asn
  variant (15)..(15): Trp or Phe
  variant (16)..(16): Ala or Met or Val or Leu or Ile
  variant (17)..(17): Thr or Gln or Ser or Asn
  variant (18)..(18): Thr or Gln or Ser or Asn
  variant (19)..(19): Ala or Met or Val or Leu or Ile
  variant (20)..(20): Asp or Glu
  variant (21)..(21): Thr or Gln or Ser or Asn
  variant (22)..(22): Asp or Glu
  variant (23)..(23): Ala or Met or Val or Leu or Ile
  variant (24)..(24): Asp or Glu
  variant (25)..(25): Asp or Glu
  variant (26)..(26): Ala or Met or Val or Leu or Ile
  variant (27)..(27): Thr or Gln or Ser or Asn or Arg or Lys
  variant (28)..(28): Thr or Gln or Ser or Asn or Arg or Lys
  variant (29)..(29): Thr or Gln or Ser or Asn or Arg or Lys
  variant (30)..(30): Thr or Gln or Ser or Asn or Arg or Lys

SEQ ID NO: 162 - protein, 30 aa, artificial; identical to SEQ ID NO: 121
  pattern
  variant (1)..(1): Thr or Gln or Ser or Asn or Arg or Lys
  variant (2)..(2): Thr or Gln or Ser or Asn or Arg or Lys
  variant (3)..(3): Thr or Gln or Ser or Asn or Arg or Lys
  variant (4)..(4): Thr or Gln or Ser or Asn or Arg or Lys
  variant (5)..(5): Ala or Met or Val or Leu or Ile
  variant (6)..(6): Asp or Glu
  variant (7)..(7): Asp or Glu
  variant (8)..(8): Ala or Met or Val or Leu or Ile
  variant (9)..(9): Ala or Met or Val or Leu or Ile
  variant (10)..(10): Asp or Glu
  variant (11)..(11): Asp or Glu
  variant (12)..(12): Ala or Met or Val or Leu or Ile
  variant (13)..(13): Trp or Phe
  variant (14)..(14): Thr or Gln or Ser or Asn
  variant (15)..(15): Trp or Phe
  variant (16)..(16): Ala or Met or Val or Leu or Ile
  variant (17)..(17): Thr or Gln or Ser or Asn
  variant (18)..(18): Thr or Gln or Ser or Asn
  variant (19)..(19): Ala or Met or Val or Leu or Ile
  variant (20)..(20): Arg or Lys
  variant (21)..(21): Thr or Gln or Ser or Asn
  variant (22)..(22): Arg or Lys
  variant (23)..(23): Ala or Met or Val or Leu or Ile
  variant (24)..(24): Arg or Lys
  variant (25)..(25): Arg or Lys
  variant (26)..(26): Ala or Met or Val or Leu or Ile
  variant (27)..(27): Thr or Gln or Ser or Asn or Arg or Lys
  variant (28)..(28): Thr or Gln or Ser or Asn or Arg or Lys
  variant (29)..(29): Thr or Gln or Ser or Asn or Arg or Lys
  variant (30)..(30): Thr or Gln or Ser or Asn or Arg or Lys

SEQ ID NO: 163 - protein, 30 aa, artificial; identical to SEQ ID NO: 121
  pattern
  variant (1)..(1): Thr or Gln or Ser or Asn or Arg or Lys
  variant (2)..(2): Thr or Gln or Ser or Asn or Arg or Lys
  variant (3)..(3): Thr or Gln or Ser or Asn or Arg or Lys
  variant (4)..(4): Thr or Gln or Ser or Asn or Arg or Lys
  variant (5)..(5): Ala or Met or Val or Leu or Ile
  variant (6)..(6): Arg or Lys
  variant (7)..(7): Arg or Lys
  variant (8)..(8): Ala or Met or Val or Leu or Ile
  variant (9)..(9): Ala or Met or Val or Leu or Ile
  variant (10)..(10): Arg or Lys
  variant (11)..(11): Arg or Lys
  variant (12)..(12): Ala or Met or Val or Leu or Ile
  variant (13)..(13): Trp or Phe
  variant (14)..(14): Thr or Gln or Ser or Asn
  variant (15)..(15): Trp or Phe
  variant (16)..(16): Ala or Met or Val or Leu or Ile
  variant (17)..(17): Thr or Gln or Ser or Asn
  variant (18)..(18): Thr or Gln or Ser or Asn
  variant (19)..(19): Ala or Met or Val or Leu or Ile
  variant (20)..(20): Ala or Met or Val or Leu or Ile
  variant (21)..(21): Asp or Glu
  variant (22)..(22): Asp or Glu
  variant (23)..(23): Ala or Met or Val or Leu or Ile
  variant (24)..(24): Asp or Glu
  variant (25)..(25): Asp or Glu
  variant (26)..(26): Ala or Met or Val or Leu or Ile
  variant (27)..(27): Thr or Gln or Ser or Asn or Arg or Lys
  variant (28)..(28): Thr or Gln or Ser or Asn or Arg or Lys
  variant (29)..(29): Thr or Gln or Ser or Asn or Arg or Lys
  variant (30)..(30): Thr or Gln or Ser or Asn or Arg or Lys

SEQ ID NO: 164 - protein, 30 aa, artificial; identical to SEQ ID NO: 121
  pattern
  variant (1)..(1): Thr or Gln or Ser or Asn or Arg or Lys
  variant (2)..(2): Thr or Gln or Ser or Asn or Arg or Lys
  variant (3)..(3): Thr or Gln or Ser or Asn or Arg or Lys
  variant (4)..(4): Thr or Gln or Ser or Asn or Arg or Lys
  variant (5)..(5): Ala or Met or Val or Leu or Ile
  variant (6)..(6): Asp or Glu
  variant (7)..(7): Asp or Glu
  variant (8)..(8): Ala or Met or Val or Leu or Ile
  variant (9)..(9): Ala or Met or Val or Leu or Ile
  variant (10)..(10): Asp or Glu
  variant (11)..(11): Asp or Glu
  variant (12)..(12): Ala or Met or Val or Leu or Ile
  variant (13)..(13): Trp or Phe
  variant (14)..(14): Thr or Gln or Ser or Asn
  variant (15)..(15): Trp or Phe
  variant (16)..(16): Ala or Met or Val or Leu or Ile
  variant (17)..(17): Thr or Gln or Ser or Asn
  variant (18)..(18): Thr or Gln or Ser or Asn
  variant (19)..(19): Ala or Met or Val or Leu or Ile
  variant (20)..(20): Ala or Met or Val or Leu or Ile
  variant (21)..(21): Arg or Lys
  variant (22)..(22): Arg or Lys
  variant (23)..(23): Ala or Met or Val or Leu or Ile
  variant (24)..(24): Arg or Lys
  variant (25)..(25): Arg or Lys
  variant (26)..(26): Ala or Met or Val or Leu or Ile
  variant (27)..(27): Thr or Gln or Ser or Asn or Arg or Lys
  variant (28)..(28): Thr or Gln or Ser or Asn or Arg or Lys
  variant (29)..(29): Thr or Gln or Ser or Asn or Arg or Lys
  variant (30)..(30): Thr or Gln or Ser or Asn or Arg or Lys

SEQ ID NO: 165 - protein, 30 aa, artificial; identical to SEQ ID NO: 121
  pattern
  variant (1)..(1): Thr or Gln or Ser or Asn or Arg or Lys
  variant (2)..(2): Thr or Gln or Ser or Asn or Arg or Lys
  variant (3)..(3): Thr or Gln or Ser or Asn or Arg or Lys
  variant (4)..(4): Thr or Gln or Ser or Asn or Arg or Lys
  variant (5)..(5): Ala or Met or Val or Leu or Ile
  variant (6)..(6): Asp or Glu
  variant (7)..(7): Asp or Glu
  variant (8)..(8): Ala or Met or Val or Leu or Ile
  variant (9)..(9): Ala or Met or Val or Leu or Ile
  variant (10)..(10): Asp or Glu
  variant (11)..(11): Asp or Glu
  variant (12)..(12): Ala or Met or Val or Leu or Ile
  variant (13)..(13): Trp or Phe
  variant (14)..(14): Thr or Gln or Ser or Asn
  variant (15)..(15): Trp or Phe
  variant (16)..(16): Ala or Met or Val or Leu or Ile
  variant (17)..(17): Arg or Lys
  variant (18)..(18): Thr or Gln or Ser or Asn
  variant (19)..(19): Ala or Met or Val or Leu or Ile
  variant (20)..(20): Arg or Lys
  variant (21)..(21): Arg or Lys
  variant (22)..(22): Arg or Lys
  variant (23)..(23): Ala or Met or Val or Leu or Ile
  variant (24)..(24): Arg or Lys
  variant (25)..(25): Arg or Lys
  variant (26)..(26): Ala or Met or Val or Leu or Ile
  variant (27)..(27): Thr or Gln or Ser or Asn or Arg or Lys
  variant (28)..(28): Thr or Gln or Ser or Asn or Arg or Lys
  variant (29)..(29): Thr or Gln or Ser or Asn or Arg or Lys
  variant (30)..(30): Thr or Gln or Ser or Asn or Arg or Lys

SEQ ID NO: 166 - protein, 30 aa, artificial; identical to SEQ ID NO: 121
  pattern
  variant (1)..(1): Thr or Gln or Ser or Asn or Arg or Lys
  variant (2)..(2): Thr or Gln or Ser or Asn or Arg or Lys
  variant (3)..(3): Thr or Gln or Ser or Asn or Arg or Lys
  variant (4)..(4): Thr or Gln or Ser or Asn or Arg or Lys
  variant (5)..(5): Ala or Met or Val or Leu or Ile
  variant (6)..(6): Arg or Lys
  variant (7)..(7): Arg or Lys
  variant (8)..(8): Trp or Phe
  variant (9)..(9): Trp or Phe
  variant (10)..(10): Arg or Lys
  variant (11)..(11): Arg or Lys
  variant (12)..(12): Ala or Met or Val or Leu or Ile
  variant (13)..(13): Ala or Met or Val or Leu or Ile
  variant (14)..(14): Thr or Gln or Ser or Asn
  variant (15)..(15): Ala or Met or Val or Leu or Ile
  variant (16)..(16): Ala or Met or Val or Leu or Ile
  variant (17)..(17): Asp or Glu
  variant (18)..(18): Thr or Gln or Ser or Asn
  variant (19)..(19): Ala or Met or Val or Leu or Ile
  variant (20)..(20): Trp or Phe
  variant (21)..(21): Asp or Glu
  variant (22)..(22): Asp or Glu
  variant (23)..(23): Ala or Met or Val or Leu or Ile
  variant (24)..(24): Thr or Gln or Ser or Asn
  variant (25)..(25): Asp or Glu
  variant (26)..(26): Trp or Phe
  variant (27)..(27): Thr or Gln or Ser or Asn or Arg or Lys
  variant (28)..(28): Thr or Gln or Ser or Asn or Arg or Lys
  variant (29)..(29): Thr or Gln or Ser or Asn or Arg or Lys
  variant (30)..(30): Thr or Gln or Ser or Asn or Arg or Lys

SEQ ID NO: 167 - protein, 30 aa, artificial; identical to SEQ ID NO: 121
  pattern
  variant (1)..(1): Thr or Gln or Ser or Asn or Arg or Lys
  variant (2)..(2): Thr or Gln or Ser or Asn or Arg or Lys
  variant (3)..(3): Thr or Gln or Ser or Asn or Arg or Lys
  variant (4)..(4): Thr or Gln or Ser or Asn or Arg or Lys
  variant (5)..(5): Ala or Met or Val or Leu or Ile
  variant (6)..(6): Asp or Glu
  variant (7)..(7): Asp or Glu
  variant (8)..(8): Trp or Phe
  variant (9)..(9): Trp or Phe
  variant (10)..(10): Asp or Glu
  variant (11)..(11): Asp or Glu
  variant (12)..(12): Ala or Met or Val or Leu or Ile
  variant (13)..(13): Ala or Met or Val or Leu or Ile
  variant (14)..(14): Thr or Gln or Ser or Asn
  variant (15)..(15): Ala or Met or Val or Leu or Ile
  variant (16)..(16): Ala or Met or Val or Leu or Ile
  variant (17)..(17): Arg or Lys
  variant (18)..(18): Thr or Gln or Ser or Asn
  variant (19)..(19): Ala or Met or Val or Leu or Ile
  variant (20)..(20): Trp or Phe
  variant (21)..(21): Arg or Lys
  variant (22)..(22): Arg or Lys
  variant (23)..(23): Ala or Met or Val or Leu or Ile
  variant (24)..(24): Thr or Gln or Ser or Asn
  variant (25)..(25): Arg or Lys
  variant (26)..(26): Trp or Phe
  variant (27)..(27): Thr or Gln or Ser or Asn or Arg or Lys
  variant (28)..(28): Thr or Gln or Ser or Asn or Arg or Lys
  variant (29)..(29): Thr or Gln or Ser or Asn or Arg or Lys
  variant (30)..(30): Thr or Gln or Ser or Asn or Arg or Lys

SEQ ID NO: 168 - protein, 30 aa, artificial; identical to SEQ ID NO: 121
  pattern
  variant (1)..(1): Thr or Gln or Ser or Asn or Arg or Lys
  variant (2)..(2): Thr or Gln or Ser or Asn or Arg or Lys
  variant (3)..(3): Thr or Gln or Ser or Asn or Arg or Lys
  variant (4)..(4): Thr or Gln or Ser or Asn or Arg or Lys
  variant (5)..(5): Ala or Met or Val or Leu or Ile
  variant (6)..(6): Arg or Lys
  variant (7)..(7): Arg or Lys
  variant (8)..(8): Trp or Phe
  variant (9)..(9): Trp or Phe
  variant (10)..(10): Arg or Lys
  variant (11)..(11): Arg or Lys
  variant (12)..(12): Ala or Met or Val or Leu or Ile
  variant (13)..(13): Ala or Met or Val or Leu or Ile
  variant (14)..(14): Thr or Gln or Ser or Asn
  variant (15)..(15): Ala or Met or Val or Leu or Ile
  variant (16)..(16): Ala or Met or Val or Leu or Ile
  variant (17)..(17): Asp or Glu
  variant (18)..(18): Thr or Gln or Ser or Asn
  variant (19)..(19): Ala or Met or Val or Leu or Ile
  variant (20)..(20): Trp or Phe
  variant (21)..(21): Thr or Gln or Ser or Asn
  variant (22)..(22): Asp or Glu
  variant (23)..(23): Ala or Met or Val or Leu or Ile
  variant (24)..(24): Asp or Glu
  variant (25)..(25): Asp or Glu
  variant (26)..(26): Trp or Phe
  variant (27)..(27): Thr or Gln or Ser or Asn or Arg or Lys
  variant (28)..(28): Thr or Gln or Ser or Asn or Arg or Lys
  variant (29)..(29): Thr or Gln or Ser or Asn or Arg or Lys
  variant (30)..(30): Thr or Gln or Ser or Asn or Arg or Lys

SEQ ID NO: 169 - protein, 30 aa, artificial; identical to SEQ ID NO: 121
  pattern
  variant (1)..(1): Thr or Gln or Ser or Asn or Arg or Lys
  variant (2)..(2): Thr or Gln or Ser or Asn or Arg or Lys
  variant (3)..(3): Thr or Gln or Ser or Asn or Arg or Lys
  variant (4)..(4): Thr or Gln or Ser or Asn or Arg or Lys
  variant (5)..(5): Ala or Met or Val or Leu or Ile
  variant (6)..(6): Asp or Glu
  variant (7)..(7): Asp or Glu
  variant (8)..(8): Trp or Phe
  variant (9)..(9): Trp or Phe
  variant (10)..(10): Asp or Glu
  variant (11)..(11): Asp or Glu
  variant (12)..(12): Ala or Met or Val or Leu or Ile
  variant (13)..(13): Ala or Met or Val or Leu or Ile
  variant (14)..(14): Thr or Gln or Ser or Asn
  variant (15)..(15): Ala or Met or Val or Leu or Ile
  variant (16)..(16): Ala or Met or Val or Leu or Ile
  variant (17)..(17): Arg or Lys
  variant (18)..(18): Thr or Gln or Ser or Asn
  variant (19)..(19): Ala or Met or Val or Leu or Ile
  variant (20)..(20): Trp or Phe
  variant (21)..(21): Thr or Gln or Ser or Asn
  variant (22)..(22): Arg or Lys
  variant (23)..(23): Ala or Met or Val or Leu or Ile
  variant (24)..(24): Arg or Lys
  variant (25)..(25): Arg or Lys
  variant (26)..(26): Trp or Phe
  variant (27)..(27): Thr or Gln or Ser or Asn or Arg or Lys
  variant (28)..(28): Thr or Gln or Ser or Asn or Arg or Lys
  variant (29)..(29): Thr or Gln or Ser or Asn or Arg or Lys
  variant (30)..(30): Thr or Gln or Ser or Asn or Arg or Lys

SEQ ID NO: 170 - protein, 30 aa, artificial; identical to SEQ ID NO: 121
  pattern
  variant (1)..(1): Thr or Gln or Ser or Asn or Arg or Lys
  variant (2)..(2): Thr or Gln or Ser or Asn or Arg or Lys
  variant (3)..(3): Thr or Gln or Ser or Asn or Arg or Lys
  variant (4)..(4): Thr or Gln or Ser or Asn or Arg or Lys
  variant (5)..(5): Ala or Met or Val or Leu or Ile
  variant (6)..(6): Arg or Lys
  variant (7)..(7): Arg or Lys
  variant (8)..(8): Trp or Phe
  variant (9)..(9): Trp or Phe
  variant (10)..(10): Arg or Lys
  variant (11)..(11): Arg or Lys
  variant (12)..(12): Ala or Met or Val or Leu or Ile
  variant (13)..(13): Ala or Met or Val or Leu or Ile
  variant (14)..(14): Thr or Gln or Ser or Asn
  variant (15)..(15): Ala or Met or Val or Leu or Ile
  variant (16)..(16): Ala or Met or Val or Leu or Ile
  variant (17)..(17): Thr or Gln or Ser or Asn
  variant (18)..(18): Thr or Gln or Ser or Asn
  variant (19)..(19): Ala or Met or Val or Leu or Ile
  variant (20)..(20): Trp or Phe
  variant (21)..(21): Asp or Glu
  variant (22)..(22): Asp or Glu
  variant (23)..(23): Ala or Met or Val or Leu or Ile
  variant (24)..(24): Asp or Glu
  variant (25)..(25): Asp or Glu
  variant (26)..(26): Trp or Phe
  variant (27)..(27): Thr or Gln or Ser or Asn or Arg or Lys
  variant (28)..(28): Thr or Gln or Ser or Asn or Arg or Lys
  variant (29)..(29): Thr or Gln or Ser or Asn or Arg or Lys
  variant (30)..(30): Thr or Gln or Ser or Asn or Arg or Lys

SEQ ID NO: 171 - protein, 30 aa, artificial; identical to SEQ ID NO: 121
  pattern
  variant (1)..(1): Thr or Gln or Ser or Asn or Arg or Lys
  variant (2)..(2): Thr or Gln or Ser or Asn or Arg or Lys
  variant (3)..(3): Thr or Gln or Ser or Asn or Arg or Lys
  variant (4)..(4): Thr or Gln or Ser or Asn or Arg or Lys
  variant (5)..(5): Ala or Met or Val or Leu or Ile
  variant (6)..(6): Asp or Glu
  variant (7)..(7): Asp or Glu
  variant (8)..(8): Trp or Phe
  variant (9)..(9): Trp or Phe
  variant (10)..(10): Asp or Glu
  variant (11)..(11): Asp or Glu
  variant (12)..(12): Ala or Met or Val or Leu or Ile
  variant (13)..(13): Ala or Met or Val or Leu or Ile
  variant (14)..(14): Thr or Gln or Ser or Asn
  variant (15)..(15): Ala or Met or Val or Leu or Ile
  variant (16)..(16): Ala or Met or Val or Leu or Ile
  variant (17)..(17): Thr or Gln or Ser or Asn
  variant (18)..(18): Thr or Gln or Ser or Asn
  variant (19)..(19): Ala or Met or Val or Leu or Ile
  variant (20)..(20): Trp or Phe
  variant (21)..(21): Arg or Lys
  variant (22)..(22): Arg or Lys
  variant (23)..(23): Ala or Met or Val or Leu or Ile
  variant (24)..(24): Arg or Lys
  variant (25)..(25): Arg or Lys
  variant (26)..(26): Trp or Phe
  variant (27)..(27): Thr or Gln or Ser or Asn or Arg or Lys
  variant (28)..(28): Thr or Gln or Ser or Asn or Arg or Lys
  variant (29)..(29): Thr or Gln or Ser or Asn or Arg or Lys
  variant (30)..(30): Thr or Gln or Ser or Asn or Arg or Lys

SEQ ID NO: 172 - protein, 30 aa, artificial; identical to SEQ ID NO: 121
  pattern
  variant (1)..(1): Thr or Gln or Ser or Asn or Arg or Lys
  variant (2)..(2): Thr or Gln or Ser or Asn or Arg or Lys
  variant (3)..(3): Thr or Gln or Ser or Asn or Arg or Lys
  variant (4)..(4): Thr or Gln or Ser or Asn or Arg or Lys
  variant (5)..(5): Ala or Met or Val or Leu or Ile
  variant (6)..(6): Asp or Glu
  variant (7)..(7): Asp or Glu
  variant (8)..(8): Trp or Phe
  variant (9)..(9): Trp or Phe
  variant (10)..(10): Asp or Glu
  variant (11)..(11): Asp or Glu
  variant (12)..(12): Ala or Met or Val or Leu or Ile
  variant (13)..(13): Ala or Met or Val or Leu or Ile
  variant (14)..(14): Thr or Gln or Ser or Asn
  variant (15)..(15): Ala or Met or Val or Leu or Ile
  variant (16)..(16): Ala or Met or Val or Leu or Ile
  variant (17)..(17): Arg or Lys
  variant (18)..(18): Thr or Gln or Ser or Asn
  variant (19)..(19): Ala or Met or Val or Leu or Ile
  variant (20)..(20): Trp or Phe
  variant (21)..(21): Arg or Lys
  variant (22)..(22): Arg or Lys
  variant (23)..(23): Ala or Met or Val or Leu or Ile
  variant (24)..(24): Arg or Lys
  variant (25)..(25): Arg or Lys
  variant (26)..(26): Trp or Phe
  variant (27)..(27): Thr or Gln or Ser or Asn or Arg or Lys
  variant (28)..(28): Thr or Gln or Ser or Asn or Arg or Lys
  variant (29)..(29): Thr or Gln or Ser or Asn or Arg or Lys
  variant (30)..(30): Thr or Gln or Ser or Asn or Arg or Lys

SEQ ID NO: 173 - protein, 30 aa, artificial
  RDWA1
NQRRLRRILNQLWQWIDDLINQLQNIRRQN

SEQ ID NO: 174 - protein, 30 aa, artificial
  RDFA1
NQRRLRRILNQLFQFIDDLINQLQNIRRQN

SEQ ID NO: 175 - protein, 30 aa, artificial
  RDWA1i
NQRRLRRILNQLWQWIDQLINDLQNIRRQN

SEQ ID NO: 176 - protein, 30 aa, artificial
  RDFA1i
NQRRLRRILNQLFQFIDQLINDLQNIRRQN

SEQ ID NO: 177 - protein, 30 aa, artificial
  RDWA1ii
NQRRLRNILNRLWQWIDQLINDLQNIRRQN

SEQ ID NO: 178 - protein, 30 aa, artificial
  RDFA1ii
NQRRLRNILNRLFQFIDQLINDLQNIRRQN

SEQ ID NO: 179 - protein, 30 aa, artificial
  RDWA2
NQRRLRRILNQLWQWINQLDNQLQDIRRQN

SEQ ID NO: 180 - protein, 30 aa, artificial
  RDFA2
NQRRLRRILNQLFQFINQLDNQLQDIRRQN

SEQ ID NO: 181 - protein, 30 aa, artificial
  KDFA2
NQKKLKKILNQLFQFINQLDNQLQDIKKQN

SEQ ID NO: 182 - protein, 30 aa, artificial
  KDFA2SV
SSKKVKKVVSSVFSFVSSVDSSVSDVKKSS

SEQ ID NO: 183 - protein, 30 aa, artificial
  RDFA2i
NQRRLRRILNQLFQFINQLDNQLQDIRQNR

SEQ ID NO: 184 - protein, 30 aa, artificial
  RDFA2i+8
RRRRLRRILRRLFQFINQLDNQLQDIRQNR

SEQ ID NO: 185 - protein, 30 aa, artificial; identical to SEQ ID NO: 184
  RDFA2i+9-NH2

SEQ ID NO: 186 - protein, 30 aa, artificial
  RDFA2i+9-NH2-Kter
KKKKLRRILRRLFQFINQLDNQLQDIKQNK

SEQ ID NO: 187 - protein, 30 aa, artificial
  KDFA2i+9-NH2-Rter
RRRRLKKILKKLFQFINQLDNQLQDIRQNR

SEQ ID NO: 188 - protein, 30 aa, artificial
  RDFA2i+8SV
RRRRVRRVVRRVFSFVSSVDSSVSDVRSSR

SEQ ID NO: 189 - protein, 30 aa, artificial; identical to SEQ ID NO: 83
  KDFA2i+8

SEQ ID NO: 190 - protein, 30 aa, artificial
  KDFA2i+7-npNH2
KKKKLKKILKKLFQFINQLDNQLQDIAQNA

SEQ ID NO: 191 - protein, 30 aa, artificial
  KDFA2i+10-Hter
HHHHLKKILKKLFQFINQLDNQLQDIHHHH

SEQ ID NO: 192 - protein, 30 aa, artificial
  RDFA2i+9(Q18R)
RRRRLRRILRRLFQFINRLDNQLQDIRQNR

SEQ ID NO: 193 - protein, 30 aa, artificial
  RDFA2ii
NQRRLRRILNQLFQFINQLDNQLQDIRNQN

SEQ ID NO: 194 - protein, 30 aa, artificial
  RDFA2ii+7
RRRRLRRILRRLFQFINQLDNQLQDIRNQN

SEQ ID NO: 195 - protein, 30 aa, artificial
  RDFA2iii
RRNQLRRILNQLFQFINQLDNQLQDINQRR

SEQ ID NO: 196 - protein, 30 aa, artificial
  RDWA2iv
NQRRLRRILNQLWQWINQLDNDLQNIRRQN

SEQ ID NO: 197 - protein, 30 aa, artificial
  RDFA2iv
NQRRLRRILNQLFQFINQLDNDLQNIRRQN

SEQ ID NO: 198 - protein, 30 aa, artificial
  RDWA2v
NQRRLRRILNRLWQWINQLDNDLQNIRRQN

SEQ ID NO: 199 - protein, 30 aa, artificial
  RDFA2v
NQRRLRNILNRLFQFINQLDNDLQNIRRQN

SEQ ID NO: 200 - protein, 30 aa, artificial
  RDWA3
NQRRLRRILNQLWQWINQLIDDLQNIRRQN

SEQ ID NO: 201 - protein, 30 aa, artificial
  RDFA3
NQRRLRRILNQLFQFINQLIDDLQNIRRQN

SEQ ID NO: 202 - protein, 30 aa, artificial
  RDWA4
NQRRLRRILNQLWQWINQLINQLDDIRRQN

SEQ ID NO: 203 - protein, 30 aa, artificial
  RDFA4
NQRRLRRILNQLFQFINQLINQLDDIRRQN

SEQ ID NO: 204 - protein, 30 aa, artificial
  RDFA4i
RQRRLRRILNQLFQFINQLINQLDDINQNR

SEQ ID NO: 205 - protein, 30 aa, artificial
  RDFA4ii
RQNRLRRILNQLFQFINQLINQLDDINQNR

SEQ ID NO: 206 - protein, 30 aa, artificial
  RDFA4iii
RRNQLRRILNQLFQFINQLINQLDDINQRR

SEQ ID NO: 207 - protein, 30 aa, artificial
  RDWA4iv
RQRRLRNILNRLWQWINQLINDLDNINQNR

SEQ ID NO: 208 - protein, 30 aa, artificial
  RDFA4iv
RQRRLRNILNRLFQFINQLINDLDNINQNR

SEQ ID NO: 209 - protein, 30 aa, artificial
  RDWA5
NQRRLQNILRRLWQWIDQLINDLQNIRRQN

SEQ ID NO: 210 - protein, 30 aa, artificial
  RDFA5
NQRRLQNILRRLFQFIDQLINDLQNIRRQN

SEQ ID NO: 211 - protein, 30 aa, artificial
  KDFA5+11-NH2
KKKKLKKILKKLFQFIDQLINDLQNIKKKK

SEQ ID NO: 212 - protein, 30 aa, artificial
  RDWA5i
NQRRLQRILRQLWQWIDQLINQLQDIRRQN

SEQ ID NO: 213 - protein, 30 aa, artificial
  RDWA5+11
RRRRLRRILRRLWQWIDQLINDLRNIRRRR

SEQ ID NO: 214 - protein, 30 aa, artificial
  RDFA5+11
RRRRLRRILRRLFQFIDQLINDLRNIRRRR

SEQ ID NO: 215 - protein, 30 aa, artificial
  KDFA5+11
KKKKLKKILKKLFQFIDQLINDLKNIKKKK

SEQ ID NO: 216 - protein, 30 aa, artificial
  RDWA6
NQRRLQNILRRLWQWINDLDNQLQNIRRQN

SEQ ID NO: 217 - protein, 30 aa, artificial
  RDFA6
NQRRLQNILRRLFQFINDLDNQLQNIRRQN

SEQ ID NO: 218 - protein, 30 aa, artificial
  RDWA6i
NQRRLQNILRRLWQWINQLDNDLQNIRRQN

SEQ ID NO: 219 - protein, 30 aa, artificial
  RDWA7
NQRRLQNILRRLWQWINQLIDDLQNIRRQN

SEQ ID NO: 220 - protein, 30 aa, artificial
  RDFA7
NQRRLQNILRRLFQFINQLIDDLQNIRRQN

SEQ ID NO: 221 - protein, 30 aa, artificial
  RDFA7+10
RRRRLRRILRRLFQFINQLIDDLQNIRRRR

SEQ ID NO: 222 - protein, 30 aa, artificial
  KDFA7+10
KKKKLKKILKKLFQFINQLIDDLQNIKKKK

SEQ ID NO: 223 - protein, 30 aa, artificial
  RDWA7i
NQRRLQRILRQLWQWINQLIDQLQDIRRQN

SEQ ID NO: 224 - protein, 30 aa, artificial
  RDWA8
NQRRLQNILRRLWQWINQLINQLDDIRRQN

SEQ ID NO: 225 - protein, 30 aa, artificial
  RDFA8
NQRRLQNILRRLFQFINQLINQLDDIRRQN

SEQ ID NO: 226 - protein, 30 aa, artificial
  RDWA8i
NQRRLQNILRRLWQWINQLINDLDNIRRQN

SEQ ID NO: 227 - protein, 30 aa, artificial
  RDFA8i
NQRRLQNILRRLFQFINQLINDLDNIRRQN

SEQ ID NO: 228 - protein, 30 aa, artificial
  RDWA9
NQRRLQNILNRLWRWIDDLINQLQNIRRQN

SEQ ID NO: 229 - protein, 30 aa, artificial
  KDFA9
NQKKLQNILNKLFKFIDDLINQLQNIKKQN

SEQ ID NO: 230 - protein, 30 aa, artificial
  RDWB10
NQRRLRRWWNQLIQLIDQLWNDLQNWRRQN

SEQ ID NO: 231 - protein, 30 aa, artificial
  RDFB10
NQRRLRRFFNQLIQLIDQLFNDLQNFRRQN

SEQ ID NO: 232 - protein, 30 aa, artificial
  RDWB11
NQRRLRRWWNQLIQLINQLWDDLQNWRRQN

SEQ ID NO: 233 - protein, 30 aa, artificial
  RDFB11
NQRRLRRFFNQLIQLINQLFDDLQNFRRQN

SEQ ID NO: 234 - protein, 30 aa, artificial
  RDWB12
NQRRLRRWWNQLIQLINQLWNQLDDWRRQN

SEQ ID NO: 235 - protein, 30 aa, artificial
  RDFB12
NQRRLRRFFNQLIQLINQLFNQLDDFRRQN

SEQ ID NO: 236 - protein, 30 aa, artificial
  KDFB12
KQKKLKKFFNQLIQLINQLFNQLDDFNQNK

SEQ ID NO: 237 - protein, 30 aa, artificial
  KDFB12SV
KSKKVKKFFSSVVSVVSSVFSSVDDFSSSK

SEQ ID NO: 238 - protein, 30 aa, artificial
  RDFB12i
RRQNLRNWWNRLIQLINQLWNDLDNWNQRR

SEQ ID NO: 239 - protein, 30 aa, artificial
  RDWB13
NQRRLQNWWRRLIQLIDQLWNDLQNWRRQN

SEQ ID NO: 240 - protein, 30 aa, artificial
  RDFB13
NQRRLQNFFRRLIQLIDQLFNDLQNFRRQN

SEQ ID NO: 241 - protein, 30 aa, artificial
  RDWB14
NQRRLQNWWRRLIQLINQLWDDLQNWRRQN

SEQ ID NO: 242 - protein, 30 aa, artificial
  RDFB14
NQRRLQNFFRRLIQLINQLFDDLQNFRRQN

SEQ ID NO: 243 - protein, 30 aa, artificial
  RDWB15
NQRRLQNWWRRLIQLINQLWNDLDNWRRQN

SEQ ID NO: 244 - protein, 30 aa, artificial
  RDFB15
NQRRLQNFFRRLIQLINQLFNDLDNFRRQN

SEQ ID NO: 245 - protein, 30 aa, artificial
  RDWC16
NQRRLRRILRRLWQWIDQLDNDLQDIRRQN

SEQ ID NO: 246 - protein, 30 aa, artificial
  RDFC16
NQRRLRRILRRLFQFIDQLDNDLQDIRRQN

SEQ ID NO: 247 - protein, 30 aa, artificial
  RDWC16Kter
NQKKLRRILRRLWQWIDQLDNDLQDIKKQN

SEQ ID NO: 248 - protein, 30 aa, artificial
  RDFC16Kter
NQKKLRRILRRLFQFIDQLDNDLQDIKKQN

SEQ ID NO: 249 - protein, 30 aa, artificial; identical to SEQ ID NO: 89
  KDFC16+9-NH2

SEQ ID NO: 250 - protein, 30 aa, artificial
  KDFC16+8SV
KKKKVKKVVKKVFSFVDSVDSDVSDVKKKK

SEQ ID NO: 251 - protein, 30 aa, artificial; identical to SEQ ID NO: 250
  KDFC16+9SV-NH2

SEQ ID NO: 252 - protein, 30 aa, artificial
  DRFC16
NQRRLDDILDDLFQFIRQLRNRLQRIRRQN

SEQ ID NO: 253 - protein, 30 aa, artificial
  DKFC16+8
KKKKLDDILDDLFQFIKQLKNKLQKIKKKK

SEQ ID NO: 254 - protein, 30 aa, artificial; identical to SEQ ID NO: 253
  DKFC16+9-NH2

SEQ ID NO: 255 - protein, 30 aa, artificial
  RDWC17
NQRRLRRILRRLWQWIDQLIDDLQDIRRQN

SEQ ID NO: 256 - protein, 30 aa, artificial
  RDFC17
NQRRLRRILRRLFQFIDQLIDDLQDIRRQN

SEQ ID NO: 257 - protein, 30 aa, artificial
  KDFC17+8
KKKKLKKILKKLFQFIDQLIDDLQDIKKKK

SEQ ID NO: 258 - protein, 30 aa, artificial
  RDWC18
NQRRLRRILRRLWQWIDQLINDLDDIRRQN

SEQ ID NO: 259 - protein, 30 aa, artificial
  RDFC18
NQRRLRRILRRLFQFIDQLINDLDDIRRQN

SEQ ID NO: 260 - protein, 30 aa, artificial
  KDFC18+8
KKKKLKKILKKLFQFIDQLINDLDDIKKKK

SEQ ID NO: 261 - protein, 30 aa, artificial
  RDWC19
NQRRLRRILRRLWQWINQLDDDLQDIRRQN

SEQ ID NO: 262 - protein, 30 aa, artificial
  RDFC19
NQRRLRRILRRLFQFINQLDDDLQDIRRQN

SEQ ID NO: 263 - protein, 30 aa, artificial
  KDFC19+8
KKKKLKKILKKLFQFINQLDDDLQDIKKKK

SEQ ID NO: 264 - protein, 30 aa, artificial
  RDWC20
NQRRLRRILRRLWQWINQLDNDLDDIRRQN

SEQ ID NO: 265 - protein, 30 aa, artificial
  RDFC20
NQRRLRRILRRLFQFINQLDNDLDDIRRQN

SEQ ID NO: 266 - protein, 30 aa, artificial
  KDFC20+8
KKKKLKKILKKLFQFINQLDNDLDDIKKKK

SEQ ID NO: 267 - protein, 30 aa, artificial
  RDWC21
NQRRLRRILRRLWQWINQLIDDLDDIRRQN

SEQ ID NO: 268 - protein, 30 aa, artificial
  RDFC21
NQRRLRRILRRLFQFINQLIDDLDDIRRQN

SEQ ID NO: 269 - protein, 30 aa, artificial
  KDFC21+8
KKKKLKKILKKLFQFINQLIDDLDDIKKKK

SEQ ID NO: 270 - protein, 30 aa, artificial; identical to SEQ ID NO: 269
  KDFC21+9-NH2

SEQ ID NO: 271 - protein, 30 aa, artificial
  DRWC21
NQRRLDDILDDLWQWINQLIRRLRRIRRQN

SEQ ID NO: 272 - protein, 30 aa, artificial
  DKWC21+8
KKKKLDDILDDLWQWINQLIKKLKKIKKKK

SEQ ID NO: 273 - protein, 30 aa, artificial
  RDWD22
NQRRLRRWWRRLIQLIDQLWDDLQDWRRQN

SEQ ID NO: 274 - protein, 30 aa, artificial
  RDFD22
NQRRLRRFFRRLIQLIDQLFDDLQDFRRQN

SEQ ID NO: 275 - protein, 30 aa, artificial
  RDWD23
NQRRLRRWWRRLIQLIDQLWNDLDDWRRQN

SEQ ID NO: 276 - protein, 30 aa, artificial
  RDFD23
NQRRLRRFFRRLIQLIDQLFNDLDDFRRQN

SEQ ID NO: 277 - protein, 30 aa, artificial
  RDWD24
NQRRLRRWWRRLIQLINQLWDDLDDWRRQN

SEQ ID NO: 278 - protein, 30 aa, artificial
  RDFD24
NQRRLRRFFRRLIQLINQLFDDLDDFRRQN

SEQ ID NO: 279 - protein, 30 aa, artificial
  KDFD24+8
KKKKLKKFFKKLIQLINQLFDDLDDFKKKK

SEQ ID NO: 280 - protein, 30 aa, artificial; identical to SEQ ID NO: 279
  KDFD24+9-NH2

SEQ ID NO: 281 - protein, 30 aa, artificial
  KDFD24+8SV
KKKKVKKFFKKVVSVVSSVFDDVDDFKKKK

SEQ ID NO: 282 - protein, 30 aa, artificial
  RD2i
NQRRLRRILNQLIQLINQLDNQLQDIRQNR

SEQ ID NO: 283 - protein, 30 aa, artificial
  RD4i
RQRRLRRILNQLIQLINQLINQLDDINQNR

SEQ ID NO: 284 - protein, 30 aa, artificial
  RD5
NQRRLQNILRRLIQLIDQLINDLQNIRRQN

SEQ ID NO: 285 - protein, 30 aa, artificial
  RD7
NQRRLQNILRRLIQLINQLIDDLQNIRRQN

SEQ ID NO: 286 - protein, 30 aa, artificial
  RD16
NQRRLRRILRRLIQLIDQLDNDLQDIRRQN

SEQ ID NO: 287 - protein, 30 aa, artificial
  KD16+9-NH2
KKKKVKKILKKLIQLIDQLDNDLQDIKKKK

SEQ ID NO: 288 - protein, 30 aa, artificial
  RD21
NQRRLRRILRRLIQLINQLIDDLDDIRRQN

SEQ ID NO: 289 - protein, 26 aa, artificial
  Melittin
GIGAVLKVLTTGLPALISWIKRKRQQ

SEQ ID NO: 290 - protein, 5 aa, artificial
  motif in prior art
  unsure (2)..(4)
GXXXG